European Patent Application EP 4 144 370 A1, published March 8, 2023. Title: Bispecific Antibodies. Applicant: Daiichi Sankyo Company, Limited Mie University. The sequence listing filed with the application follows.

SEQUENCE LISTING (198 sequences)

SEQ ID NO: 1 - protein, 9 aa, Artificial
  Peptide sequence of NY-ESO
SLLMWITQC

SEQ ID NO: 2 - protein, 10 aa, Artificial
  Peptide sequence of MAGEC-1
ILFGISLREV

SEQ ID NO: 3 - DNA, 26 bp, Artificial
  Primer for analyzing scFv sequence
ctcttcgctattacgccagctggcga

SEQ ID NO: 4 - DNA, 30 bp, Artificial
  Primer for analyzing scFv sequence
ataacaatttcacacaggaaacagctatga

SEQ ID NO: 5 - DNA, 360 bp, Artificial
  Nucleotide sequence of a heavy chain variable region of NYA-0001
gaggtgcagctggtggagtctgggggaggcgtggtccagcctgggaggtccctgacaccctcctgttcagcgtctggattctccatccgtagttatgatatacactgggtccgccaggctccaggcaaggggctagagtgggtggccactatatcatatgatggaagtcagaagtacttcgcagactccgtgaagggccgatttaccatcttcagagacgaatcggagaacatggtgtatctgcaaatgagcggcctgagagttgaggacacggctgtttatcactgtgcgagagggagtagtggtcattatgaggcttttgatatctggggccaagggacaatggtcaccgtctcttca

SEQ ID NO: 6 - protein, 120 aa, Artificial
  Amino acid sequence of a heavy chain variable region of NYA-0001
EVQLVESGGGVVQPGRSLTPSCSASGFSIRSYDIHWVRQAPGKGLEWVATISYDGSQKYFADSVKGRFTIFRDESENMVYLQMSGLRVEDTAVYHCARGSSGHYEAFDIWGQGTMVTVSS

SEQ ID NO: 7 - DNA, 333 bp, Artificial
  Nucleotide sequence of a light chain variable region of NYA-0001
cagtctgtgttgacgcagccgccctcagtgtctgcggccccaggacagaaggtcaccatctcctgctctggaagcagctccaacattgggaataattatgtatcctggtaccagcagctcccaggaacagcccccaaactcctcatttatgacaataataagcgaccctcagggattcctgaccgattctctggctccaagtctggcacgtcagccaccctgggcatcaccggactccagactggggacgaggccgattattactgcggaacatgggatagcagcctgagtgccccttgggtgttcggcggagggaccaaggtcaccgtccta

SEQ ID NO: 8 - protein, 111 aa, Artificial
  Amino acid sequence of a light chain variable region of NYA-0001
QSVLTQPPSVSAAPGQKVTISCSGSSSNIGNNYVSWYQQLPGTAPKLLIYDNNKRPSGIPDRFSGSKSGTSATLGITGLQTGDEADYYCGTWDSSLSAPWVFGGGTKVTVL

SEQ ID NO: 9 - DNA, 360 bp, Artificial
  Nucleotide sequence of a heavy chain variable region of NYA-0060
gaggtgcagctggtggagtctgggggaggcgtggtccagcctgggaggtccctgacaccctcctgttcagcgtctggattctccatccgtagctatgatatacactgggtccgcctggctccaggcaaggggctagagtgggtggccactatatcatatgatggaagtcagaagtacttcgcagactccgtgaagggccgatttaccatcttcagagacgaatcggagaacatggtgtatctgcaaatgagcggcctgagagttgaggacacggctgtttatcactgtgcgagagggagtagtggtcattatgaggcttttgatatctggggccaagggacaatggtcaccgtctcttca

SEQ ID NO: 10 - protein, 120 aa, Artificial
  Amino acid sequence of a heavy chain variable region of NYA-0060
EVQLVESGGGVVQPGRSLTPSCSASGFSIRSYDIHWVRLAPGKGLEWVATISYDGSQKYFADSVKGRFTIFRDESENMVYLQMSGLRVEDTAVYHCARGSSGHYEAFDIWGQGTMVTVSS

SEQ ID NO: 11 - DNA, 333 bp, Artificial; identical to SEQ ID NO: 7
  Nucleotide sequence of a light chain variable region of NYA-0060

SEQ ID NO: 12 - protein, 111 aa, Artificial; identical to SEQ ID NO: 8
  Amino acid sequence of a light chain variable region of NYA-0060

SEQ ID NO: 13 - DNA, 360 bp, Artificial; identical to SEQ ID NO: 5
  Nucleotide sequence of a heavy chain variable region of NYA-0068

SEQ ID NO: 14 - protein, 120 aa, Artificial; identical to SEQ ID NO: 6
  Amino acid sequence of a heavy chain variable region of NYA-0068

SEQ ID NO: 15 - DNA, 333 bp, Artificial
  Nucleotide sequence of a light chain variable region of NYA-0068
cagtctgtgttgacgcagccgccctcagtgtctgcggccccaggacagaaggtcaccatctcctgctctggaagcagctccaacattgggaattggtatgtatcctggtaccagcagctcccaggaacagcccccaaactcctcatttatgacaataataagcgaccctcagggattcctgaccgattctctggctccaagtctggcacgtcagccaccctgggcatcaccggactccagactggggacgaggccgattattactgcggaacatgggatagcagcctgagtgccccttgggtgttcggcggagggaccaaggtcaccgtccta

SEQ ID NO: 16 - protein, 111 aa, Artificial
  Amino acid sequence of a light chain variable region of NYA-0068
QSVLTQPPSVSAAPGQKVTISCSGSSSNIGNWYVSWYQQLPGTAPKLLIYDNNKRPSGIPDRFSGSKSGTSATLGITGLQTGDEADYYCGTWDSSLSAPWVFGGGTKVTVL

SEQ ID NO: 17 - DNA, 360 bp, Artificial; identical to SEQ ID NO: 5
  Nucleotide sequence of a heavy chain variable region of NYA-0082

SEQ ID NO: 18 - protein, 120 aa, Artificial; identical to SEQ ID NO: 6
  Amino acid sequence of a heavy chain variable region of NYA-0082

SEQ ID NO: 19 - DNA, 333 bp, Artificial
  Nucleotide sequence of a light chain variable region of NYA-0082
cagtctgtgttgacgcagccgccctcagtgtctgcggccccaggacagaaggtcaccatctcctgctctggaagcagctccaacattgggaataattatgtatcctggtaccagcggctcccaggaacagcccccaaactcctcatttatgacaataataagcgaccctcagggattcctgaccgattctctggctccaagtctggcacgtcagccaccctgggcatcaccggactccagactggggacgaggccgattattactgcggatcatgggatagcagcctgagtgccccttgggtgttcggcggagggaccaaggtcaccgtccta

SEQ ID NO: 20 - protein, 111 aa, Artificial
  Amino acid sequence of a light chain variable region of NYA-0082
QSVLTQPPSVSAAPGQKVTISCSGSSSNIGNNYVSWYQRLPGTAPKLLIYDNNKRPSGIPDRFSGSKSGTSATLGITGLQTGDEADYYCGSWDSSLSAPWVFGGGTKVTVL

SEQ ID NO: 21 - DNA, 876 bp, Artificial
  Full-length nucleotide sequence of NYA-1163
atgaaacacctgtggttcttcctcctgctggtggcagctcccagatgggtgctgagcggagaggtgcagctggtggagtctgggggaggcgtggtccagcctgggaggtccctgacaccctcctgttcagcgtctggattctccatccgtagctatgatatacactgggtccgcctggctccaggcaaggggctagagtgggtggccactatatcatatgatggaagtcagaagtacttcgcagactccgtgaagggccgatttaccatcttcagagacgaatcggagaacatggtgtatctgcaaatgagcggcctgagagttgaggacacggctgtttatcactgtgcgagagggagtagtggtcattatgaggcttttgatatctggggccaagggacaatggtcaccgtctcttcaggtggaggcggttcaggcggaggtggcagcggcggtggcgggagtcagtctgtgttgacgcagccgccctcagtgtctgcggccccaggacagaaggtcaccatctcctgctctggaagcagctccaacattgggaataattatgtatcctggtaccagcagctcccaggaacagcccccaaactcctcatttatgacaataataagcgaccctcagggattcctgaccgattctctggctccaagtctggcacgtcagccaccctgggcatcaccggactccagactggggacgaggccgattattactgcggaacatgggatagcagcctgagtgccccttgggtgttcggcggagggaccaaggtcaccgtcctaggcgcggccgcaggtgcaggtggtgattacaaagatgatgacgataaaggtgcagcggcgcatcaccatcatcaccac

SEQ ID NO: 22 - DNA, 876 bp, Artificial
  Full-length nucleotide sequence of NYA-2023
atgaaacacctgtggttcttcctcctgctggtggcagctcccagatgggtgctgagcggagaggtgcagctggtggagtctgggggaggcgtggtccagcctgggaggtccctgacaccctcctgttcagcgtctggattctccatccgtagttatgatatacactgggtccgccaggctccaggcaaggggctagagtgggtggccactatatcatatgatggaagtcagaagtacttcgcagactccgtgaagggccgatttaccatcttcagagacgaatcggagaacatggtgtatctgcaaatgagcggcctgagagttgaggacacggctgtttatcactgtgcgagagggagtagtggtcattatgaggcttttgatatctggggccaagggacaatggtcaccgtctcttcaggtggaggcggttcaggcggaggtggcagcggcggtggcgggagtcagtctgtgttgacgcagccgccctcagtgtctgcggccccaggacagaaggtcaccatctcctgctctggaagcagctccaacattgggaattggtatgtatcctggtaccagcagctcccaggaacagcccccaaactcctcatttatgacaataataagcgaccctcagggattcctgaccgattctctggctccaagtctggcacgtcagccaccctgggcatcaccggactccagactggggacgaggccgattattactgcggaacatgggatagcagcctgagtgccccttgggtgttcggcggagggaccaaggtcaccgtcctaggcgcggccgcaggtgcaggtggtgattacaaagatgatgacgataaaggtgcagcggcgcatcaccatcatcaccac

SEQ ID NO: 23 - DNA, 876 bp, Artificial
  Full-length nucleotide sequence of NYA-2027
atgaaacacctgtggttcttcctcctgctggtggcagctcccagatgggtgctgagcggagaggtgcagctggtggagtctgggggaggcgtggtccagcctgggaggtccctgacaccctcctgttcagcgtctggattctccatccgtagttatgatatacactgggtccgccaggctccaggcaaggggctagagtgggtggccactatatcatatgatggaagtcagaagtacttcgcagactccgtgaagggccgatttaccatcttcagagacgaatcggagaacatggtgtatctgcaaatgagcggcctgagagttgaggacacggctgtttatcactgtgcgagagggagtagtggtcattatgaggcttttgatatctggggccaagggacaatggtcaccgtctcttcaggtggaggcggttcaggcggaggtggcagcggcggtggcgggagtcagtctgtgttgacgcagccgccctcagtgtctgcggccccaggacagaaggtcaccatctcctgctctggaagcagctccaacattgggaataattatgtatcctggtaccagcagctcccaggaacagcccccaaactcctcatttatgacaataataagcgaccctcagggattcctgaccgattctctggctccaagtctggcacgtcagccaccctgggcatcaccggactccagactggggacgaggccgattattactgcggatcatgggatagcagcctgagtgccccttgggtgttcggcggagggaccaaggtcaccgtcctaggcgcggccgcaggtgcaggtggtgattacaaagatgatgacgataaaggtgcagcggcgcatcaccatcatcaccac

SEQ ID NO: 24 - DNA, 876 bp, Artificial
  Full-length nucleotide sequence of NYA-1143
atgaaacacctgtggttcttcctcctgctggtggcagctcccagatgggtgctgagcggagaggtgcagctggtggagtctgggggaggcgtggtccagcctgggaggtccctgacaccctcctgttcagcgtctggattctccatccgtagctatgatatacactgggtccgcctggctccaggcaaggggctagagtgggtggccactatatcatatgatggaagtcagaagtacttcgcagactccgtgaagggccgatttaccatcttcagagacgaatcggagaacatggtgtatctgcaaatgagcggcctgagagttgaggacacggctgtttatcactgtgcgagagggagtagtggtcattatgaggcttttgatatctggggccaagggacaatggtcaccgtctcttcaggtggaggcggttcaggcggaggtggcagcggcggtggcgggagtcagtctgtgttgacgcagccgccctcagtgtctgcggccccaggacagaaggtcaccatctcctgctctggaagcagctccaacattgggaattggtatgtatcctggtaccagcagctcccaggaacagcccccaaactcctcatttatgacaataataagcgaccctcagggattcctgaccgattctctggctccaagtctggcacgtcagccaccctgggcatcaccggactccagactggggacgaggccgattattactgcggaacatgggatagcagcctgagtgccccttgggtgttcggcggagggaccaaggtcaccgtcctaggcgcggccgcaggtgcaggtggtgattacaaagatgatgacgataaaggtgcagcggcgcatcaccatcatcaccac

SEQ ID NO: 25 - DNA, 876 bp, Artificial
  Full-length nucleotide sequence of NYA-2143
atgaaacacctgtggttcttcctcctgctggtggcagctcccagatgggtgctgagcggagaggtgcagctggtggagtctgggggaggcgtggtccagcctgggaggtccctgacaccctcctgttcagcgtctggattctccatccgtagctatgatatacactgggtccgcctggctccaggcaaggggctagagtgggtggccactatatcatatgatggaagtcagaagtacttcgcagactccgtgaagggccgatttaccatcttcagagacgaatcggagaacatggtgtatctgcaaatgagcggcctgagagttgaggacacggctgtttatcactgtgcgagagggagtagtggtcattatgaggcttttgatatctggggccaagggacaatggtcaccgtctcttcaggtggaggcggttcaggcggaggtggcagcggcggtggcgggagtcagtctgtgttgacgcagccgccctcagtgtctgcggccccaggacagaaggtcaccatctcctgctctggaagcagctccaacattgggaattggtatgtatcctggtaccagcggctcccaggaacagcccccaaactcctcatttatgacaataataagcgaccctcagggattcctgaccgattctctggctccaagtctggcacgtcagccaccctgggcatcaccggactccagactggggacgaggccgattattactgcggaacatgggatagcagcctgagtgccccttgggtgttcggcggagggaccaaggtcaccgtcctaggcgcggccgcaggtgcaggtggtgattacaaagatgatgacgataaaggtgcagcggcgcatcaccatcatcaccac

SEQ ID NO: 26 - protein, 292 aa, Artificial
  Full-length amino acid sequence of NYA-1163
MKHLWFFLLLVAAPRWVLSGEVQLVESGGGVVQPGRSLTPSCSASGFSIRSYDIHWVRLAPGKGLEWVATISYDGSQKYFADSVKGRFTIFRDESENMVYLQMSGLRVEDTAVYHCARGSSGHYEAFDIWGQGTMVTVSSGGGGSGGGGSGGGGSQSVLTQPPSVSAAPGQKVTISCSGSSSNIGNNYVSWYQQLPGTAPKLLIYDNNKRPSGIPDRFSGSKSGTSATLGITGLQTGDEADYYCGTWDSSLSAPWVFGGGTKVTVLGAAAGAGGDYKDDDDKGAAAHHHHHH

SEQ ID NO: 27 - protein, 292 aa, Artificial
  Full-length amino acid sequence of NYA-2023
MKHLWFFLLLVAAPRWVLSGEVQLVESGGGVVQPGRSLTPSCSASGFSIRSYDIHWVRQAPGKGLEWVATISYDGSQKYFADSVKGRFTIFRDESENMVYLQMSGLRVEDTAVYHCARGSSGHYEAFDIWGQGTMVTVSSGGGGSGGGGSGGGGSQSVLTQPPSVSAAPGQKVTISCSGSSSNIGNWYVSWYQQLPGTAPKLLIYDNNKRPSGIPDRFSGSKSGTSATLGITGLQTGDEADYYCGTWDSSLSAPWVFGGGTKVTVLGAAAGAGGDYKDDDDKGAAAHHHHHH

SEQ ID NO: 28 - protein, 292 aa, Artificial
  Full-length amino acid sequence of NYA-2027
MKHLWFFLLLVAAPRWVLSGEVQLVESGGGVVQPGRSLTPSCSASGFSIRSYDIHWVRQAPGKGLEWVATISYDGSQKYFADSVKGRFTIFRDESENMVYLQMSGLRVEDTAVYHCARGSSGHYEAFDIWGQGTMVTVSSGGGGSGGGGSGGGGSQSVLTQPPSVSAAPGQKVTISCSGSSSNIGNNYVSWYQQLPGTAPKLLIYDNNKRPSGIPDRFSGSKSGTSATLGITGLQTGDEADYYCGSWDSSLSAPWVFGGGTKVTVLGAAAGAGGDYKDDDDKGAAAHHHHHH

SEQ ID NO: 29 - protein, 292 aa, Artificial
  Full-length amino acid sequence of NYA-1143
MKHLWFFLLLVAAPRWVLSGEVQLVESGGGVVQPGRSLTPSCSASGFSIRSYDIHWVRLAPGKGLEWVATISYDGSQKYFADSVKGRFTIFRDESENMVYLQMSGLRVEDTAVYHCARGSSGHYEAFDIWGQGTMVTVSSGGGGSGGGGSGGGGSQSVLTQPPSVSAAPGQKVTISCSGSSSNIGNWYVSWYQQLPGTAPKLLIYDNNKRPSGIPDRFSGSKSGTSATLGITGLQTGDEADYYCGTWDSSLSAPWVFGGGTKVTVLGAAAGAGGDYKDDDDKGAAAHHHHHH

SEQ ID NO: 30 - protein, 292 aa, Artificial
  Full-length amino acid sequence of NYA-2143
MKHLWFFLLLVAAPRWVLSGEVQLVESGGGVVQPGRSLTPSCSASGFSIRSYDIHWVRLAPGKGLEWVATISYDGSQKYFADSVKGRFTIFRDESENMVYLQMSGLRVEDTAVYHCARGSSGHYEAFDIWGQGTMVTVSSGGGGSGGGGSGGGGSQSVLTQPPSVSAAPGQKVTISCSGSSSNIGNWYVSWYQRLPGTAPKLLIYDNNKRPSGIPDRFSGSKSGTSATLGITGLQTGDEADYYCGTWDSSLSAPWVFGGGTKVTVLGAAAGAGGDYKDDDDKGAAAHHHHHH

SEQ ID NO: 31 - DNA, 876 bp, Artificial
  Full-length nucleotide sequence of NYA-1154
atgaaacacctgtggttcttcctcctgctggtggcagctcccagatgggtgctgagcggagaggtgcagctggtggagtctgggggaggcgtggtccagcctgggaggtccctgacaccctcctgttcagcgtctggattctccatccgtagttatgatatgcactgggtccgccaggctccaggcaaggggctagagtgggtggccactatatcatatgatggaagtcagaagtacttcgcagactccgtgaagggccgatttaccatcttcagagacgaatcggagaacatggtgtatctgcaaatgagcggcctgagagttgaggacacggccgtttatcactgtgcgagagggagtagtaatcattatgaggcttttgatatctggggccaagggacaatggtcaccgtctcttcaggtggaggcggttcaggcggaggtggcagcggcggtggcgggagtcagtctgtgttgacgcagccgccctcagtgtctgcggccccaggacagaaggtcaccatctcctgctctggaagcagctccaacattgggaataattatgtatcctggtaccagcggctcccaggaacagcccccaaactcctcatttatgacaataataagcgaccctcagggattcctgaccgattctctggctccaagtctggcacgtcagccaccctgggcatcaccggactccagactggggacgaggccgattactactgcggagcatgggatagcagcctgagtgccccttgggtgttcggcggagggaccaaggtcaccgtcctaggcgcggccgcaggtgcaggtggtgattacaaagatgatgacgataaaggtgcagcggcgcatcaccatcatcaccac

SEQ ID NO: 32 - protein, 292 aa, Artificial
  Full-length amino acid sequence of NYA-1154
MKHLWFFLLLVAAPRWVLSGEVQLVESGGGVVQPGRSLTPSCSASGFSIRSYDMHWVRQAPGKGLEWVATISYDGSQKYFADSVKGRFTIFRDESENMVYLQMSGLRVEDTAVYHCARGSSNHYEAFDIWGQGTMVTVSSGGGGSGGGGSGGGGSQSVLTQPPSVSAAPGQKVTISCSGSSSNIGNNYVSWYQRLPGTAPKLLIYDNNKRPSGIPDRFSGSKSGTSATLGITGLQTGDEADYYCGAWDSSLSAPWVFGGGTKVTVLGAAAGAGGDYKDDDDKGAAAHHHHHH

SEQ ID NO: 33 - protein, 290 aa, Artificial
  Amino acid sequence of truncated form of HLA-A*0201(UniProtKB-P01892)
MSHSMRYFFTSVSRPGRGEPRFIAVGYVDDTQFVRFDSDAASQRMEPRAPWIEQEGPEYWDGETRKVKAHSQTHRVDLGTLRGYYNQSEAGSHTVQRMYGCDVGSDWRFLRGYHQYAYDGKDYIALKEDLRSWTAADMAAQTTKHKWEAAHVAEQLRAYLEGTCVEWLRRYLENGKETLQRTDAPKTHMTHHAVSDHEATLRCWALSFYPAEITLTWQRDGEDQTQDTELVETRPAGDGTFQKWAAVVVPSGQEQRYTCHVQHEGLPKPLTLRWEGLNDIFEAQKIEWHE

SEQ ID NO: 34 - protein, 100 aa, Artificial [sequence omitted]

SEQ ID NO: 35 - DNA, 876 bp, Artificial
  Full-length nucleotide sequence of NYA-2035
atgaaacacctgtggttcttcctcctgctggtggcagctcccagatgggtgctgagcggagaggtgcagctggtggagtctgggggaggcgtggtccagcctgggaggtccctgacaccctcctgttcagcgtctggattctccatccgtagctatgatatacactgggtccgcctggctccaggcaaggggctagagtgggtggccactatatcatatgatggaagtcagaagtacttcgcagactccgtgaagggccgatttaccatcttcagagacgaatcggagaacatggtgtatctgcaaatgagcggcctgagagttgaggacacggctgtttatcactgtgcgagagggagtagtggtcattatgaggcttttgatatctggggccaagggacaatggtcaccgtctcttcaggtggaggcggttcaggcggaggtggcagcggcggtggcgggagtcagtctgtgttgacgcagccgccctcagtgtctgcggccccaggacagaaggtcaccatctcctgctctggaagcagctccaacattgggaattggaaggtatcctggtaccagcagctcccaggaacagcccccaaactcctcatttatgacaataataagcgaccctcagggattcctgaccgattctctggctccaagtctggcacgtcagccaccctgggcatcaccggactccagactggggacgaggccgattattactgcggaacatgggatagcagcctgagtgccccttgggtgttcggcggagggaccaaggtcaccgtcctaggcgcggccgcaggtgcaggtggtgattacaaagatgatgacgataaaggtgcagcggcgcatcaccatcatcaccac

SEQ ID NO: 36 - protein, 292 aa, Artificial
  Full-length amino acid sequence of NYA-2035
MKHLWFFLLLVAAPRWVLSGEVQLVESGGGVVQPGRSLTPSCSASGFSIRSYDIHWVRLAPGKGLEWVATISYDGSQKYFADSVKGRFTIFRDESENMVYLQMSGLRVEDTAVYHCARGSSGHYEAFDIWGQGTMVTVSSGGGGSGGGGSGGGGSQSVLTQPPSVSAAPGQKVTISCSGSSSNIGNWKVSWYQQLPGTAPKLLIYDNNKRPSGIPDRFSGSKSGTSATLGITGLQTGDEADYYCGTWDSSLSAPWVFGGGTKVTVLGAAAGAGGDYKDDDDKGAAAHHHHHH

SEQ ID NO: 37 - protein, 120 aa, Artificial
  Amino acid sequence of NYA-1143-VH01
EVQLVESGGGLVQPGGSLRLSCAASGFSIRSYDIHWVRLAPGKGLEWVATISYDGSQKYYADSVKGRFTISRDESKNTLYLQMNSLRAEDTAVYHCARGSSGHYEAFDIWGQGTLVTVSS

SEQ ID NO: 38 - protein, 120 aa, Artificial
  Amino acid sequence of NYA-1143-VH02
QVQLVESGGGVVQPGRSLRLSCAASGFSIRSYDMHWVRQAPGKGLEWVATISYDGSQKYYADSVKGRFTISRDNSKNTLYLQMSSLRAEDTAVYHCARGSSGHYEAFDIWGQGTLVTVSS

SEQ ID NO: 39 - protein, 120 aa, Artificial
  Amino acid sequence of NYA-1143-VH03
EVQLVESGGGLVQPGGSLRLSCAASGFSIRSYDIHWVRQAPGKGLEWVATISYDGSQKYYADSVKGRFTISRDESKNTLYLQMNSLRAEDTAVYHCARGSSGHYEAFDIWGQGTLVTVSS

SEQ ID NO: 40 - protein, 111 aa, Artificial
  Amino acid sequence of NYA-1143-VL01
QSVLTQPPSASGTPGQRVTISCSGSSSNIGNWYVSWYQQLPGTAPKLLIYDNNKRPSGVPDRFSGSKSGTSASLAISGLQSEDEADYYCGTWDSSLSAPWVFGGGTKLTVL

SEQ ID NO: 41 - DNA, 876 bp, Artificial
  Full-length nucleotide sequence of NYA-2044
atgaaacacctgtggttcttcctcctgctggtggcagctcccagatgggtgctgagcggtgaggtacagctggtggaatccggtggaggccttgtgcaaccgggaggctccctgcgactctcttgcgccgcatctggcttttccatacgatcctacgatattcattgggtccgactcgcccctggcaaaggtcttgaatgggttgccactatctcctacgacgggtctcagaaatattatgcggattcagtgaaggggcggttcacaatttcacgagacgagtcaaagaatacactgtacctccaaatgaattcactgagagccgaggatactgcagtctatcattgtgcaagagggtcctcaggccactacgaggcctttgatatatggggccaaggcaccttggtaaccgttagtagcggaggtggaggaagcggaggcggcggttccggaggaggtggaagtcaatccgttctgactcagccaccctccgtgagtgcagcgcctggacagaaggtcacaatatcatgttctggctcttcaagcaacatcggaaactggtacgtgagctggtaccagcagctccccggcacggcgcccaagcttctgatatatgacaacaacaaacggcccagtggaatccctgacagattcagtgggtctaaaagtggtacaagcgctaccctgggtatcaccggattgcagaccggagatgaggcggactattattgcggaacctgggactccagcctgagcgctccctgggttttcggcggaggtactaaggttaccgtcttgggcgcggccgcaggtgcaggtggtgattacaaagatgatgacgataaaggtgcagcggcgcatcaccatcatcaccac

SEQ ID NO: 42 - DNA, 876 bp, Artificial
  Full-length nucleotide sequence of NYA-2045
atgaaacacctgtggttcttcctcctgctggtggcagctcccagatgggtgctgagcggtgaggtacagctggtggaatccggtggaggccttgtgcaaccgggaggctccctgcgactctcttgcgccgcatctggcttttccatacgatcctacgatattcattgggtccgactcgcccctggcaaaggtcttgaatgggttgccactatctcctacgacgggtctcagaaatattatgcggattcagtgaaggggcggttcacaatttcacgagacgagtcaaagaatacactgtacctccaaatgaattcactgagagccgaggatactgcagtctatcattgtgcaagagggtcctcaggccactacgaggcctttgatatatggggccaaggcaccttggtaaccgttagtagcggaggtggaggaagcggaggcggcggttccggaggaggtggaagtcaatccgttctgactcagccaccctccgcctctggcaccccgggccaacgggtcacaatatcatgttctggctcttcaagcaacatcggaaactggtacgtgagctggtaccagcagctccccggcacggcgcccaagcttctgatatatgacaacaacaaacggcccagtggagttcctgacagattcagtgggtctaaaagtggtacaagcgctagcctggccataagtggtctgcagagtgaagatgaggcggactattattgcggaacctgggactccagcctgagcgctccctgggttttcggcggaggtactaagctgaccgtcttgggcgcggccgcaggtgcaggtggtgattacaaagatgatgacgataaaggtgcagcggcgcatcaccatcatcaccac

SEQ ID NO: 43 - DNA, 876 bp, Artificial
  Full-length nucleotide sequence of NYA-2047
atgaaacacctgtggttcttcctcctgctggtggcagctcccagatgggtgctgagcggtcaagtacagctggtggaatccggtggaggcgtggtccagccgggacgcagcttgagactgtcctgcgctgcatctggcttttccatacgatcctacgatatgcactgggttcgccaagcccctggcaaaggtcttgaatgggttgccactatctcctacgacgggtctcagaaatattacgcggattcagtgaaggggcggttcacaatttcacgggacaattcaaagaataccttgtatctccagatgtcttcactgagagccgaggatactgcagtctatcattgtgcaagagggtcctcaggccactacgaggcctttgatatatggggccaaggcaccttggtaaccgttagtagcggaggtggaggaagcggaggcggcggttccggaggaggtggaagtcaatccgttctgactcagccaccctccgtgagtgcagcgcctggacagaaggtcacaatatcatgttctggctcttcaagcaacatcggaaactggtacgtgagctggtaccagcagctccccggcacggcgcccaagcttctgatatatgacaacaacaaacggcccagtggaatccctgacagattcagtgggtctaaaagtggtacaagcgctaccctgggtatcaccggattgcagaccggagatgaggcggactattattgcggaacctgggactccagcctgagcgctccctgggttttcggcggaggtactaaggttaccgtcttgggcgcggccgcaggtgcaggtggtgattacaaagatgatgacgataaaggtgcagcggcgcatcaccatcatcaccac

SEQ ID NO: 44 - DNA, 876 bp, Artificial
  Full-length nucleotide sequence of NYA-2048
atgaaacacctgtggttcttcctcctgctggtggcagctcccagatgggtgctgagcggacaagttcaactcgtggaatctggtggaggggtggtacaaccaggccggtcacttagactgtcctgcgctgcgagtggattttccatcagatcttacgacatgcactgggttcgccaagcacccggaaagggtttggaatgggtggctacgatctcctacgatggatcccagaagtattacgccgacagcgtcaagggccgatttacaatatcacgggacaattcaaagaataccttgtatctccagatgtcttcactgagagccgaggatactgcagtctatcattgtgcaagagggtcctcaggccactacgaggcctttgatatatggggccaaggcaccttggtaaccgttagtagcggaggtggaggaagcggaggcggcggttccggaggaggtggaagtcaatccgttctgactcagccaccctccgcctctggcaccccgggccaacgggtcacaatatcatgttctggctcttcaagcaacatcggaaactggtacgtgagctggtaccagcagctccccggcacggcgcccaagcttctgatatatgacaacaacaaacggcccagtggagttcctgacagattcagtgggtctaaaagtggtacaagcgctagcctggccataagtggtctgcagagtgaagatgaggcggactattattgcggaacctgggactccagcctgagcgctccctgggttttcggcggaggtactaagctgaccgtcttgggcgcggccgcaggtgcaggtggtgattacaaagatgatgacgataaaggtgcagcggcgcatcaccatcatcaccac

SEQ ID NO: 45 - DNA, 876 bp, Artificial
  Full-length nucleotide sequence of NYA-2060
atgaaacacctgtggttcttcctcctgctggtggcagctcccagatgggtgctgagcggtgaggtacagctggtggaatccggtggaggccttgtgcaaccgggaggctccctgcgactctcttgcgccgcatctggcttttccatacgatcctacgatattcattgggtccgacaagcccctggcaaaggtcttgaatgggttgccactatctcctacgacgggtctcagaaatattatgcggattcagtgaaggggcggttcacaatttcacgagacgagtcaaagaatacactgtacctccaaatgaattcactgagagccgaggatactgcagtctatcattgtgcaagagggtcctcaggccactacgaggcctttgatatatggggccaaggcaccttggtaaccgttagtagcggaggtggaggaagcggaggcggcggttccggaggaggtggaagtcaatccgttctgactcagccaccctccgtgagtgcagcgcctggacagaaggtcacaatatcatgttctggctcttcaagcaacatcggaaactggtacgtgagctggtaccagcagctccccggcacggcgcccaagcttctgatatatgacaacaacaaacggcccagtggaatccctgacagattcagtgggtctaaaagtggtacaagcgctaccctgggtatcaccggattgcagaccggagatgaggcggactattattgcggaacctgggactccagcctgagcgctccctgggttttcggcggaggtactaaggttaccgtcttgggcgcggccgcaggtgcaggtggtgattacaaagatgatgacgataaaggtgcagcggcgcatcaccatcatcaccac

SEQ ID NO: 46 - DNA, 876 bp, Artificial
  Full-length nucleotide sequence of NYA-2061
atgaaacacctgtggttcttcctcctgctggtggcagctcccagatgggtgctgagcggtgaggtacagctggtggaatccggtggaggccttgtgcaaccgggaggctccctgcgactctcttgcgccgcatctggcttttccatacgatcctacgatattcattgggtccgacaagcccctggcaaaggtcttgaatgggttgccactatctcctacgacgggtctcagaaatattatgcggattcagtgaaggggcggttcacaatttcacgagacgagtcaaagaatacactgtacctccaaatgaattcactgagagccgaggatactgcagtctatcattgtgcaagagggtcctcaggccactacgaggcctttgatatatggggccaaggcaccttggtaaccgttagtagcggaggtggaggaagcggaggcggcggttccggaggaggtggaagtcaatccgttctgactcagccaccctccgcctctggcaccccgggccaacgggtcacaatatcatgttctggctcttcaagcaacatcggaaactggtacgtgagctggtaccagcagctccccggcacggcgcccaagcttctgatatatgacaacaacaaacggcccagtggagttcctgacagattcagtgggtctaaaagtggtacaagcgctagcctggccataagtggtctgcagagtgaagatgaggcggactattattgcggaacctgggactccagcctgagcgctccctgggttttcggcggaggtactaagctgaccgtcttgggcgcggccgcaggtgcaggtggtgattacaaagatgatgacgataaaggtgcagcggcgcatcaccatcatcaccac

SEQ ID NO: 47 - protein, 292 aa, Artificial
  Full-length amino acid sequence of NYA-2044
MKHLWFFLLLVAAPRWVLSGEVQLVESGGGLVQPGGSLRLSCAASGFSIRSYDIHWVRLAPGKGLEWVATISYDGSQKYYADSVKGRFTISRDESKNTLYLQMNSLRAEDTAVYHCARGSSGHYEAFDIWGQGTLVTVSSGGGGSGGGGSGGGGSQSVLTQPPSVSAAPGQKVTISCSGSSSNIGNWYVSWYQQLPGTAPKLLIYDNNKRPSGIPDRFSGSKSGTSATLGITGLQTGDEADYYCGTWDSSLSAPWVFGGGTKVTVLGAAAGAGGDYKDDDDKGAAAHHHHHH

SEQ ID NO: 48 - protein, 292 aa, Artificial
  Full-length amino acid sequence of NYA-2045
MKHLWFFLLLVAAPRWVLSGEVQLVESGGGLVQPGGSLRLSCAASGFSIRSYDIHWVRLAPGKGLEWVATISYDGSQKYYADSVKGRFTISRDESKNTLYLQMNSLRAEDTAVYHCARGSSGHYEAFDIWGQGTLVTVSSGGGGSGGGGSGGGGSQSVLTQPPSASGTPGQRVTISCSGSSSNIGNWYVSWYQQLPGTAPKLLIYDNNKRPSGVPDRFSGSKSGTSASLAISGLQSEDEADYYCGTWDSSLSAPWVFGGGTKLTVLGAAAGAGGDYKDDDDKGAAAHHHHHH

SEQ ID NO: 49 - protein, 246 aa, Artificial
  Full-length amino acid sequence of NYA-0082
EVQLVESGGGVVQPGRSLTPSCSASGFSIRSYDIHWVRQAPGKGLEWVATISYDGSQKYFADSVKGRFTIFRDESENMVYLQMSGLRVEDTAVYHCARGSSGHYEAFDIWGQGTMVTVSSGGGGSGGGGSGGGGSQSVLTQPPSVSAAPGQKVTISCSGSSSNIGNNYVSWYQRLPGTAPKLLIYDNNKRPSGIPDRFSGSKSGTSATLGITGLQTGDEADYYCGSWDSSLSAPWVFGGGTKVTVL

SEQ ID NO: 50 - protein, 292 aa, Artificial
  Full-length amino acid sequence of NYA-2047
MKHLWFFLLLVAAPRWVLSGQVQLVESGGGVVQPGRSLRLSCAASGFSIRSYDMHWVRQAPGKGLEWVATISYDGSQKYYADSVKGRFTISRDNSKNTLYLQMSSLRAEDTAVYHCARGSSGHYEAFDIWGQGTLVTVSSGGGGSGGGGSGGGGSQSVLTQPPSVSAAPGQKVTISCSGSSSNIGNWYVSWYQQLPGTAPKLLIYDNNKRPSGIPDRFSGSKSGTSATLGITGLQTGDEADYYCGTWDSSLSAPWVFGGGTKVTVLGAAAGAGGDYKDDDDKGAAAHHHHHH

SEQ ID NO: 51 - protein, 292 aa, Artificial
  Full-length amino acid sequence of NYA-2048
MKHLWFFLLLVAAPRWVLSGQVQLVESGGGVVQPGRSLRLSCAASGFSIRSYDMHWVRQAPGKGLEWVATISYDGSQKYYADSVKGRFTISRDNSKNTLYLQMSSLRAEDTAVYHCARGSSGHYEAFDIWGQGTLVTVSSGGGGSGGGGSGGGGSQSVLTQPPSASGTPGQRVTISCSGSSSNIGNWYVSWYQQLPGTAPKLLIYDNNKRPSGVPDRFSGSKSGTSASLAISGLQSEDEADYYCGTWDSSLSAPWVFGGGTKLTVLGAAAGAGGDYKDDDDKGAAAHHHHHH

SEQ ID NO: 52 - protein, 292 aa, Artificial
  Full-length amino acid sequence of NYA-2060
MKHLWFFLLLVAAPRWVLSGEVQLVESGGGLVQPGGSLRLSCAASGFSIRSYDIHWVRQAPGKGLEWVATISYDGSQKYYADSVKGRFTISRDESKNTLYLQMNSLRAEDTAVYHCARGSSGHYEAFDIWGQGTLVTVSSGGGGSGGGGSGGGGSQSVLTQPPSVSAAPGQKVTISCSGSSSNIGNWYVSWYQQLPGTAPKLLIYDNNKRPSGIPDRFSGSKSGTSATLGITGLQTGDEADYYCGTWDSSLSAPWVFGGGTKVTVLGAAAGAGGDYKDDDDKGAAAHHHHHH

SEQ ID NO: 53 - protein, 292 aa, Artificial
  Full-length amino acid sequence of NYA-2061
MKHLWFFLLLVAAPRWVLSGEVQLVESGGGLVQPGGSLRLSCAASGFSIRSYDIHWVRQAPGKGLEWVATISYDGSQKYYADSVKGRFTISRDESKNTLYLQMNSLRAEDTAVYHCARGSSGHYEAFDIWGQGTLVTVSSGGGGSGGGGSGGGGSQSVLTQPPSASGTPGQRVTISCSGSSSNIGNWYVSWYQQLPGTAPKLLIYDNNKRPSGVPDRFSGSKSGTSASLAISGLQSEDEADYYCGTWDSSLSAPWVFGGGTKLTVLGAAAGAGGDYKDDDDKGAAAHHHHHH

SEQ ID NO: 54 - protein, 8 aa, Artificial
  Amino acid sequence of NYA-0001-CDRH1
GFSIRSYD

SEQ ID NO: 55 - protein, 8 aa, Artificial
  Amino acid sequence of NYA-0001-CDRH2
ISYDGSQK

SEQ ID NO: 56 - protein, 13 aa, Artificial
  Amino acid sequence of NYA-0001-CDRH3
ARGSSGHYEAFDI

SEQ ID NO: 57 - protein, 8 aa, Artificial
  Amino acid sequence of NYA-0001-CDRL1
SSNIGNNY

SEQ ID NO: 58 - protein, 3 aa, Artificial
  Amino acid sequence of NYA-0001-CDRL2
DNN

SEQ ID NO: 59 - protein, 12 aa, Artificial
  Amino acid sequence of NYA-0001-CDRL3
GTWDSSLSAPWV

SEQ ID NO: 60 - protein, 8 aa, Artificial
  Amino acid sequence of NYA-2023-CDRL1
SSNIGNWY

SEQ ID NO: 61 - protein, 12 aa, Artificial
  Amino acid sequence of NYA-2027-CDRL3
GSWDSSLSAPWV

SEQ ID NO: 62 - protein, 13 aa, Artificial
  Amino acid sequence of NYA-1154-CDRH3
ARGSSNHYEAFDI

SEQ ID NO: 63 - protein, 12 aa, Artificial
  Amino acid sequence of NYA-1154-CDRL3
GAWDSSLSAPWV

SEQ ID NO: 64 - protein, 8 aa, Artificial
  Amino acid sequence of NYA-0035-CDRL1
SSNIGNWK

SEQ ID NO: 65 - DNA, 867 bp, Artificial
  Full-length nucleotide sequence of NYC-0003
atgaaacacctgtggttcttcctcctgctggtggcagctcccagatgggtgctgagcggcgaagtccagctgttggagtcaggtggcggattggtgcaacctggcgggtcactgaggctgagttgtgcagctagcggcttcacattctctacgtatcagatgagctgggtgagacaggctccaggaaagggtctggaatgggtcagcgggattgtgtctagcggtggctccactgcctatgccgatagcgtaaaaggccgctttacgatctctcgggacaactctaagaacacactctatctgcagatgaattcccttagagccgaagataccgccgtgtactactgtgctggggaactgctcccgtattacggtatggacgtttggggccaaggcaccactgtcacagtgagttccggtggaggcgggtcaggcggaggcggtagtggaggtggaggatcacaaagcgagctgacacagcctaggtccgtatccggaagtccagggcagagcgtcaccatcagctgcactggcacctctcgagatgtcggcggatacaactacgtgtcttggtatcagcagcatcccggcaaagcgcccaaactcatcatacacgacgtgattgagcggtccagtggggttcccgatcgtttcagcgggtcaaagtccggaaataccgcaagcctgaccatttctgggcttcaggcagaggatgaggctgactactactgctggtcctttgccgggagctattacgtgtttgggacagggactgacgtgactgttctgggcgcggccgcaggtgcaggtggtgattacaaagatgatgacgataaaggtgcagcggcgcatcaccatcatcaccac

SEQ ID NO: 66 - DNA, 867 bp, Artificial
  Full-length nucleotide sequence of NYC-0004
atgaaacacctgtggttcttcctcctgctggtggcagctcccagatgggtgctgagcggcgaagtccagctgttggagtcaggtggcggattggtgcaacctggcgggtcactgaggctgagttgtgcagctagcggcttcacattctctacgtatcagatgagctgggtgagacaggctccaggaaagggtctggaatgggtcagcgggattgtgtctagcggtggctccactgcctatgccgatagcgtaaaaggccgctttacgatctctcgggacaactctaagaacacactctatctgcagatgaattcccttagagccgaagataccgccgtgtactactgtgctggggaactgctcccgtattacggtatggacgtttggggccaaggcaccactgtcacagtgagttccggtggaggcgggtcaggcggaggcggtagtggaggtggaggatcacaaagcgagctgacacagcctaggtccgtatccggaagtccagggcagagcgtcaccatcagctgcactggcaccgagcgagatgtcggcggatacaactacgtgtcttggtatcagcagcatcccggcaaagcgcccaaactcatcatacacgacgtgattgagcggtccagtggggttcccgatcgtttcagcgggtcaaagtccggaaataccgcaagcctgaccatttctgggcttcaggcagaggatgaggctgactactactgctggtcctttgccgggggctattacgtgtttgggacagggactgacgtgactgttctgggcgcggccgcaggtgcaggtggtgattacaaagatgatgacgataaaggtgcagcggcgcatcaccatcatcaccac

SEQ ID NO: 67 - protein, 289 aa, Artificial
  Full-length amino acid sequence of NYC-0003
MKHLWFFLLLVAAPRWVLSGEVQLLESGGGLVQPGGSLRLSCAASGFTFSTYQMSWVRQAPGKGLEWVSGIVSSGGSTAYADSVKGRFTISRDNSKNTLYLQMNSLRAEDTAVYYCAGELLPYYGMDVWGQGTTVTVSSGGGGSGGGGSGGGGSQSELTQPRSVSGSPGQSVTISCTGTSRDVGGYNYVSWYQQHPGKAPKLIIHDVIERSSGVPDRFSGSKSGNTASLTISGLQAEDEADYYCWSFAGSYYVFGTGTDVTVLGAAAGAGGDYKDDDDKGAAAHHHHHH

SEQ ID NO: 68 - protein, 289 aa, Artificial
  Full-length amino acid sequence of NYC-0004
MKHLWFFLLLVAAPRWVLSGEVQLLESGGGLVQPGGSLRLSCAASGFTFSTYQMSWVRQAPGKGLEWVSGIVSSGGSTAYADSVKGRFTISRDNSKNTLYLQMNSLRAEDTAVYYCAGELLPYYGMDVWGQGTTVTVSSGGGGSGGGGSGGGGSQSELTQPRSVSGSPGQSVTISCTGTERDVGGYNYVSWYQQHPGKAPKLIIHDVIERSSGVPDRFSGSKSGNTASLTISGLQAEDEADYYCWSFAGGYYVFGTGTDVTVLGAAAGAGGDYKDDDDKGAAAHHHHHH

SEQ ID NO: 69 - DNA, 876 bp, Artificial
  Full-length nucleotide sequence of NYA-0001
atgaaacacctgtggttcttcctcctgctggtggcagctcccagatgggtgctgagcggagaggtgcagctggtggagtctgggggaggcgtggtccagcctgggaggtccctgacaccctcctgttcagcgtctggattctccatccgtagttatgatatacactgggtccgccaggctccaggcaaggggctagagtgggtggccactatatcatatgatggaagtcagaagtacttcgcagactccgtgaagggccgatttaccatcttcagagacgaatcggagaacatggtgtatctgcaaatgagcggcctgagagttgaggacacggctgtttatcactgtgcgagagggagtagtggtcattatgaggcttttgatatctggggccaagggacaatggtcaccgtctcttcaggtggaggcggttcaggcggaggtggcagcggcggtggcgggagtcagtctgtgttgacgcagccgccctcagtgtctgcggccccaggacagaaggtcaccatctcctgctctggaagcagctccaacattgggaataattatgtatcctggtaccagcagctcccaggaacagcccccaaactcctcatttatgacaataataagcgaccctcagggattcctgaccgattctctggctccaagtctggcacgtcagccaccctgggcatcaccggactccagactggggacgaggccgattattactgcggaacatgggatagcagcctgagtgccccttgggtgttcggcggagggaccaaggtcaccgtcctaggcgcggccgcaggtgcaggtggtgattacaaagatgatgacgataaaggtgcagcggcgcatcaccatcatcaccac

SEQ ID NO: 70 - protein, 292 aa, Artificial
  Full-length amino acid sequence of NYA-0001
MKHLWFFLLLVAAPRWVLSGEVQLVESGGGVVQPGRSLTPSCSASGFSIRSYDIHWVRQAPGKGLEWVATISYDGSQKYFADSVKGRFTIFRDESENMVYLQMSGLRVEDTAVYHCARGSSGHYEAFDIWGQGTMVTVSSGGGGSGGGGSGGGGSQSVLTQPPSVSAAPGQKVTISCSGSSSNIGNNYVSWYQQLPGTAPKLLIYDNNKRPSGIPDRFSGSKSGTSATLGITGLQTGDEADYYCGTWDSSLSAPWVFGGGTKVTVLGAAAGAGGDYKDDDDKGAAAHHHHHH

SEQ ID NO: 71 - DNA, 738 bp, Artificial
  Full-length nucleotide sequence of HC1
atgaaacacctgtggttcttcctcctgctggtggcagctcccagatgggtgctgagcgacaaaactcacacatgcccaccctgcccagcacctgaagccgcagggggaccctcagtcttcctcttccccccaaaacccaaggacaccctcatgatctcccggacccctgaggtcacatgcgtggtggtgtcagtgagccacgaagaccctgaggtcaagttcaactggtacgtggacggcgtggaggtgcataatgccaagacaaagccccgggaggagcagtacaacagcacgtaccgggtggtcagcgtcctcaccgtcctgcaccaggactggctgaatggcaaggagtacaagtgcaaggtctccaacaaagccctcccagcccccatcgagaaaaccatctccaaagccaaaggccagccccgggaaccacaggtgtacgtgctgcccccatcccgggacgagctgaccaagaaccaggtcagcctgctgtgcctggtcaaaggcttctatcccagcgacatcgccgtggagtgggagagcaatggccagcccgagaacaactacctgacctggcctcccgtgctggactccgacggctccttcttcctctacagcaagctcaccgtggacaagagcaggtggcagcagggcaacgtcttctcatgctccgtgatgcatgaggctctgcacaaccactacacccagaagagcctctccctgtctcccggcaag

SEQ ID NO: 72 - DNA, 2235 bp, Artificial
  Full-length nucleotide sequence of NYF-0016-HC2
atgaaacacctgtggttcttcctcctgctggtggcagctcccagatgggtgctgagcggagaggtgcagctggtggagtctgggggaggcgtggtccagcctgggaggtccctgacaccctcctgttcagcgtctggattctccatccgtagctatgatatacactgggtccgcctggctccaggcaaggggctagagtgggtggccactatatcatatgatggaagtcagaagtacttcgcagactccgtgaagggccgatttaccatcttcagagacgaatcggagaacatggtgtatctgcaaatgagcggcctgagagttgaggacacggctgtttatcactgtgcgagagggagtagtggtcattatgaggcttttgatatctggggccaagggacaatggtcaccgtctcttcaggtggaggcggttcaggcggaggtggcagcggcggtggcgggagtcagtctgtgttgacgcagccgccctcagtgtctgcggccccaggacagaaggtcaccatctcctgctctggaagcagctccaacattgggaattggtatgtatcctggtaccagcagctcccaggaacagcccccaaactcctcatttatgacaataataagcgaccctcagggattcctgaccgattctctggctccaagtctggcacgtcagccaccctgggcatcaccggactccagactggggacgaggccgattattactgcggaacatgggatagcagcctgagtgccccttgggtgttcggcggagggaccaaggtcaccgtcctagggggaggcggttcagaagtgcagctggtggaatccggggggggcctggtgcagcctggggggagcctgagactgagttgtgccgcctctggggtgacatttaactactatggcatgtcttggatccgccaggcacctggaaagggcctggagtgggtggccagcatcactaggtccggcgggcgaatctactatcccgacagcgtcaagggcaggttcacaatttcccgcgagaacacacagaaaactctgtacctgcagatgaatagcctgagagccgaagatacagctgtgtactattgcactctggacggcagggatgggtgggtcgcctattgggggcagggaaccctggtgacagtcagctccggaggaggaggatctggcggaggaggcagtgggggaggcgggtcaaactttatgctcactcagccgtcctctgtttctggcgtacctggccaacgggtgaccattagctgtacgggtaataccgggaatatcgggtctaactacgtgaactggtatcagcagcttccagggacagctcccaagttgctgatctatcgcgacgacaaaagaccctcaggggtccctgaccgatttagtggcagcaaaagcggtacttccgcttccctggcgataaccggctttcaggccgaagatgaggcagactactattgccagtcatattccagcggcttcatcttcggaggcggaactaagctgacagtgttggcagccgagcccaaatcttctgacaaaactcacacatgcccaccctgcccagcacctgaagccgcagggggaccctcagtcttcctcttccccccaaaacccaaggacaccctcatgatctcccggacccctgaggtcacatgcgtggtggtgtcagtgagccacgaagaccctgaggtcaagttcaactggtacgtggacggcgtggaggtgcataatgccaagacaaagccccgggaggagcagtacaacagcacgtaccgggtggtcagcgtcctcaccgtcctgcaccaggactggctgaatggcaaggagtacaagtgcaaggtctccaacaaagccctcccagcccccatcgagaaaaccatctccaaagccaaaggccagccccgggaaccacaggtgtacgtgtaccccccatcccgggacgagctgaccaagaaccaggtcagcctgacctgcctggtcaaaggcttctatcccagcgacatcgccgtggagtgggagagcaatggccagcccgagaacaactacaagaccacccctcccgtgctggactccgacggctccttcgccctcgtgagcaagctcaccgtggacaagagcaggtggcagcagggcaacgtcttctcatgctccgtgatgcatgaggctctgcacaaccactacacccagaagagcctctccctgtctcccggcaag

SEQ ID NO: 73 - DNA, 2235 bp, Artificial
  Full-length nucleotide sequence of NYF-0019-HC2
atgaaacacctgtggttcttcctcctgctggtggcagctcccagatgggtgctgagcggagaggtgcagctggtggagtctgggggaggcgtggtccagcctgggaggtccctgacaccctcctgttcagcgtctggattctccatccgtagctatgatatacactgggtccgcctggctccaggcaaggggctagagtgggtggccactatatcatatgatggaagtcagaagtacttcgcagactccgtgaagggccgatttaccatcttcagagacgaatcggagaacatggtgtatctgcaaatgagcggcctgagagttgaggacacggctgtttatcactgtgcgagagggagtagtggtcattatgaggcttttgatatctggggccaagggacaatggtcaccgtctcttcaggtggaggcggttcaggcggaggtggcagcggcggtggcgggagtcagtctgtgttgacgcagccgccctcagtgtctgcggccccaggacagaaggtcaccatctcctgctctggaagcagctccaacattgggaattggtatgtatcctggtaccagcggctcccaggaacagcccccaaactcctcatttatgacaataataagcgaccctcagggattcctgaccgattctctggctccaagtctggcacgtcagccaccctgggcatcaccggactccagactggggacgaggccgattattactgcggaacatgggatagcagcctgagtgccccttgggtgttcggcggagggaccaaggtcaccgtcctagggggaggcggttcagaagtgcagctggtggaatccggggggggcctggtgcagcctggggggagcctgagactgagttgtgccgcctctggggtgacatttaactactatggcatgtcttggatccgccaggcacctggaaagggcctggagtgggtggccagcatcactaggtccggcgggcgaatctactatcccgacagcgtcaagggcaggttcacaatttcccgcgagaacacacagaaaactctgtacctgcagatgaatagcctgagagccgaagatacagctgtgtactattgcactctggacggcagggatgggtgggtcgcctattgggggcagggaaccctggtgacagtcagctccggaggaggaggatctggcggaggaggcagtgggggaggcgggtcaaactttatgctcactcagccgtcctctgtttctggcgtacctggccaacgggtgaccattagctgtacgggtaataccgggaatatcgggtctaactacgtgaactggtatcagcagcttccagggacagctcccaagttgctgatctatcgcgacgacaaaagaccctcaggggtccctgaccgatttagtggcagcaaaagcggtacttccgcttccctggcgataaccggctttcaggccgaagatgaggcagactactattgccagtcatattccagcggcttcatcttcggaggcggaactaagctgacagtgttggcagccgagcccaaatcttctgacaaaactcacacatgcccaccctgcccagcacctgaagccgcagggggaccctcagtcttcctcttccccccaaaacccaaggacaccctcatgatctcccggacccctgaggtcacatgcgtggtggtgtcagtgagccacgaagaccctgaggtcaagttcaactggtacgtggacggcgtggaggtgcataatgccaagacaaagccccgggaggagcagtacaacagcacgtaccgggtggtcagcgtcctcaccgtcctgcaccaggactggctgaatggcaaggagtacaagtgcaaggtctccaacaaagccctcccagcccccatcgagaaaaccatctccaaagccaaaggccagccccgggaaccacaggtgtacgtgtaccccccatcccgggacgagctgaccaagaaccaggtcagcctgacctgcctggtcaaaggcttctatcccagcgacatcgccgtggagtgggagagcaatggccagcccgagaacaactacaagaccacccctcccgtgctggactccgacggctccttcgccctcgtgagcaagctcaccgtggacaagagcaggtggcagcagggcaacgtcttctcatgctccgtgatgcatgaggctctgcacaaccactacacccagaagagcctctccctgtctcccggcaag

SEQ ID NO: 74 - DNA, 2235 bp, Artificial
  Full-length nucleotide sequence of NYF-0022-HC2
atgaaacacctgtggttcttcctcctgctggtggcagctcccagatgggtgctgagcggagaggtgcagctggtggagtctgggggaggcgtggtccagcctgggaggtccctgacaccctcctgttcagcgtctggattctccatccgtagctatgatatacactgggtccgcctggctccaggcaaggggctagagtgggtggccactatatcatatgatggaagtcagaagtacttcgcagactccgtgaagggccgatttaccatcttcagagacgaatcggagaacatggtgtatctgcaaatgagcggcctgagagttgaggacacggctgtttatcactgtgcgagagggagtagtggtcattatgaggcttttgatatctggggccaagggacaatggtcaccgtctcttcaggtggaggcggttcaggcggaggtggcagcggcggtggcgggagtcagtctgtgttgacgcagccgccctcagtgtctgcggccccaggacagaaggtcaccatctcctgctctggaagcagctccaacattgggaataattatgtatcctggtaccagcagctcccaggaacagcccccaaactcctcatttatgacaataataagcgaccctcagggattcctgaccgattctctggctccaagtctggcacgtcagccaccctgggcatcaccggactccagactggggacgaggccgattattactgcggaacatgggatagcagcctgagtgccccttgggtgttcggcggagggaccaaggtcaccgtcctagggggaggcggttcagaagtgcagctggtggaatccggggggggcctggtgcagcctggggggagcctgagactgagttgtgccgcctctggggtgacatttaactactatggcatgtcttggatccgccaggcacctggaaagggcctggagtgggtggccagcatcactaggtccggcgggcgaatctactatcccgacagcgtcaagggcaggttcacaatttcccgcgagaacacacagaaaactctgtacctgcagatgaatagcctgagagccgaagatacagctgtgtactattgcactctggacggcagggatgggtgggtcgcctattgggggcagggaaccctggtgacagtcagctccggaggaggaggatctggcggaggaggcagtgggggaggcgggtcaaactttatgctcactcagccgtcctctgtttctggcgtacctggccaacgggtgaccattagctgtacgggtaataccgggaatatcgggtctaactacgtgaactggtatcagcagcttccagggacagctcccaagttgctgatctatcgcgacgacaaaagaccctcaggggtccctgaccgatttagtggcagcaaaagcggtacttccgcttccctggcgataaccggctttcaggccgaagatgaggcagactactattgccagtcatattccagcggcttcatcttcggaggcggaactaagctgacagtgttggcagccgagcccaaatcttctgacaaaactcacacatgcccaccctgcccagcacctgaagccgcagggggaccctcagtcttcctcttccccccaaaacccaaggacaccctcatgatctcccggacccctgaggtcacatgcgtggtggtgtcagtgagccacgaagaccctgaggtcaagttcaactggtacgtggacggcgtggaggtgcataatgccaagacaaagccccgggaggagcagtacaacagcacgtaccgggtggtcagcgtcctcaccgtcctgcaccaggactggctgaatggcaaggagtacaagtgcaaggtctccaacaaagccctcccagcccccatcgagaaaaccatctccaaagccaaaggccagccccgggaaccacaggtgtacgtgtaccccccatcccgggacgagctgaccaagaaccaggtcagcctgacctgcctggtcaaaggcttctatcccagcgacatcgccgtggagtgggagagcaatggccagcccgagaacaactacaagaccacccctcccgtgctggactccgacggctccttcgccctcgtgagcaagctcaccgtggacaagagcaggtggcagcagggcaacgtcttctcatgctccgtgatgcatgaggctctgcacaaccactacacccagaagagcctctccctgtctcccggcaag

SEQ ID NO: 75 - DNA, 2235 bp, Artificial
  Full-length nucleotide sequence of NYF-0023-HC2
atgaaacacctgtggttcttcctcctgctggtggcagctcccagatgggtgctgagcggagaggtgcagctggtggagtctgggggaggcgtggtccagcctgggaggtccctgacaccctcctgttcagcgtctggattctccatccgtagttatgatatacactgggtccgccaggctccaggcaaggggctagagtgggtggccactatatcatatgatggaagtcagaagtacttcgcagactccgtgaagggccgatttaccatcttcagagacgaatcggagaacatggtgtatctgcaaatgagcggcctgagagttgaggacacggctgtttatcactgtgcgagagggagtagtggtcattatgaggcttttgatatctggggccaagggacaatggtcaccgtctcttcaggtggaggcggttcaggcggaggtggcagcggcggtggcgggagtcagtctgtgttgacgcagccgccctcagtgtctgcggccccaggacagaaggtcaccatctcctgctctggaagcagctccaacattgggaattggtatgtatcctggtaccagcagctcccaggaacagcccccaaactcctcatttatgacaataataagcgaccctcagggattcctgaccgattctctggctccaagtctggcacgtcagccaccctgggcatcaccggactccagactggggacgaggccgattattactgcggaacatgggatagcagcctgagtgccccttgggtgttcggcggagggaccaaggtcaccgtcctagggggaggcggttcagaagtgcagctggtggaatccggggggggcctggtgcagcctggggggagcctgagactgagttgtgccgcctctggggtgacatttaactactatggcatgtcttggatccgccaggcacctggaaagggcctggagtgggtggccagcatcactaggtccggcgggcgaatctactatcccgacagcgtcaagggcaggttcacaatttcccgcgagaacacacagaaaactctgtacctgcagatgaatagcctgagagccgaagatacagctgtgtactattgcactctggacggcagggatgggtgggtcgcctattgggggcagggaaccctggtgacagtcagctccggaggaggaggatctggcggaggaggcagtgggggaggcgggtcaaactttatgctcactcagccgtcctctgtttctggcgtacctggccaacgggtgaccattagctgtacgggtaataccgggaatatcgggtctaactacgtgaactggtatcagcagcttccagggacagctcccaagttgctgatctatcgcgacgacaaaagaccctcaggggtccctgaccgatttagtggcagcaaaagcggtacttccgcttccctggcgataaccggctttcaggccgaagatgaggcagactactattgccagtcatattccagcggcttcatcttcggaggcggaactaagctgacagtgttggcagccgagcccaaatcttctgacaaaactcacacatgcccaccctgcccagcacctgaagccgcagggggaccctcagtcttcctcttccccccaaaacccaaggacaccctcatgatctcccggacccctgaggtcacatgcgtggtggtgtcagtgagccacgaagaccctgaggtcaagttcaactggtacgtggacggcgtggaggtgcataatgccaagacaaagccccgggaggagcagtacaacagcacgtaccgggtggtcagcgtcctcaccgtcctgcaccaggactggctgaatggcaaggagtacaagtgcaaggtctccaacaaagccctcccagcccccatcgagaaaaccatctccaaagccaaaggccagccccgggaaccacaggtgtacgtgtaccccccatcccgggacgagctgaccaagaaccaggtcagcctgacctgcctggtcaaaggcttctatcccagcgacatcgccgtggagtgggagagcaatggccagcccgagaacaactacaagaccacccctcccgtgctggactccgacggctccttcgccctcgtgagcaagctcaccgtggacaagagcaggtggcagcagggcaacgtcttctcatgctccgtgatgcatgaggctctgcacaaccactacacccagaagagcctctccctgtctcccggcaag

SEQ ID NO: 76 - DNA, 2235 bp, Artificial
  Full-length nucleotide sequence of NYF-0027-HC2
atgaaacacctgtggttcttcctcctgctggtggcagctcccagatgggtgctgagcggagaggtgcagctggtggagtctgggggaggcgtggtccagcctgggaggtccctgacaccctcctgttcagcgtctggattctccatccgtagttatgatatacactgggtccgccaggctccaggcaaggggctagagtgggtggccactatatcatatgatggaagtcagaagtacttcgcagactccgtgaagggccgatttaccatcttcagagacgaatcggagaacatggtgtatctgcaaatgagcggcctgagagttgaggacacggctgtttatcactgtgcgagagggagtagtggtcattatgaggcttttgatatctggggccaagggacaatggtcaccgtctcttcaggtggaggcggttcaggcggaggtggcagcggcggtggcgggagtcagtctgtgttgacgcagccgccctcagtgtctgcggccccaggacagaaggtcaccatctcctgctctggaagcagctccaacattgggaataattatgtatcctggtaccagcagctcccaggaacagcccccaaactcctcatttatgacaataataagcgaccctcagggattcctgaccgattctctggctccaagtctggcacgtcagccaccctgggcatcaccggactccagactggggacgaggccgattattactgcggatcatgggatagcagcctgagtgccccttgggtgttcggcggagggaccaaggtcaccgtcctagggggaggcggttcagaagtgcagctggtggaatccggggggggcctggtgcagcctggggggagcctgagactgagttgtgccgcctctggggtgacatttaactactatggcatgtcttggatccgccaggcacctggaaagggcctggagtgggtggccagcatcactaggtccggcgggcgaatctactatcccgacagcgtcaagggcaggttcacaatttcccgcgagaacacacagaaaactctgtacctgcagatgaatagcctgagagccgaagatacagctgtgtactattgcactctggacggcagggatgggtgggtcgcctattgggggcagggaaccctggtgacagtcagctccggaggaggaggatctggcggaggaggcagtgggggaggcgggtcaaactttatgctcactcagccgtcctctgtttctggcgtacctggccaacgggtgaccattagctgtacgggtaataccgggaatatcgggtctaactacgtgaactggtatcagcagcttccagggacagctcccaagttgctgatctatcgcgacgacaaaagaccctcaggggtccctgaccgatttagtggcagcaaaagcggtacttccgcttccctggcgataaccggctttcaggccgaagatgaggcagactactattgccagtcatattccagcggcttcatcttcggaggcggaactaagctgacagtgttggcagccgagcccaaatcttctgacaaaactcacacatgcccaccctgcccagcacctgaagccgcagggggaccctcagtcttcctcttccccccaaaacccaaggacaccctcatgatctcccggacccctgaggtcacatgcgtggtggtgtcagtgagccacgaagaccctgaggtcaagttcaactggtacgtggacggcgtggaggtgcataatgccaagacaaagccccgggaggagcagtacaacagcacgtaccgggtggtcagcgtcctcaccgtcctgcaccaggactggctgaatggcaaggagtacaagtgcaaggtctccaacaaagccctcccagcccccatcgagaaaaccatctccaaagccaaaggccagccccgggaaccacaggtgtacgtgtaccccccatcccgggacgagctgaccaagaaccaggtcagcctgacctgcctggtcaaaggcttctatcccagcgacatcgccgtggagtgggagagcaatggccagcccgagaacaactacaagaccacccctcccgtgctggactccgacggctccttcgccctcgtgagcaagctcaccgtggacaagagcaggtggcagcagggcaacgtcttctcatgctccgtgatgcatgaggctctgcacaaccactacacccagaagagcctctccctgtctcccggcaag

SEQ ID NO: 77 - DNA, 2235 bp, Artificial
  Full-length nucleotide sequence of NYF-0035-HC2
atgaaacacctgtggttcttcctcctgctggtggcagctcccagatgggtgctgagcggagaggtgcagctggtggagtctgggggaggcgtggtccagcctgggaggtccctgacaccctcctgttcagcgtctggattctccatccgtagctatgatatacactgggtccgcctggctccaggcaaggggctagagtgggtggccactatatcatatgatggaagtcagaagtacttcgcagactccgtgaagggccgatttaccatcttcagagacgaatcggagaacatggtgtatctgcaaatgagcggcctgagagttgaggacacggctgtttatcactgtgcgagagggagtagtggtcattatgaggcttttgatatctggggccaagggacaatggtcaccgtctcttcaggtggaggcggttcaggcggaggtggcagcggcggtggcgggagtcagtctgtgttgacgcagccgccctcagtgtctgcggccccaggacagaaggtcaccatctcctgctctggaagcagctccaacattgggaattggaaggtatcctggtaccagcagctcccaggaacagcccccaaactcctcatttatgacaataataagcgaccctcagggattcctgaccgattctctggctccaagtctggcacgtcagccaccctgggcatcaccggactccagactggggacgaggccgattattactgcggaacatgggatagcagcctgagtgccccttgggtgttcggcggagggaccaaggtcaccgtcctagggggaggcggttcagaagtgcagctggtggaatccggggggggcctggtgcagcctggggggagcctgagactgagttgtgccgcctctggggtgacatttaactactatggcatgtcttggatccgccaggcacctggaaagggcctggagtgggtggccagcatcactaggtccggcgggcgaatctactatcccgacagcgtcaagggcaggttcacaatttcccgcgagaacacacagaaaactctgtacctgcagatgaatagcctgagagccgaagatacagctgtgtactattgcactctggacggcagggatgggtgggtcgcctattgggggcagggaaccctggtgacagtcagctccggaggaggaggatctggcggaggaggcagtgggggaggcgggtcaaactttatgctcactcagccgtcctctgtttctggcgtacctggccaacgggtgaccattagctgtacgggtaataccgggaatatcgggtctaactacgtgaactggtatcagcagcttccagggacagctcccaagttgctgatctatcgcgacgacaaaagaccctcaggggtccctgaccgatttagtggcagcaaaagcggtacttccgcttccctggcgataaccggctttcaggccgaagatgaggcagactactattgccagtcatattccagcggcttcatcttcggaggcggaactaagctgacagtgttggcagccgagcccaaatcttctgacaaaactcacacatgcccaccctgcccagcacctgaagccgcagggggaccctcagtcttcctcttccccccaaaacccaaggacaccctcatgatctcccggacccctgaggtcacatgcgtggtggtgtcagtgagccacgaagaccctgaggtcaagttcaactggtacgtggacggcgtggaggtgcataatgccaagacaaagccccgggaggagcagtacaacagcacgtaccgggtggtcagcgtcctcaccgtcctgcaccaggactggctgaatggcaaggagtacaagtgcaaggtctccaacaaagccctcccagcccccatcgagaaaaccatctccaaagccaaaggccagccccgggaaccacaggtgtacgtgtaccccccatcccgggacgagctgaccaagaaccaggtcagcctgacctgcctggtcaaaggcttctatcccagcgacatcgccgtggagtgggagagcaatggccagcccgagaacaactacaagaccacccctcccgtgctggactccgacggctccttcgccctcgtgagcaagctcaccgtggacaagagcaggtggcagcagggcaacgtcttctcatgctccgtgatgcatgaggctctgcacaaccactacacccagaagagcctctccctgtctcccggcaag

SEQ ID NO: 78 - DNA, 2235 bp, Artificial
  Full-length nucleotide sequence of NYF-0044-HC2
atgaaacacctgtggttcttcctcctgctggtggcagctcccagatgggtgctgagcggtgaggtacagctggtggaatccggtggaggccttgtgcaaccgggaggctccctgcgactctcttgcgccgcatctggcttttccatacgatcctacgatattcattgggtccgactcgcccctggcaaaggtcttgaatgggttgccactatctcctacgacgggtctcagaaatattatgcggattcagtgaaggggcggttcacaatttcacgagacgagtcaaagaatacactgtacctccaaatgaattcactgagagccgaggatactgcagtctatcattgtgcaagagggtcctcaggccactacgaggcctttgatatatggggccaaggcaccttggtaaccgttagtagcggaggtggaggaagcggaggcggcggttccggaggaggtggaagtcaatccgttctgactcagccaccctccgtgagtgcagcgcctggacagaaggtcacaatatcatgttctggctcttcaagcaacatcggaaactggtacgtgagctggtaccagcagctccccggcacggcgcccaagcttctgatatatgacaacaacaaacggcccagtggaatccctgacagattcagtgggtctaaaagtggtacaagcgctaccctgggtatcaccggattgcagaccggagatgaggcggactattattgcggaacctgggactccagcctgagcgctccctgggttttcggcggaggtactaaggttaccgtcttgggaggaggcggttcagaagtgcagctggtggaatccggggggggcctggtgcagcctggggggagcctgagactgagttgtgccgcctctggggtgacatttaactactatggcatgtcttggatccgccaggcacctggaaagggcctggagtgggtggccagcatcactaggtccggcgggcgaatctactatcccgacagcgtcaagggcaggttcacaatttcccgcgagaacacacagaaaactctgtacctgcagatgaatagcctgagagccgaagatacagctgtgtactattgcactctggacggcagggatgggtgggtcgcctattgggggcagggaaccctggtgacagtcagctccggaggaggaggatctggcggaggaggcagtgggggaggcgggtcaaactttatgctcactcagccgtcctctgtttctggcgtacctggccaacgggtgaccattagctgtacgggtaataccgggaatatcgggtctaactacgtgaactggtatcagcagcttccagggacagctcccaagttgctgatctatcgcgacgacaaaagaccctcaggggtccctgaccgatttagtggcagcaaaagcggtacttccgcttccctggcgataaccggctttcaggccgaagatgaggcagactactattgccagtcatattccagcggcttcatcttcggaggcggaactaagctgacagtgttggcagccgagcccaaatcttctgacaaaactcacacatgcccaccctgcccagcacctgaagccgcagggggaccctcagtcttcctcttccccccaaaacccaaggacaccctcatgatctcccggacccctgaggtcacatgcgtggtggtgtcagtgagccacgaagaccctgaggtcaagttcaactggtacgtggacggcgtggaggtgcataatgccaagacaaagccccgggaggagcagtacaacagcacgtaccgggtggtcagcgtcctcaccgtcctgcaccaggactggctgaatggcaaggagtacaagtgcaaggtctccaacaaagccctcccagcccccatcgagaaaaccatctccaaagccaaaggccagccccgggaaccacaggtgtacgtgtaccccccatcccgggacgagctgaccaagaaccaggtcagcctgacctgcctggtcaaaggcttctatcccagcgacatcgccgtggagtgggagagcaatggccagcccgagaacaactacaagaccacccctcccgtgctggactccgacggctccttcgccctcgtgagcaagctcaccgtggacaagagcaggtggcagcagggcaacgtcttctcatgctccgtgatgcatgaggctctgcacaaccactacacccagaagagcctctccctgtctcccggcaag

SEQ ID NO: 79 - DNA, 2235 bp, Artificial
  Full-length nucleotide sequence of NYF-0045-HC2
atgaaacacctgtggttcttcctcctgctggtggcagctcccagatgggtgctgagcggtgaggtacagctggtggaatccggtggaggccttgtgcaaccgggaggctccctgcgactctcttgcgccgcatctggcttttccatacgatcctacgatattcattgggtccgactcgcccctggcaaaggtcttgaatgggttgccactatctcctacgacgggtctcagaaatattatgcggattcagtgaaggggcggttcacaatttcacgagacgagtcaaagaatacactgtacctccaaatgaattcactgagagccgaggatactgcagtctatcattgtgcaagagggtcctcaggccactacgaggcctttgatatatggggccaaggcaccttggtaaccgttagtagcggaggtggaggaagcggaggcggcggttccggaggaggtggaagtcaatccgttctgactcagccaccctccgcctctggcaccccgggccaacgggtcacaatatcatgttctggctcttcaagcaacatcggaaactggtacgtgagctggtaccagcagctccccggcacggcgcccaagcttctgatatatgacaacaacaaacggcccagtggagttcctgacagattcagtgggtctaaaagtggtacaagcgctagcctggccataagtggtctgcagagtgaagatgaggcggactattattgcggaacctgggactccagcctgagcgctccctgggttttcggcggaggtactaagctgaccgtcttgggaggaggcggttcagaagtgcagctggtggaatccggggggggcctggtgcagcctggggggagcctgagactgagttgtgccgcctctggggtgacatttaactactatggcatgtcttggatccgccaggcacctggaaagggcctggagtgggtggccagcatcactaggtccggcgggcgaatctactatcccgacagcgtcaagggcaggttcacaatttcccgcgagaacacacagaaaactctgtacctgcagatgaatagcctgagagccgaagatacagctgtgtactattgcactctggacggcagggatgggtgggtcgcctattgggggcagggaaccctggtgacagtcagctccggaggaggaggatctggcggaggaggcagtgggggaggcgggtcaaactttatgctcactcagccgtcctctgtttctggcgtacctggccaacgggtgaccattagctgtacgggtaataccgggaatatcgggtctaactacgtgaactggtatcagcagcttccagggacagctcccaagttgctgatctatcgcgacgacaaaagaccctcaggggtccctgaccgatttagtggcagcaaaagcggtacttccgcttccctggcgataaccggctttcaggccgaagatgaggcagactactattgccagtcatattccagcggcttcatcttcggaggcggaactaagctgacagtgttggcagccgagcccaaatcttctgacaaaactcacacatgcccaccctgcccagcacctgaagccgcagggggaccctcagtcttcctcttccccccaaaacccaaggacaccctcatgatctcccggacccctgaggtcacatgcgtggtggtgtcagtgagccacgaagaccctgaggtcaagttcaactggtacgtggacggcgtggaggtgcataatgccaagacaaagccccgggaggagcagtacaacagcacgtaccgggtggtcagcgtcctcaccgtcctgcaccaggactggctgaatggcaaggagtacaagtgcaaggtctccaacaaagccctcccagcccccatcgagaaaaccatctccaaagccaaaggccagccccgggaaccacaggtgtacgtgtaccccccatcccgggacgagctgaccaagaaccaggtcagcctgacctgcctggtcaaaggcttctatcccagcgacatcgccgtggagtgggagagcaatggccagcccgagaacaactacaagaccacccctcccgtgctggactccgacggctccttcgccctcgtgagcaagctcaccgtggacaagagcaggtggcagcagggcaacgtcttctcatgctccgtgatgcatgaggctctgcacaaccactacacccagaagagcctctccctgtctcccggcaag

SEQ ID NO: 80 - DNA, 2235 bp, Artificial
  Full-length nucleotide sequence of NYF-0047-HC2
atgaaacacctgtggttcttcctcctgctggtggcagctcccagatgggtgctgagcggtcaagtacagctggtggaatccggtggaggcgtggtccagccgggacgcagcttgagactgtcctgcgctgcatctggcttttccatacgatcctacgatatgcactgggttcgccaagcccctggcaaaggtcttgaatgggttgccactatctcctacgacgggtctcagaaatattacgcggattcagtgaaggggcggttcacaatttcacgggacaattcaaagaataccttgtatctccagatgtcttcactgagagccgaggatactgcagtctatcattgtgcaagagggtcctcaggccactacgaggcctttgatatatggggccaaggcaccttggtaaccgttagtagcggaggtggaggaagcggaggcggcggttccggaggaggtggaagtcaatccgttctgactcagccaccctccgtgagtgcagcgcctggacagaaggtcacaatatcatgttctggctcttcaagcaacatcggaaactggtacgtgagctggtaccagcagctccccggcacggcgcccaagcttctgatatatgacaacaacaaacggcccagtggaatccctgacagattcagtgggtctaaaagtggtacaagcgctaccctgggtatcaccggattgcagaccggagatgaggcggactattattgcggaacctgggactccagcctgagcgctccctgggttttcggcggaggtactaaggttaccgtcttgggaggaggcggttcagaagtgcagctggtggaatccggggggggcctggtgcagcctggggggagcctgagactgagttgtgccgcctctggggtgacatttaactactatggcatgtcttggatccgccaggcacctggaaagggcctggagtgggtggccagcatcactaggtccggcgggcgaatctactatcccgacagcgtcaagggcaggttcacaatttcccgcgagaacacacagaaaactctgtacctgcagatgaatagcctgagagccgaagatacagctgtgtactattgcactctggacggcagggatgggtgggtcgcctattgggggcagggaaccctggtgacagtcagctccggaggaggaggatctggcggaggaggcagtgggggaggcgggtcaaactttatgctcactcagccgtcctctgtttctggcgtacctggccaacgggtgaccattagctgtacgggtaataccgggaatatcgggtctaactacgtgaactggtatcagcagcttccagggacagctcccaagttgctgatctatcgcgacgacaaaagaccctcaggggtccctgaccgatttagtggcagcaaaagcggtacttccgcttccctggcgataaccggctttcaggccgaagatgaggcagactactattgccagtcatattccagcggcttcatcttcggaggcggaactaagctgacagtgttggcagccgagcccaaatcttctgacaaaactcacacatgcccaccctgcccagcacctgaagccgcagggggaccctcagtcttcctcttccccccaaaacccaaggacaccctcatgatctcccggacccctgaggtcacatgcgtggtggtgtcagtgagccacgaagaccctgaggtcaagttcaactggtacgtggacggcgtggaggtgcataatgccaagacaaagccccgggaggagcagtacaacagcacgtaccgggtggtcagcgtcctcaccgtcctgcaccaggactggctgaatggcaaggagtacaagtgcaaggtctccaacaaagccctcccagcccccatcgagaaaaccatctccaaagccaaaggccagccccgggaaccacaggtgtacgtgtaccccccatcccgggacgagctgaccaagaaccaggtcagcctgacctgcctggtcaaaggcttctatcccagcgacatcgccgtggagtgggagagcaatggccagcccgagaacaactacaagaccacccctcccgtgctggactccgacggctccttcgccctcgtgagcaagctcaccgtggacaagagcaggtggcagcagggcaacgtcttctcatgctccgtgatgcatgaggctctgcacaaccactacacccagaagagcctctccctgtctcccggcaag

SEQ ID NO: 81 - DNA, 2235 bp, Artificial
  Full-length nucleotide sequence of NYF-0048-HC2
atgaaacacctgtggttcttcctcctgctggtggcagctcccagatgggtgctgagcggacaagttcaactcgtggaatctggtggaggggtggtacaaccaggccggtcacttagactgtcctgcgctgcgagtggattttccatcagatcttacgacatgcactgggttcgccaagcacccggaaagggtttggaatgggtggctacgatctcctacgatggatcccagaagtattacgccgacagcgtcaagggccgatttacaatatcacgggacaattcaaagaataccttgtatctccagatgtcttcactgagagccgaggatactgcagtctatcattgtgcaagagggtcctcaggccactacgaggcctttgatatatggggccaaggcaccttggtaaccgttagtagcggaggtggaggaagcggaggcggcggttccggaggaggtggaagtcaatccgttctgactcagccaccctccgcctctggcaccccgggccaacgggtcacaatatcatgttctggctcttcaagcaacatcggaaactggtacgtgagctggtaccagcagctccccggcacggcgcccaagcttctgatatatgacaacaacaaacggcccagtggagttcctgacagattcagtgggtctaaaagtggtacaagcgctagcctggccataagtggtctgcagagtgaagatgaggcggactattattgcggaacctgggactccagcctgagcgctccctgggttttcggcggaggtactaagctgaccgtcttgggaggaggcggttcagaagtgcagctggtggaatccggggggggcctggtgcagcctggggggagcctgagactgagttgtgccgcctctggggtgacatttaactactatggcatgtcttggatccgccaggcacctggaaagggcctggagtgggtggccagcatcactaggtccggcgggcgaatctactatcccgacagcgtcaagggcaggttcacaatttcccgcgagaacacacagaaaactctgtacctgcagatgaatagcctgagagccgaagatacagctgtgtactattgcactctggacggcagggatgggtgggtcgcctattgggggcagggaaccctggtgacagtcagctccggaggaggaggatctggcggaggaggcagtgggggaggcgggtcaaactttatgctcactcagccgtcctctgtttctggcgtacctggccaacgggtgaccattagctgtacgggtaataccgggaatatcgggtctaactacgtgaactggtatcagcagcttccagggacagctcccaagttgctgatctatcgcgacgacaaaagaccctcaggggtccctgaccgatttagtggcagcaaaagcggtacttccgcttccctggcgataaccggctttcaggccgaagatgaggcagactactattgccagtcatattccagcggcttcatcttcggaggcggaactaagctgacagtgttggcagccgagcccaaatcttctgacaaaactcacacatgcccaccctgcccagcacctgaagccgcagggggaccctcagtcttcctcttccccccaaaacccaaggacaccctcatgatctcccggacccctgaggtcacatgcgtggtggtgtcagtgagccacgaagaccctgaggtcaagttcaactggtacgtggacggcgtggaggtgcataatgccaagacaaagccccgggaggagcagtacaacagcacgtaccgggtggtcagcgtcctcaccgtcctgcaccaggactggctgaatggcaaggagtacaagtgcaaggtctccaacaaagccctcccagcccccatcgagaaaaccatctccaaagccaaaggccagccccgggaaccacaggtgtacgtgtaccccccatcccgggacgagctgaccaagaaccaggtcagcctgacctgcctggtcaaaggcttctatcccagcgacatcgccgtggagtgggagagcaatggccagcccgagaacaactacaagaccacccctcccgtgctggactccgacggctccttcgccctcgtgagcaagctcaccgtggacaagagcaggtggcagcagggcaacgtcttctcatgctccgtgatgcatgaggctctgcacaaccactacacccagaagagcctctccctgtctcccggcaag

SEQ ID NO: 82 - DNA, 2235 bp, Artificial
  Full-length nucleotide sequence of NYF-0060-HC2
atgaaacacctgtggttcttcctcctgctggtggcagctcccagatgggtgctgagcggtgaggtacagctggtggaatccggtggaggccttgtgcaaccgggaggctccctgcgactctcttgcgccgcatctggcttttccatacgatcctacgatattcattgggtccgacaagcccctggcaaaggtcttgaatgggttgccactatctcctacgacgggtctcagaaatattatgcggattcagtgaaggggcggttcacaatttcacgagacgagtcaaagaatacactgtacctccaaatgaattcactgagagccgaggatactgcagtctatcattgtgcaagagggtcctcaggccactacgaggcctttgatatatggggccaaggcaccttggtaaccgttagtagcggaggtggaggaagcggaggcggcggttccggaggaggtggaagtcaatccgttctgactcagccaccctccgtgagtgcagcgcctggacagaaggtcacaatatcatgttctggctcttcaagcaacatcggaaactggtacgtgagctggtaccagcagctccccggcacggcgcccaagcttctgatatatgacaacaacaaacggcccagtggaatccctgacagattcagtgggtctaaaagtggtacaagcgctaccctgggtatcaccggattgcagaccggagatgaggcggactattattgcggaacctgggactccagcctgagcgctccctgggttttcggcggaggtactaaggttaccgtcttgggaggaggcggttcagaagtgcagctggtggaatccggggggggcctggtgcagcctggggggagcctgagactgagttgtgccgcctctggggtgacatttaactactatggcatgtcttggatccgccaggcacctggaaagggcctggagtgggtggccagcatcactaggtccggcgggcgaatctactatcccgacagcgtcaagggcaggttcacaatttcccgcgagaacacacagaaaactctgtacctgcagatgaatagcctgagagccgaagatacagctgtgtactattgcactctggacggcagggatgggtgggtcgcctattgggggcagggaaccctggtgacagtcagctccggaggaggaggatctggcggaggaggcagtgggggaggcgggtcaaactttatgctcactcagccgtcctctgtttctggcgtacctggccaacgggtgaccattagctgtacgggtaataccgggaatatcgggtctaactacgtgaactggtatcagcagcttccagggacagctcccaagttgctgatctatcgcgacgacaaaagaccctcaggggtccctgaccgatttagtggcagcaaaagcggtacttccgcttccctggcgataaccggctttcaggccgaagatgaggcagactactattgccagtcatattccagcggcttcatcttcggaggcggaactaagctgacagtgttggcagccgagcccaaatcttctgacaaaactcacacatgcccaccctgcccagcacctgaagccgcagggggaccctcagtcttcctcttccccccaaaacccaaggacaccctcatgatctcccggacccctgaggtcacatgcgtggtggtgtcagtgagccacgaagaccctgaggtcaagttcaactggtacgtggacggcgtggaggtgcataatgccaagacaaagccccgggaggagcagtacaacagcacgtaccgggtggtcagcgtcctcaccgtcctgcaccaggactggctgaatggcaaggagtacaagtgcaaggtctccaacaaagccctcccagcccccatcgagaaaaccatctccaaagccaaaggccagccccgggaaccacaggtgtacgtgtaccccccatcccgggacgagctgaccaagaaccaggtcagcctgacctgcctggtcaaaggcttctatcccagcgacatcgccgtggagtgggagagcaatggccagcccgagaacaactacaagaccacccctcccgtgctggactccgacggctccttcgccctcgtgagcaagctcaccgtggacaagagcaggtggcagcagggcaacgtcttctcatgctccgtgatgcatgaggctctgcacaaccactacacccagaagagcctctccctgtctcccggcaag

SEQ ID NO: 83 - DNA, 2235 bp, Artificial
  Full-length nucleotide sequence of NYF-0061-HC2
atgaaacacctgtggttcttcctcctgctggtggcagctcccagatgggtgctgagcggtgaggtacagctggtggaatccggtggaggccttgtgcaaccgggaggctccctgcgactctcttgcgccgcatctggcttttccatacgatcctacgatattcattgggtccgacaagcccctggcaaaggtcttgaatgggttgccactatctcctacgacgggtctcagaaatattatgcggattcagtgaaggggcggttcacaatttcacgagacgagtcaaagaatacactgtacctccaaatgaattcactgagagccgaggatactgcagtctatcattgtgcaagagggtcctcaggccactacgaggcctttgatatatggggccaaggcaccttggtaaccgttagtagcggaggtggaggaagcggaggcggcggttccggaggaggtggaagtcaatccgttctgactcagccaccctccgcctctggcaccccgggccaacgggtcacaatatcatgttctggctcttcaagcaacatcggaaactggtacgtgagctggtaccagcagctccccggcacggcgcccaagcttctgatatatgacaacaacaaacggcccagtggagttcctgacagattcagtgggtctaaaagtggtacaagcgctagcctggccataagtggtctgcagagtgaagatgaggcggactattattgcggaacctgggactccagcctgagcgctccctgggttttcggcggaggtactaagctgaccgtcttgggaggaggcggttcagaagtgcagctggtggaatccggggggggcctggtgcagcctggggggagcctgagactgagttgtgccgcctctggggtgacatttaactactatggcatgtcttggatccgccaggcacctggaaagggcctggagtgggtggccagcatcactaggtccggcgggcgaatctactatcccgacagcgtcaagggcaggttcacaatttcccgcgagaacacacagaaaactctgtacctgcagatgaatagcctgagagccgaagatacagctgtgtactattgcactctggacggcagggatgggtgggtcgcctattgggggcagggaaccctggtgacagtcagctccggaggaggaggatctggcggaggaggcagtgggggaggcgggtcaaactttatgctcactcagccgtcctctgtttctggcgtacctggccaacgggtgaccattagctgtacgggtaataccgggaatatcgggtctaactacgtgaactggtatcagcagcttccagggacagctcccaagttgctgatctatcgcgacgacaaaagaccctcaggggtccctgaccgatttagtggcagcaaaagcggtacttccgcttccctggcgataaccggctttcaggccgaagatgaggcagactactattgccagtcatattccagcggcttcatcttcggaggcggaactaagctgacagtgttggcagccgagcccaaatcttctgacaaaactcacacatgcccaccctgcccagcacctgaagccgcagggggaccctcagtcttcctcttccccccaaaacccaaggacaccctcatgatctcccggacccctgaggtcacatgcgtggtggtgtcagtgagccacgaagaccctgaggtcaagttcaactggtacgtggacggcgtggaggtgcataatgccaagacaaagccccgggaggagcagtacaacagcacgtaccgggtggtcagcgtcctcaccgtcctgcaccaggactggctgaatggcaaggagtacaagtgcaaggtctccaacaaagccctcccagcccccatcgagaaaaccatctccaaagccaaaggccagccccgggaaccacaggtgtacgtgtaccccccatcccgggacgagctgaccaagaaccaggtcagcctgacctgcctggtcaaaggcttctatcccagcgacatcgccgtggagtgggagagcaatggccagcccgagaacaactacaagaccacccctcccgtgctggactccgacggctccttcgccctcgtgagcaagctcaccgtggacaagagcaggtggcagcagggcaacgtcttctcatgctccgtgatgcatgaggctctgcacaaccactacacccagaagagcctctccctgtctcccggcaag

SEQ ID NO: 84 - protein, 246 aa, Artificial
  Full-length amino acid sequence of HC1
MKHLWFFLLLVAAPRWVLSDKTHTCPPCPAPEAAGGPSVFLFPPKPKDTLMISRTPEVTCVVVSVSHEDPEVKFNWYVDGVEVHNAKTKPREEQYNSTYRVVSVLTVLHQDWLNGKEYKCKVSNKALPAPIEKTISKAKGQPREPQVYVLPPSRDELTKNQVSLLCLVKGFYPSDIAVEWESNGQPENNYLTWPPVLDSDGSFFLYSKLTVDKSRWQQGNVFSCSVMHEALHNHYTQKSLSLSPGK

SEQ ID NO: 85 - protein, 745 aa, Artificial
  Full-length amino acid sequence of NYF-0016-HC
MKHLWFFLLLVAAPRWVLSGEVQLVESGGGVVQPGRSLTPSCSASGFSIRSYDIHWVRLAPGKGLEWVATISYDGSQKYFADSVKGRFTIFRDESENMVYLQMSGLRVEDTAVYHCARGSSGHYEAFDIWGQGTMVTVSSGGGGSGGGGSGGGGSQSVLTQPPSVSAAPGQKVTISCSGSSSNIGNWYVSWYQQLPGTAPKLLIYDNNKRPSGIPDRFSGSKSGTSATLGITGLQTGDEADYYCGTWDSSLSAPWVFGGGTKVTVLGGGGSEVQLVESGGGLVQPGGSLRLSCAASGVTFNYYGMSWIRQAPGKGLEWVASITRSGGRIYYPDSVKGRFTISRENTQKTLYLQMNSLRAEDTAVYYCTLDGRDGWVAYWGQGTLVTVSSGGGGSGGGGSGGGGSNFMLTQPSSVSGVPGQRVTISCTGNTGNIGSNYVNWYQQLPGTAPKLLIYRDDKRPSGVPDRFSGSKSGTSASLAITGFQAEDEADYYCQSYSSGFIFGGGTKLTVLAAEPKSSDKTHTCPPCPAPEAAGGPSVFLFPPKPKDTLMISRTPEVTCVVVSVSHEDPEVKFNWYVDGVEVHNAKTKPREEQYNSTYRVVSVLTVLHQDWLNGKEYKCKVSNKALPAPIEKTISKAKGQPREPQVYVYPPSRDELTKNQVSLTCLVKGFYPSDIAVEWESNGQPENNYKTTPPVLDSDGSFALVSKLTVDKSRWQQGNVFSCSVMHEALHNHYTQKSLSLSPGK

SEQ ID NO: 86 - protein, 745 aa, Artificial
  Full-length amino acid sequence of NYF-0019-HC2
MKHLWFFLLLVAAPRWVLSGEVQLVESGGGVVQPGRSLTPSCSASGFSIRSYDIHWVRLAPGKGLEWVATISYDGSQKYFADSVKGRFTIFRDESENMVYLQMSGLRVEDTAVYHCARGSSGHYEAFDIWGQGTMVTVSSGGGGSGGGGSGGGGSQSVLTQPPSVSAAPGQKVTISCSGSSSNIGNWYVSWYQRLPGTAPKLLIYDNNKRPSGIPDRFSGSKSGTSATLGITGLQTGDEADYYCGTWDSSLSAPWVFGGGTKVTVLGGGGSEVQLVESGGGLVQPGGSLRLSCAASGVTFNYYGMSWIRQAPGKGLEWVASITRSGGRIYYPDSVKGRFTISRENTQKTLYLQMNSLRAEDTAVYYCTLDGRDGWVAYWGQGTLVTVSSGGGGSGGGGSGGGGSNFMLTQPSSVSGVPGQRVTISCTGNTGNIGSNYVNWYQQLPGTAPKLLIYRDDKRPSGVPDRFSGSKSGTSASLAITGFQAEDEADYYCQSYSSGFIFGGGTKLTVLAAEPKSSDKTHTCPPCPAPEAAGGPSVFLFPPKPKDTLMISRTPEVTCVVVSVSHEDPEVKFNWYVDGVEVHNAKTKPREEQYNSTYRVVSVLTVLHQDWLNGKEYKCKVSNKALPAPIEKTISKAKGQPREPQVYVYPPSRDELTKNQVSLTCLVKGFYPSDIAVEWESNGQPENNYKTTPPVLDSDGSFALVSKLTVDKSRWQQGNVFSCSVMHEALHNHYTQKSLSLSPGK

SEQ ID NO: 87 - protein, 745 aa, Artificial
  Full-length amino acid sequence of NYF-0022-HC2
MKHLWFFLLLVAAPRWVLSGEVQLVESGGGVVQPGRSLTPSCSASGFSIRSYDIHWVRLAPGKGLEWVATISYDGSQKYFADSVKGRFTIFRDESENMVYLQMSGLRVEDTAVYHCARGSSGHYEAFDIWGQGTMVTVSSGGGGSGGGGSGGGGSQSVLTQPPSVSAAPGQKVTISCSGSSSNIGNNYVSWYQQLPGTAPKLLIYDNNKRPSGIPDRFSGSKSGTSATLGITGLQTGDEADYYCGTWDSSLSAPWVFGGGTKVTVLGGGGSEVQLVESGGGLVQPGGSLRLSCAASGVTFNYYGMSWIRQAPGKGLEWVASITRSGGRIYYPDSVKGRFTISRENTQKTLYLQMNSLRAEDTAVYYCTLDGRDGWVAYWGQGTLVTVSSGGGGSGGGGSGGGGSNFMLTQPSSVSGVPGQRVTISCTGNTGNIGSNYVNWYQQLPGTAPKLLIYRDDKRPSGVPDRFSGSKSGTSASLAITGFQAEDEADYYCQSYSSGFIFGGGTKLTVLAAEPKSSDKTHTCPPCPAPEAAGGPSVFLFPPKPKDTLMISRTPEVTCVVVSVSHEDPEVKFNWYVDGVEVHNAKTKPREEQYNSTYRVVSVLTVLHQDWLNGKEYKCKVSNKALPAPIEKTISKAKGQPREPQVYVYPPSRDELTKNQVSLTCLVKGFYPSDIAVEWESNGQPENNYKTTPPVLDSDGSFALVSKLTVDKSRWQQGNVFSCSVMHEALHNHYTQKSLSLSPGK

SEQ ID NO: 88 - protein, 745 aa, Artificial
  Full-length amino acid sequence of NYF-0023-HC2
MKHLWFFLLLVAAPRWVLSGEVQLVESGGGVVQPGRSLTPSCSASGFSIRSYDIHWVRQAPGKGLEWVATISYDGSQKYFADSVKGRFTIFRDESENMVYLQMSGLRVEDTAVYHCARGSSGHYEAFDIWGQGTMVTVSSGGGGSGGGGSGGGGSQSVLTQPPSVSAAPGQKVTISCSGSSSNIGNWYVSWYQQLPGTAPKLLIYDNNKRPSGIPDRFSGSKSGTSATLGITGLQTGDEADYYCGTWDSSLSAPWVFGGGTKVTVLGGGGSEVQLVESGGGLVQPGGSLRLSCAASGVTFNYYGMSWIRQAPGKGLEWVASITRSGGRIYYPDSVKGRFTISRENTQKTLYLQMNSLRAEDTAVYYCTLDGRDGWVAYWGQGTLVTVSSGGGGSGGGGSGGGGSNFMLTQPSSVSGVPGQRVTISCTGNTGNIGSNYVNWYQQLPGTAPKLLIYRDDKRPSGVPDRFSGSKSGTSASLAITGFQAEDEADYYCQSYSSGFIFGGGTKLTVLAAEPKSSDKTHTCPPCPAPEAAGGPSVFLFPPKPKDTLMISRTPEVTCVVVSVSHEDPEVKFNWYVDGVEVHNAKTKPREEQYNSTYRVVSVLTVLHQDWLNGKEYKCKVSNKALPAPIEKTISKAKGQPREPQVYVYPPSRDELTKNQVSLTCLVKGFYPSDIAVEWESNGQPENNYKTTPPVLDSDGSFALVSKLTVDKSRWQQGNVFSCSVMHEALHNHYTQKSLSLSPGK

SEQ ID NO: 89 - protein, 745 aa, Artificial
  Full-length amino acid sequence of NYF-0027-HC2
MKHLWFFLLLVAAPRWVLSGEVQLVESGGGVVQPGRSLTPSCSASGFSIRSYDIHWVRQAPGKGLEWVATISYDGSQKYFADSVKGRFTIFRDESENMVYLQMSGLRVEDTAVYHCARGSSGHYEAFDIWGQGTMVTVSSGGGGSGGGGSGGGGSQSVLTQPPSVSAAPGQKVTISCSGSSSNIGNNYVSWYQQLPGTAPKLLIYDNNKRPSGIPDRFSGSKSGTSATLGITGLQTGDEADYYCGSWDSSLSAPWVFGGGTKVTVLGGGGSEVQLVESGGGLVQPGGSLRLSCAASGVTFNYYGMSWIRQAPGKGLEWVASITRSGGRIYYPDSVKGRFTISRENTQKTLYLQMNSLRAEDTAVYYCTLDGRDGWVAYWGQGTLVTVSSGGGGSGGGGSGGGGSNFMLTQPSSVSGVPGQRVTISCTGNTGNIGSNYVNWYQQLPGTAPKLLIYRDDKRPSGVPDRFSGSKSGTSASLAITGFQAEDEADYYCQSYSSGFIFGGGTKLTVLAAEPKSSDKTHTCPPCPAPEAAGGPSVFLFPPKPKDTLMISRTPEVTCVVVSVSHEDPEVKFNWYVDGVEVHNAKTKPREEQYNSTYRVVSVLTVLHQDWLNGKEYKCKVSNKALPAPIEKTISKAKGQPREPQVYVYPPSRDELTKNQVSLTCLVKGFYPSDIAVEWESNGQPENNYKTTPPVLDSDGSFALVSKLTVDKSRWQQGNVFSCSVMHEALHNHYTQKSLSLSPGK

SEQ ID NO: 90 - protein, 745 aa, Artificial
  Full-length amino acid sequence of NYF-0035-HC2
MKHLWFFLLLVAAPRWVLSGEVQLVESGGGVVQPGRSLTPSCSASGFSIRSYDIHWVRLAPGKGLEWVATISYDGSQKYFADSVKGRFTIFRDESENMVYLQMSGLRVEDTAVYHCARGSSGHYEAFDIWGQGTMVTVSSGGGGSGGGGSGGGGSQSVLTQPPSVSAAPGQKVTISCSGSSSNIGNWKVSWYQQLPGTAPKLLIYDNNKRPSGIPDRFSGSKSGTSATLGITGLQTGDEADYYCGTWDSSLSAPWVFGGGTKVTVLGGGGSEVQLVESGGGLVQPGGSLRLSCAASGVTFNYYGMSWIRQAPGKGLEWVASITRSGGRIYYPDSVKGRFTISRENTQKTLYLQMNSLRAEDTAVYYCTLDGRDGWVAYWGQGTLVTVSSGGGGSGGGGSGGGGSNFMLTQPSSVSGVPGQRVTISCTGNTGNIGSNYVNWYQQLPGTAPKLLIYRDDKRPSGVPDRFSGSKSGTSASLAITGFQAEDEADYYCQSYSSGFIFGGGTKLTVLAAEPKSSDKTHTCPPCPAPEAAGGPSVFLFPPKPKDTLMISRTPEVTCVVVSVSHEDPEVKFNWYVDGVEVHNAKTKPREEQYNSTYRVVSVLTVLHQDWLNGKEYKCKVSNKALPAPIEKTISKAKGQPREPQVYVYPPSRDELTKNQVSLTCLVKGFYPSDIAVEWESNGQPENNYKTTPPVLDSDGSFALVSKLTVDKSRWQQGNVFSCSVMHEALHNHYTQKSLSLSPGK

SEQ ID NO: 91 - protein, 745 aa, Artificial
  Full-length amino acid sequence of NYF-0044-HC2
MKHLWFFLLLVAAPRWVLSGEVQLVESGGGLVQPGGSLRLSCAASGFSIRSYDIHWVRLAPGKGLEWVATISYDGSQKYYADSVKGRFTISRDESKNTLYLQMNSLRAEDTAVYHCARGSSGHYEAFDIWGQGTLVTVSSGGGGSGGGGSGGGGSQSVLTQPPSVSAAPGQKVTISCSGSSSNIGNWYVSWYQQLPGTAPKLLIYDNNKRPSGIPDRFSGSKSGTSATLGITGLQTGDEADYYCGTWDSSLSAPWVFGGGTKVTVLGGGGSEVQLVESGGGLVQPGGSLRLSCAASGVTFNYYGMSWIRQAPGKGLEWVASITRSGGRIYYPDSVKGRFTISRENTQKTLYLQMNSLRAEDTAVYYCTLDGRDGWVAYWGQGTLVTVSSGGGGSGGGGSGGGGSNFMLTQPSSVSGVPGQRVTISCTGNTGNIGSNYVNWYQQLPGTAPKLLIYRDDKRPSGVPDRFSGSKSGTSASLAITGFQAEDEADYYCQSYSSGFIFGGGTKLTVLAAEPKSSDKTHTCPPCPAPEAAGGPSVFLFPPKPKDTLMISRTPEVTCVVVSVSHEDPEVKFNWYVDGVEVHNAKTKPREEQYNSTYRVVSVLTVLHQDWLNGKEYKCKVSNKALPAPIEKTISKAKGQPREPQVYVYPPSRDELTKNQVSLTCLVKGFYPSDIAVEWESNGQPENNYKTTPPVLDSDGSFALVSKLTVDKSRWQQGNVFSCSVMHEALHNHYTQKSLSLSPGK

SEQ ID NO: 92 - protein, 745 aa, Artificial
  Full-length amino acid sequence of NYF-0045-HC2
MKHLWFFLLLVAAPRWVLSGEVQLVESGGGLVQPGGSLRLSCAASGFSIRSYDIHWVRLAPGKGLEWVATISYDGSQKYYADSVKGRFTISRDESKNTLYLQMNSLRAEDTAVYHCARGSSGHYEAFDIWGQGTLVTVSSGGGGSGGGGSGGGGSQSVLTQPPSASGTPGQRVTISCSGSSSNIGNWYVSWYQQLPGTAPKLLIYDNNKRPSGVPDRFSGSKSGTSASLAISGLQSEDEADYYCGTWDSSLSAPWVFGGGTKLTVLGGGGSEVQLVESGGGLVQPGGSLRLSCAASGVTFNYYGMSWIRQAPGKGLEWVASITRSGGRIYYPDSVKGRFTISRENTQKTLYLQMNSLRAEDTAVYYCTLDGRDGWVAYWGQGTLVTVSSGGGGSGGGGSGGGGSNFMLTQPSSVSGVPGQRVTISCTGNTGNIGSNYVNWYQQLPGTAPKLLIYRDDKRPSGVPDRFSGSKSGTSASLAITGFQAEDEADYYCQSYSSGFIFGGGTKLTVLAAEPKSSDKTHTCPPCPAPEAAGGPSVFLFPPKPKDTLMISRTPEVTCVVVSVSHEDPEVKFNWYVDGVEVHNAKTKPREEQYNSTYRVVSVLTVLHQDWLNGKEYKCKVSNKALPAPIEKTISKAKGQPREPQVYVYPPSRDELTKNQVSLTCLVKGFYPSDIAVEWESNGQPENNYKTTPPVLDSDGSFALVSKLTVDKSRWQQGNVFSCSVMHEALHNHYTQKSLSLSPGK

SEQ ID NO: 93 - protein, 745 aa, Artificial
  Full-length amino acid sequence of NYF-0047-HC2
MKHLWFFLLLVAAPRWVLSGQVQLVESGGGVVQPGRSLRLSCAASGFSIRSYDMHWVRQAPGKGLEWVATISYDGSQKYYADSVKGRFTISRDNSKNTLYLQMSSLRAEDTAVYHCARGSSGHYEAFDIWGQGTLVTVSSGGGGSGGGGSGGGGSQSVLTQPPSVSAAPGQKVTISCSGSSSNIGNWYVSWYQQLPGTAPKLLIYDNNKRPSGIPDRFSGSKSGTSATLGITGLQTGDEADYYCGTWDSSLSAPWVFGGGTKVTVLGGGGSEVQLVESGGGLVQPGGSLRLSCAASGVTFNYYGMSWIRQAPGKGLEWVASITRSGGRIYYPDSVKGRFTISRENTQKTLYLQMNSLRAEDTAVYYCTLDGRDGWVAYWGQGTLVTVSSGGGGSGGGGSGGGGSNFMLTQPSSVSGVPGQRVTISCTGNTGNIGSNYVNWYQQLPGTAPKLLIYRDDKRPSGVPDRFSGSKSGTSASLAITGFQAEDEADYYCQSYSSGFIFGGGTKLTVLAAEPKSSDKTHTCPPCPAPEAAGGPSVFLFPPKPKDTLMISRTPEVTCVVVSVSHEDPEVKFNWYVDGVEVHNAKTKPREEQYNSTYRVVSVLTVLHQDWLNGKEYKCKVSNKALPAPIEKTISKAKGQPREPQVYVYPPSRDELTKNQVSLTCLVKGFYPSDIAVEWESNGQPENNYKTTPPVLDSDGSFALVSKLTVDKSRWQQGNVFSCSVMHEALHNHYTQKSLSLSPGK

SEQ ID NO: 94 - protein, 745 aa, Artificial
  Full-length amino acid sequence of NYF-0048-HC2
MKHLWFFLLLVAAPRWVLSGQVQLVESGGGVVQPGRSLRLSCAASGFSIRSYDMHWVRQAPGKGLEWVATISYDGSQKYYADSVKGRFTISRDNSKNTLYLQMSSLRAEDTAVYHCARGSSGHYEAFDIWGQGTLVTVSSGGGGSGGGGSGGGGSQSVLTQPPSASGTPGQRVTISCSGSSSNIGNWYVSWYQQLPGTAPKLLIYDNNKRPSGVPDRFSGSKSGTSASLAISGLQSEDEADYYCGTWDSSLSAPWVFGGGTKLTVLGGGGSEVQLVESGGGLVQPGGSLRLSCAASGVTFNYYGMSWIRQAPGKGLEWVASITRSGGRIYYPDSVKGRFTISRENTQKTLYLQMNSLRAEDTAVYYCTLDGRDGWVAYWGQGTLVTVSSGGGGSGGGGSGGGGSNFMLTQPSSVSGVPGQRVTISCTGNTGNIGSNYVNWYQQLPGTAPKLLIYRDDKRPSGVPDRFSGSKSGTSASLAITGFQAEDEADYYCQSYSSGFIFGGGTKLTVLAAEPKSSDKTHTCPPCPAPEAAGGPSVFLFPPKPKDTLMISRTPEVTCVVVSVSHEDPEVKFNWYVDGVEVHNAKTKPREEQYNSTYRVVSVLTVLHQDWLNGKEYKCKVSNKALPAPIEKTISKAKGQPREPQVYVYPPSRDELTKNQVSLTCLVKGFYPSDIAVEWESNGQPENNYKTTPPVLDSDGSFALVSKLTVDKSRWQQGNVFSCSVMHEALHNHYTQKSLSLSPGK

SEQ ID NO: 95 - protein, 745 aa, Artificial
  Full-length amino acid sequence of NYF-0060-HC2
MKHLWFFLLLVAAPRWVLSGEVQLVESGGGLVQPGGSLRLSCAASGFSIRSYDIHWVRQAPGKGLEWVATISYDGSQKYYADSVKGRFTISRDESKNTLYLQMNSLRAEDTAVYHCARGSSGHYEAFDIWGQGTLVTVSSGGGGSGGGGSGGGGSQSVLTQPPSVSAAPGQKVTISCSGSSSNIGNWYVSWYQQLPGTAPKLLIYDNNKRPSGIPDRFSGSKSGTSATLGITGLQTGDEADYYCGTWDSSLSAPWVFGGGTKVTVLGGGGSEVQLVESGGGLVQPGGSLRLSCAASGVTFNYYGMSWIRQAPGKGLEWVASITRSGGRIYYPDSVKGRFTISRENTQKTLYLQMNSLRAEDTAVYYCTLDGRDGWVAYWGQGTLVTVSSGGGGSGGGGSGGGGSNFMLTQPSSVSGVPGQRVTISCTGNTGNIGSNYVNWYQQLPGTAPKLLIYRDDKRPSGVPDRFSGSKSGTSASLAITGFQAEDEADYYCQSYSSGFIFGGGTKLTVLAAEPKSSDKTHTCPPCPAPEAAGGPSVFLFPPKPKDTLMISRTPEVTCVVVSVSHEDPEVKFNWYVDGVEVHNAKTKPREEQYNSTYRVVSVLTVLHQDWLNGKEYKCKVSNKALPAPIEKTISKAKGQPREPQVYVYPPSRDELTKNQVSLTCLVKGFYPSDIAVEWESNGQPENNYKTTPPVLDSDGSFALVSKLTVDKSRWQQGNVFSCSVMHEALHNHYTQKSLSLSPGK

SEQ ID NO: 96 - protein, 745 aa, Artificial
  Full-length amino acid sequence of NYF-0061-HC2
MKHLWFFLLLVAAPRWVLSGEVQLVESGGGLVQPGGSLRLSCAASGFSIRSYDIHWVRQAPGKGLEWVATISYDGSQKYYADSVKGRFTISRDESKNTLYLQMNSLRAEDTAVYHCARGSSGHYEAFDIWGQGTLVTVSSGGGGSGGGGSGGGGSQSVLTQPPSASGTPGQRVTISCSGSSSNIGNWYVSWYQQLPGTAPKLLIYDNNKRPSGVPDRFSGSKSGTSASLAISGLQSEDEADYYCGTWDSSLSAPWVFGGGTKLTVLGGGGSEVQLVESGGGLVQPGGSLRLSCAASGVTFNYYGMSWIRQAPGKGLEWVASITRSGGRIYYPDSVKGRFTISRENTQKTLYLQMNSLRAEDTAVYYCTLDGRDGWVAYWGQGTLVTVSSGGGGSGGGGSGGGGSNFMLTQPSSVSGVPGQRVTISCTGNTGNIGSNYVNWYQQLPGTAPKLLIYRDDKRPSGVPDRFSGSKSGTSASLAITGFQAEDEADYYCQSYSSGFIFGGGTKLTVLAAEPKSSDKTHTCPPCPAPEAAGGPSVFLFPPKPKDTLMISRTPEVTCVVVSVSHEDPEVKFNWYVDGVEVHNAKTKPREEQYNSTYRVVSVLTVLHQDWLNGKEYKCKVSNKALPAPIEKTISKAKGQPREPQVYVYPPSRDELTKNQVSLTCLVKGFYPSDIAVEWESNGQPENNYKTTPPVLDSDGSFALVSKLTVDKSRWQQGNVFSCSVMHEALHNHYTQKSLSLSPGK

SEQ ID NO: 97 - DNA, 1404 bp, Artificial
  Full-length nucleotide sequence of NYA-0001-Fab-HC1-k delete
atgaaacacctgtggttcttcctcctgctggtggcagctcccagatgggtgctgagcgaggtgcagctggtggagtctgggggaggcgtggtccagcctgggaggtccctgacaccctcctgttcagcgtctggattctccatccgtagttatgatatacactgggtccgccaggctccaggcaaggggctagagtgggtggccactatatcatatgatggaagtcagaagtacttcgcagactccgtgaagggccgatttaccatcttcagagacgaatcggagaacatggtgtatctgcaaatgagcggcctgagagttgaggacacggctgtttatcactgtgcgagagggagtagtggtcattatgaggcttttgatatctggggccaagggacaatggtcaccgtctcttcagcctccaccaagggcccaagcgtcttccccctggcaccctcctccaagagcacctctggcggcacagccgccctgggctgcctggtcaaggactacttccccgaacccgtgaccgtgagctggaactcaggcgccctgaccagcggcgtgcacaccttccccgctgtcctgcagtcctcaggactctactccctcagcagcgtggtgaccgtgccctccagcagcttgggcacccagacctacatctgcaacgtgaatcacaagcccagcaacaccaaggtggacaagagagttgagcccaaatcttgtgacaaaactcacacatgcccaccctgcccagcacctgaagccgcagggggaccctcagtcttcctcttccccccaaaacccaaggacaccctcatgatctcccggacccctgaggtcacatgcgtggtggtgtcagtgagccacgaagaccctgaggtcaagttcaactggtacgtggacggcgtggaggtgcataatgccaagacaaagccccgggaggagcagtacaacagcacgtaccgggtggtcagcgtcctcaccgtcctgcaccaggactggctgaatggcaaggagtacaagtgcaaggtctccaacaaagccctcccagcccccatcgagaaaaccatctccaaagccaaaggccagccccgggaaccacaggtgtacgtgctgcccccatcccgggacgagctgaccaagaaccaggtcagcctgctgtgcctggtcaaaggcttctatcccagcgacatcgccgtggagtgggagagcaatggccagcccgagaacaactacctgacctggcctcccgtgctggactccgacggctccttcttcctctacagcaagctcaccgtggacaagagcaggtggcagcagggcaacgtcttctcatgctccgtgatgcatgaggctctgcacaaccactacacccagaagagcctctccctgtctcccggc

SEQ ID NO: 98 - DNA, 711 bp, Artificial
  Full-length nucleotide sequence of NYA-0001-LC
atggtgctgcagacccaggtgttcatctccctgctgctgtggatctccggcgcgtacggccagtctgtgttgacgcagccgccctcagtgtctgcggccccaggacagaaggtcaccatctcctgctctggaagcagctccaacattgggaataattatgtatcctggtaccagcagctcccaggaacagcccccaaactcctcatttatgacaataataagcgaccctcagggattcctgaccgattctctggctccaagtctggcacgtcagccaccctgggcatcaccggactccagactggggacgaggccgattattactgcggaacatgggatagcagcctgagtgccccttgggtgttcggcggagggaccaaggtcaccgtcctaggccagcctaaggctgcccctagcgtgaccctgttccctccttccagcgaggagcttcaagctaacaaggccaccctggtgtgtcttatctctgacttctaccctggcgctgtgaccgtggcctggaaggctgacagctcccctgtgaaggccggagtggagaccaccacacctagcaagcagtctaacaacaagtacgctgccagctcctacctgagccttacccctgagcagtggaagtctcacagaagctactcctgtcaagtgacccacgagggcagcaccgtggagaagaccgtggctcctaccgagtgttcc

SEQ ID NO: 99 - protein, 468 aa, Artificial
  Full-length amino acid sequence of NYA-0001-Fab-HC1-k delete
MKHLWFFLLLVAAPRWVLSEVQLVESGGGVVQPGRSLTPSCSASGFSIRSYDIHWVRQAPGKGLEWVATISYDGSQKYFADSVKGRFTIFRDESENMVYLQMSGLRVEDTAVYHCARGSSGHYEAFDIWGQGTMVTVSSASTKGPSVFPLAPSSKSTSGGTAALGCLVKDYFPEPVTVSWNSGALTSGVHTFPAVLQSSGLYSLSSVVTVPSSSLGTQTYICNVNHKPSNTKVDKRVEPKSCDKTHTCPPCPAPEAAGGPSVFLFPPKPKDTLMISRTPEVTCVVVSVSHEDPEVKFNWYVDGVEVHNAKTKPREEQYNSTYRVVSVLTVLHQDWLNGKEYKCKVSNKALPAPIEKTISKAKGQPREPQVYVLPPSRDELTKNQVSLLCLVKGFYPSDIAVEWESNGQPENNYLTWPPVLDSDGSFFLYSKLTVDKSRWQQGNVFSCSVMHEALHNHYTQKSLSLSPG

SEQ ID NO: 100 - protein, 237 aa, Artificial
  Full-length amino acid sequence of NYA-0001-LC
MVLQTQVFISLLLWISGAYGQSVLTQPPSVSAAPGQKVTISCSGSSSNIGNNYVSWYQQLPGTAPKLLIYDNNKRPSGIPDRFSGSKSGTSATLGITGLQTGDEADYYCGTWDSSLSAPWVFGGGTKVTVLGQPKAAPSVTLFPPSSEELQANKATLVCLISDFYPGAVTVAWKADSSPVKAGVETTTPSKQSNNKYAASSYLSLTPEQWKSHRSYSCQVTHEGSTVEKTVAPTECS

SEQ ID NO: 101 - DNA, 1404 bp, Artificial
  Full-length nucleotide sequence of NYA-1143-Fab-HC1-k delete
atgaaacacctgtggttcttcctcctgctggtggcagctcccagatgggtgctgagcgaggtgcagctggtggagtctgggggaggcgtggtccagcctgggaggtccctgacaccctcctgttcagcgtctggattctccatccgtagctatgatatacactgggtccgcctggctccaggcaaggggctagagtgggtggccactatatcatatgatggaagtcagaagtacttcgcagactccgtgaagggccgatttaccatcttcagagacgaatcggagaacatggtgtatctgcaaatgagcggcctgagagttgaggacacggctgtttatcactgtgcgagagggagtagtggtcattatgaggcttttgatatctggggccaagggacaatggtcaccgtctcttcagcctccaccaagggcccaagcgtcttccccctggcaccctcctccaagagcacctctggcggcacagccgccctgggctgcctggtcaaggactacttccccgaacccgtgaccgtgagctggaactcaggcgccctgaccagcggcgtgcacaccttccccgctgtcctgcagtcctcaggactctactccctcagcagcgtggtgaccgtgccctccagcagcttgggcacccagacctacatctgcaacgtgaatcacaagcccagcaacaccaaggtggacaagagagttgagcccaaatcttgtgacaaaactcacacatgcccaccctgcccagcacctgaagccgcagggggaccctcagtcttcctcttccccccaaaacccaaggacaccctcatgatctcccggacccctgaggtcacatgcgtggtggtgtcagtgagccacgaagaccctgaggtcaagttcaactggtacgtggacggcgtggaggtgcataatgccaagacaaagccccgggaggagcagtacaacagcacgtaccgggtggtcagcgtcctcaccgtcctgcaccaggactggctgaatggcaaggagtacaagtgcaaggtctccaacaaagccctcccagcccccatcgagaaaaccatctccaaagccaaaggccagccccgggaaccacaggtgtacgtgctgcccccatcccgggacgagctgaccaagaaccaggtcagcctgctgtgcctggtcaaaggcttctatcccagcgacatcgccgtggagtgggagagcaatggccagcccgagaacaactacctgacctggcctcccgtgctggactccgacggctccttcttcctctacagcaagctcaccgtggacaagagcaggtggcagcagggcaacgtcttctcatgctccgtgatgcatgaggctctgcacaaccactacacccagaagagcctctccctgtctcccggc

SEQ ID NO: 102 - DNA, 711 bp, Artificial
  Full-length nucleotide sequence of NYA-1143-LC
atggtgctgcagacccaggtgttcatctccctgctgctgtggatctccggcgcgtacggccagtctgtgttgacgcagccgccctcagtgtctgcggccccaggacagaaggtcaccatctcctgctctggaagcagctccaacattgggaattggtatgtatcctggtaccagcagctcccaggaacagcccccaaactcctcatttatgacaataataagcgaccctcagggattcctgaccgattctctggctccaagtctggcacgtcagccaccctgggcatcaccggactccagactggggacgaggccgattattactgcggaacatgggatagcagcctgagtgccccttgggtgttcggcggagggaccaaggtcaccgtcctaggccagcctaaggctgcccctagcgtgaccctgttccctccttccagcgaggagcttcaagctaacaaggccaccctggtgtgtcttatctctgacttctaccctggcgctgtgaccgtggcctggaaggctgacagctcccctgtgaaggccggagtggagaccaccacacctagcaagcagtctaacaacaagtacgctgccagctcctacctgagccttacccctgagcagtggaagtctcacagaagctactcctgtcaagtgacccacgagggcagcaccgtggagaagaccgtggctcctaccgagtgttcc

SEQ ID NO: 103 - DNA, 1476 bp, Artificial
  Full-length nucleotide sequence of C3E-7085-HC2-k delete
atgaaacacctgtggttcttcctcctgctggtggcagctcccagatgggtgctgagcggagaagtgcagctggtggaatccggggggggcctggtgcagcctggggggagcctgagactgagttgtgccgcctctggggtgacatttaactactatggcatgtcttggatccgccaggcacctggaaagggcctggagtgggtggccagcatcactaggtccggcgggcgaatctactatcccgacagcgtcaagggcaggttcacaatttcccgcgagaacacacagaaaactctgtacctgcagatgaatagcctgagagccgaagatacagctgtgtactattgcactctggacggcagggatgggtgggtcgcctattgggggcagggaaccctggtgacagtcagctccggaggaggaggatctggcggaggaggcagtgggggaggcgggtcaaactttatgctcactcagccgtcctctgtttctggcgtacctggccaacgggtgaccattagctgtacgggtaataccgggaatatcgggtctaactacgtgaactggtatcagcagcttccagggacagctcccaagttgctgatctatcgcgacgacaaaagaccctcaggggtccctgaccgatttagtggcagcaaaagcggtacttccgcttccctggcgataaccggctttcaggccgaagatgaggcagactactattgccagtcatattccagcggcttcatcttcggaggcggaactaagctgacagtgttggcagccgagcccaaatcttctgacaaaactcacacatgcccaccctgcccagcacctgaagccgcagggggaccctcagtcttcctcttccccccaaaacccaaggacaccctcatgatctcccggacccctgaggtcacatgcgtggtggtgtcagtgagccacgaagaccctgaggtcaagttcaactggtacgtggacggcgtggaggtgcataatgccaagacaaagccccgggaggagcagtacaacagcacgtaccgggtggtcagcgtcctcaccgtcctgcaccaggactggctgaatggcaaggagtacaagtgcaaggtctccaacaaagccctcccagcccccatcgagaaaaccatctccaaagccaaaggccagccccgggaaccacaggtgtacgtgtaccccccatcccgggacgagctgaccaagaaccaggtcagcctgacctgcctggtcaaaggcttctatcccagcgacatcgccgtggagtgggagagcaatggccagcccgagaacaactacaagaccacccctcccgtgctggactccgacggctccttcgccctcgtgagcaagctcaccgtggacaagagcaggtggcagcagggcaacgtcttctcatgctccgtgatgcatgaggctctgcacaaccactacacccagaagagcctctccctgtctccc

SEQ ID NO: 104 - protein, 468 aa, Artificial
  Full-length amino acid sequence of NYA-1143-Fab-HC1-k delete
MKHLWFFLLLVAAPRWVLSEVQLVESGGGVVQPGRSLTPSCSASGFSIRSYDIHWVRLAPGKGLEWVATISYDGSQKYFADSVKGRFTIFRDESENMVYLQMSGLRVEDTAVYHCARGSSGHYEAFDIWGQGTMVTVSSASTKGPSVFPLAPSSKSTSGGTAALGCLVKDYFPEPVTVSWNSGALTSGVHTFPAVLQSSGLYSLSSVVTVPSSSLGTQTYICNVNHKPSNTKVDKRVEPKSCDKTHTCPPCPAPEAAGGPSVFLFPPKPKDTLMISRTPEVTCVVVSVSHEDPEVKFNWYVDGVEVHNAKTKPREEQYNSTYRVVSVLTVLHQDWLNGKEYKCKVSNKALPAPIEKTISKAKGQPREPQVYVLPPSRDELTKNQVSLLCLVKGFYPSDIAVEWESNGQPENNYLTWPPVLDSDGSFFLYSKLTVDKSRWQQGNVFSCSVMHEALHNHYTQKSLSLSPG

SEQ ID NO: 105 - protein, 237 aa, Artificial
  Full-length amino acid sequence of NYA-1143-LC
MVLQTQVFISLLLWISGAYGQSVLTQPPSVSAAPGQKVTISCSGSSSNIGNWYVSWYQQLPGTAPKLLIYDNNKRPSGIPDRFSGSKSGTSATLGITGLQTGDEADYYCGTWDSSLSAPWVFGGGTKVTVLGQPKAAPSVTLFPPSSEELQANKATLVCLISDFYPGAVTVAWKADSSPVKAGVETTTPSKQSNNKYAASSYLSLTPEQWKSHRSYSCQVTHEGSTVEKTVAPTECS

SEQ ID NO: 106 - protein, 493 aa, Artificial
  Full-length amino acid sequence of C3E-7085-HC2-k delete
MKHLWFFLLLVAAPRWVLSGEVQLVESGGGLVQPGGSLRLSCAASGVTFNYYGMSWIRQAPGKGLEWVASITRSGGRIYYPDSVKGRFTISRENTQKTLYLQMNSLRAEDTAVYYCTLDGRDGWVAYWGQGTLVTVSSGGGGSGGGGSGGGGSNFMLTQPSSVSGVPGQRVTISCTGNTGNIGSNYVNWYQQLPGTAPKLLIYRDDKRPSGVPDRFSGSKSGTSASLAITGFQAEDEADYYCQSYSSGFIFGGGTKLTVLAAEPKSSDKTHTCPPCPAPEAAGGPSVFLFPPKPKDTLMISRTPEVTCVVVSVSHEDPEVKFNWYVDGVEVHNAKTKPREEQYNSTYRVVSVLTVLHQDWLNGKEYKCKVSNKALPAPIEKTISKAKGQPREPQVYVYPPSRDELTKNQVSLTCLVKGFYPSDIAVEWESNGQPENNYKTTPPVLDSDGSFALVSKLTVDKSRWQQGNVFSCSVMHEALHNHYTQKSLSLSPG

SEQ ID NO: 107 - DNA, 1497 bp, Artificial
  Full-length nucleotide sequence of NYA-1143-HC1-k delete
atgaaacacctgtggttcttcctcctgctggtggcagctcccagatgggtgctgagcggagaggtgcagctggtggagtctgggggaggcgtggtccagcctgggaggtccctgacaccctcctgttcagcgtctggattctccatccgtagctatgatatacactgggtccgcctggctccaggcaaggggctagagtgggtggccactatatcatatgatggaagtcagaagtacttcgcagactccgtgaagggccgatttaccatcttcagagacgaatcggagaacatggtgtatctgcaaatgagcggcctgagagttgaggacacggctgtttatcactgtgcgagagggagtagtggtcattatgaggcttttgatatctggggccaagggacaatggtcaccgtctcttcaggtggaggcggttcaggcggaggtggcagcggcggtggcgggagtcagtctgtgttgacgcagccgccctcagtgtctgcggccccaggacagaaggtcaccatctcctgctctggaagcagctccaacattgggaattggtatgtatcctggtaccagcagctcccaggaacagcccccaaactcctcatttatgacaataataagcgaccctcagggattcctgaccgattctctggctccaagtctggcacgtcagccaccctgggcatcaccggactccagactggggacgaggccgattattactgcggaacatgggatagcagcctgagtgccccttgggtgttcggcggagggaccaaggtcaccgtcctagcagccgagcccaaatcttctgacaaaactcacacatgcccaccctgcccagcacctgaagccgcagggggaccctcagtcttcctcttccccccaaaacccaaggacaccctcatgatctcccggacccctgaggtcacatgcgtggtggtgtcagtgagccacgaagaccctgaggtcaagttcaactggtacgtggacggcgtggaggtgcataatgccaagacaaagccccgggaggagcagtacaacagcacgtaccgggtggtcagcgtcctcaccgtcctgcaccaggactggctgaatggcaaggagtacaagtgcaaggtctccaacaaagccctcccagcccccatcgagaaaaccatctccaaagccaaaggccagccccgggaaccacaggtgtacgtgctgcccccatcccgggacgagctgaccaagaaccaggtcagcctgctgtgcctggtcaaaggcttctatcccagcgacatcgccgtggagtgggagagcaatggccagcccgagaacaactacctgacctggcctcccgtgctggactccgacggctccttcttcctctacagcaagctcaccgtggacaagagcaggtggcagcagggcaacgtcttctcatgctccgtgatgcatgaggctctgcacaaccactacacccagaagagcctctccctgtctcccggc

SEQ ID NO: 108 - protein, 499 aa, Artificial
  Full-length amino acid sequence of NYA-1143-HC1-k delete
MKHLWFFLLLVAAPRWVLSGEVQLVESGGGVVQPGRSLTPSCSASGFSIRSYDIHWVRLAPGKGLEWVATISYDGSQKYFADSVKGRFTIFRDESENMVYLQMSGLRVEDTAVYHCARGSSGHYEAFDIWGQGTMVTVSSGGGGSGGGGSGGGGSQSVLTQPPSVSAAPGQKVTISCSGSSSNIGNWYVSWYQQLPGTAPKLLIYDNNKRPSGIPDRFSGSKSGTSATLGITGLQTGDEADYYCGTWDSSLSAPWVFGGGTKVTVLAAEPKSSDKTHTCPPCPAPEAAGGPSVFLFPPKPKDTLMISRTPEVTCVVVSVSHEDPEVKFNWYVDGVEVHNAKTKPREEQYNSTYRVVSVLTVLHQDWLNGKEYKCKVSNKALPAPIEKTISKAKGQPREPQVYVLPPSRDELTKNQVSLLCLVKGFYPSDIAVEWESNGQPENNYLTWPPVLDSDGSFFLYSKLTVDKSRWQQGNVFSCSVMHEALHNHYTQKSLSLSPG

SEQ ID NO: 109 - DNA, 2142 bp, Artificial
  Full-length nucleotide sequence of C3E-7085-NYA-1154-Fab-HC2-k delete
atgaaacacctgtggttcttcctcctgctggtggcagctcccagatgggtgctgagcggagaagtgcagctggtggaatccggggggggcctggtgcagcctggggggagcctgagactgagttgtgccgcctctggggtgacatttaactactatggcatgtcttggatccgccaggcacctggaaagggcctggagtgggtggccagcatcactaggtccggcgggcgaatctactatcccgacagcgtcaagggcaggttcacaatttcccgcgagaacacacagaaaactctgtacctgcagatgaatagcctgagagccgaagatacagctgtgtactattgcactctggacggcagggatgggtgggtcgcctattgggggcagggaaccctggtgacagtcagctccggaggaggaggatctggcggaggaggcagtgggggaggcgggtcaaactttatgctcactcagccgtcctctgtttctggcgtacctggccaacgggtgaccattagctgtacgggtaataccgggaatatcgggtctaactacgtgaactggtatcagcagcttccagggacagctcccaagttgctgatctatcgcgacgacaaaagaccctcaggggtccctgaccgatttagtggcagcaaaagcggtacttccgcttccctggcgataaccggctttcaggccgaagatgaggcagactactattgccagtcatattccagcggcttcatcttcggaggcggaactaagctgacagtgttggggggaggcggttcagaggtgcagctggtggagtctgggggaggcgtggtccagcctgggaggtccctgacaccctcctgttcagcgtctggattctccatccgtagttatgatatgcactgggtccgccaggctccaggcaaggggctagagtgggtggccactatatcatatgatggaagtcagaagtacttcgcagactccgtgaagggccgatttaccatcttcagagacgaatcggagaacatggtgtatctgcaaatgagcggcctgagagttgaggacacggccgtttatcactgtgcgagagggagtagtaatcattatgaggcttttgatatctggggccaagggacaatggtcaccgtctcttcagcctccaccaagggcccaagcgtcttccccctggcaccctcctccaagagcacctctggcggcacagccgccctgggctgcctggtcaaggactacttccccgaacccgtgaccgtgagctggaactcaggcgccctgaccagcggcgtgcacaccttccccgctgtcctgcagtcctcaggactctactccctcagcagcgtggtgaccgtgccctccagcagcttgggcacccagacctacatctgcaacgtgaatcacaagcccagcaacaccaaggtggacaagagagttgagcccaaatcttgtgacaaaactcacacatgcccaccctgcccagcacctgaagccgcagggggaccctcagtcttcctcttccccccaaaacccaaggacaccctcatgatctcccggacccctgaggtcacatgcgtggtggtgtcagtgagccacgaagaccctgaggtcaagttcaactggtacgtggacggcgtggaggtgcataatgccaagacaaagccccgggaggagcagtacaacagcacgtaccgggtggtcagcgtcctcaccgtcctgcaccaggactggctgaatggcaaggagtacaagtgcaaggtctccaacaaagccctcccagcccccatcgagaaaaccatctccaaagccaaaggccagccccgggaaccacaggtgtacgtgtaccccccatcccgggacgagctgaccaagaaccaggtcagcctgacctgcctggtcaaaggcttctatcccagcgacatcgccgtggagtgggagagcaatggccagcccgagaacaactacaagaccacccctcccgtgctggactccgacggctccttcgccctcgtgagcaagctcaccgtggacaagagcaggtggcagcagggcaacgtcttctcatgctccgtgatgcatgaggctctgcacaaccactacacccagaagagcctctccctgtctcccggc

SEQ ID NO: 110 - DNA, 711 bp, Artificial
  Full-length nucleotide sequence of NYA-1154-LC
atggtgctgcagacccaggtgttcatctccctgctgctgtggatctccggcgcgtacggccagtctgtgttgacgcagccgccctcagtgtctgcggccccaggacagaaggtcaccatctcctgctctggaagcagctccaacattgggaataattatgtatcctggtaccagcggctcccaggaacagcccccaaactcctcatttatgacaataataagcgaccctcagggattcctgaccgattctctggctccaagtctggcacgtcagccaccctgggcatcaccggactccagactggggacgaggccgattactactgcggagcatgggatagcagcctgagtgccccttgggtgttcggcggagggaccaaggtcaccgtcctaggccagcctaaggctgcccctagcgtgaccctgttccctccttccagcgaggagcttcaagctaacaaggccaccctggtgtgtcttatctctgacttctaccctggcgctgtgaccgtggcctggaaggctgacagctcccctgtgaaggccggagtggagaccaccacacctagcaagcagtctaacaacaagtacgctgccagctcctacctgagccttacccctgagcagtggaagtctcacagaagctactcctgtcaagtgacccacgagggcagcaccgtggagaagaccgtggctcctaccgagtgttcc

SEQ ID NO: 111 - DNA, 735 bp, Artificial
  Full-length nucleotide sequence of OAA-HC1-k delete
atgaaacacctgtggttcttcctcctgctggtggcagctcccagatgggtgctgagcgacaaaactcacacatgcccaccctgcccagcacctgaagccgcagggggaccctcagtcttcctcttccccccaaaacccaaggacaccctcatgatctcccggacccctgaggtcacatgcgtggtggtgtcagtgagccacgaagaccctgaggtcaagttcaactggtacgtggacggcgtggaggtgcataatgccaagacaaagccccgggaggagcagtacaacagcacgtaccgggtggtcagcgtcctcaccgtcctgcaccaggactggctgaatggcaaggagtacaagtgcaaggtctccaacaaagccctcccagcccccatcgagaaaaccatctccaaagccaaaggccagccccgggaaccacaggtgtacgtgctgcccccatcccgggacgagctgaccaagaaccaggtcagcctgctgtgcctggtcaaaggcttctatcccagcgacatcgccgtggagtgggagagcaatggccagcccgagaacaactacctgacctggcctcccgtgctggactccgacggctccttcttcctctacagcaagctcaccgtggacaagagcaggtggcagcagggcaacgtcttctcatgctccgtgatgcatgaggctctgcacaaccactacacccagaagagcctctccctgtctcccggc

SEQ ID NO: 112 - protein, 714 aa, Artificial
  Full-length amino acid sequence of C3E-7085-NYA-1154-Fab-HC2-k delete
MKHLWFFLLLVAAPRWVLSGEVQLVESGGGLVQPGGSLRLSCAASGVTFNYYGMSWIRQAPGKGLEWVASITRSGGRIYYPDSVKGRFTISRENTQKTLYLQMNSLRAEDTAVYYCTLDGRDGWVAYWGQGTLVTVSSGGGGSGGGGSGGGGSNFMLTQPSSVSGVPGQRVTISCTGNTGNIGSNYVNWYQQLPGTAPKLLIYRDDKRPSGVPDRFSGSKSGTSASLAITGFQAEDEADYYCQSYSSGFIFGGGTKLTVLGGGGSEVQLVESGGGVVQPGRSLTPSCSASGFSIRSYDMHWVRQAPGKGLEWVATISYDGSQKYFADSVKGRFTIFRDESENMVYLQMSGLRVEDTAVYHCARGSSNHYEAFDIWGQGTMVTVSSASTKGPSVFPLAPSSKSTSGGTAALGCLVKDYFPEPVTVSWNSGALTSGVHTFPAVLQSSGLYSLSSVVTVPSSSLGTQTYICNVNHKPSNTKVDKRVEPKSCDKTHTCPPCPAPEAAGGPSVFLFPPKPKDTLMISRTPEVTCVVVSVSHEDPEVKFNWYVDGVEVHNAKTKPREEQYNSTYRVVSVLTVLHQDWLNGKEYKCKVSNKALPAPIEKTISKAKGQPREPQVYVYPPSRDELTKNQVSLTCLVKGFYPSDIAVEWESNGQPENNYKTTPPVLDSDGSFALVSKLTVDKSRWQQGNVFSCSVMHEALHNHYTQKSLSLSPG

SEQ ID NO: 113 - protein, 237 aa, Artificial
  Full-length amino acid sequence of NYA-1154-LC
MVLQTQVFISLLLWISGAYGQSVLTQPPSVSAAPGQKVTISCSGSSSNIGNNYVSWYQRLPGTAPKLLIYDNNKRPSGIPDRFSGSKSGTSATLGITGLQTGDEADYYCGAWDSSLSAPWVFGGGTKVTVLGQPKAAPSVTLFPPSSEELQANKATLVCLISDFYPGAVTVAWKADSSPVKAGVETTTPSKQSNNKYAASSYLSLTPEQWKSHRSYSCQVTHEGSTVEKTVAPTECS

SEQ ID NO: 114 - protein, 245 aa, Artificial
  Full-length amino acid sequence of OAA-HC1-k delete
MKHLWFFLLLVAAPRWVLSDKTHTCPPCPAPEAAGGPSVFLFPPKPKDTLMISRTPEVTCVVVSVSHEDPEVKFNWYVDGVEVHNAKTKPREEQYNSTYRVVSVLTVLHQDWLNGKEYKCKVSNKALPAPIEKTISKAKGQPREPQVYVLPPSRDELTKNQVSLLCLVKGFYPSDIAVEWESNGQPENNYLTWPPVLDSDGSFFLYSKLTVDKSRWQQGNVFSCSVMHEALHNHYTQKSLSLSPG

SEQ ID NO: 115 - DNA, 2232 bp, Artificial
  Full-length nucleotide sequence of NYF-0010-HC2-k delete
atgaaacacctgtggttcttcctcctgctggtggcagctcccagatgggtgctgagcggagaggtgcagctggtggagtctgggggaggcgtggtccagcctgggaggtccctgacaccctcctgttcagcgtctggattctccatccgtagttatgatatgcactgggtccgccaggctccaggcaaggggctagagtgggtggccactatatcatatgatggaagtcagaagtacttcgcagactccgtgaagggccgatttaccatcttcagagacgaatcggagaacatggtgtatctgcaaatgagcggcctgagagttgaggacacggccgtttatcactgtgcgagagggagtagtaatcattatgaggcttttgatatctggggccaagggacaatggtcaccgtctcttcaggtggaggcggttcaggcggaggtggcagcggcggtggcgggagtcagtctgtgttgacgcagccgccctcagtgtctgcggccccaggacagaaggtcaccatctcctgctctggaagcagctccaacattgggaataattatgtatcctggtaccagcggctcccaggaacagcccccaaactcctcatttatgacaataataagcgaccctcagggattcctgaccgattctctggctccaagtctggcacgtcagccaccctgggcatcaccggactccagactggggacgaggccgattactactgcggagcatgggatagcagcctgagtgccccttgggtgttcggcggagggaccaaggtcaccgtcctagggggaggcggttcagaagtgcagctggtggaatccggggggggcctggtgcagcctggggggagcctgagactgagttgtgccgcctctggggtgacatttaactactatggcatgtcttggatccgccaggcacctggaaagggcctggagtgggtggccagcatcactaggtccggcgggcgaatctactatcccgacagcgtcaagggcaggttcacaatttcccgcgagaacacacagaaaactctgtacctgcagatgaatagcctgagagccgaagatacagctgtgtactattgcactctggacggcagggatgggtgggtcgcctattgggggcagggaaccctggtgacagtcagctccggaggaggaggatctggcggaggaggcagtgggggaggcgggtcaaactttatgctcactcagccgtcctctgtttctggcgtacctggccaacgggtgaccattagctgtacgggtaataccgggaatatcgggtctaactacgtgaactggtatcagcagcttccagggacagctcccaagttgctgatctatcgcgacgacaaaagaccctcaggggtccctgaccgatttagtggcagcaaaagcggtacttccgcttccctggcgataaccggctttcaggccgaagatgaggcagactactattgccagtcatattccagcggcttcatcttcggaggcggaactaagctgacagtgttggcagccgagcccaaatcttctgacaaaactcacacatgcccaccctgcccagcacctgaagccgcagggggaccctcagtcttcctcttccccccaaaacccaaggacaccctcatgatctcccggacccctgaggtcacatgcgtggtggtgtcagtgagccacgaagaccctgaggtcaagttcaactggtacgtggacggcgtggaggtgcataatgccaagacaaagccccgggaggagcagtacaacagcacgtaccgggtggtcagcgtcctcaccgtcctgcaccaggactggctgaatggcaaggagtacaagtgcaaggtctccaacaaagccctcccagcccccatcgagaaaaccatctccaaagccaaaggccagccccgggaaccacaggtgtacgtgtaccccccatcccgggacgagctgaccaagaaccaggtcagcctgacctgcctggtcaaaggcttctatcccagcgacatcgccgtggagtgggagagcaatggccagcccgagaacaactacaagaccacccctcccgtgctggactccgacggctccttcgccctcgtgagcaagctcaccgtggacaagagcaggtggcagcagggcaacgtcttctcatgctccgtgatgcatgaggctctgcacaaccactacacccagaagagcctctccctgtctcccggc

SEQ ID NO: 116 - DNA, 2232 bp, Artificial
  Full-length nucleotide sequence of NYF-0004-HC2-k delete
atgaaacacctgtggttcttcctcctgctggtggcagctcccagatgggtgctgagcggagaagtgcagctggtggaatccggggggggcctggtgcagcctggggggagcctgagactgagttgtgccgcctctggggtgacatttaactactatggcatgtcttggatccgccaggcacctggaaagggcctggagtgggtggccagcatcactaggtccggcgggcgaatctactatcccgacagcgtcaagggcaggttcacaatttcccgcgagaacacacagaaaactctgtacctgcagatgaatagcctgagagccgaagatacagctgtgtactattgcactctggacggcagggatgggtgggtcgcctattgggggcagggaaccctggtgacagtcagctccggaggaggaggatctggcggaggaggcagtgggggaggcgggtcaaactttatgctcactcagccgtcctctgtttctggcgtacctggccaacgggtgaccattagctgtacgggtaataccgggaatatcgggtctaactacgtgaactggtatcagcagcttccagggacagctcccaagttgctgatctatcgcgacgacaaaagaccctcaggggtccctgaccgatttagtggcagcaaaagcggtacttccgcttccctggcgataaccggctttcaggccgaagatgaggcagactactattgccagtcatattccagcggcttcatcttcggaggcggaactaagctgacagtgttggggggaggcggttcagaggtgcagctggtggagtctgggggaggcgtggtccagcctgggaggtccctgacaccctcctgttcagcgtctggattctccatccgtagttatgatatgcactgggtccgccaggctccaggcaaggggctagagtgggtggccactatatcatatgatggaagtcagaagtacttcgcagactccgtgaagggccgatttaccatcttcagagacgaatcggagaacatggtgtatctgcaaatgagcggcctgagagttgaggacacggccgtttatcactgtgcgagagggagtagtaatcattatgaggcttttgatatctggggccaagggacaatggtcaccgtctcttcaggtggaggcggttcaggcggaggtggcagcggcggtggcgggagtcagtctgtgttgacgcagccgccctcagtgtctgcggccccaggacagaaggtcaccatctcctgctctggaagcagctccaacattgggaataattatgtatcctggtaccagcggctcccaggaacagcccccaaactcctcatttatgacaataataagcgaccctcagggattcctgaccgattctctggctccaagtctggcacgtcagccaccctgggcatcaccggactccagactggggacgaggccgattactactgcggagcatgggatagcagcctgagtgccccttgggtgttcggcggagggaccaaggtcaccgtcctagcagccgagcccaaatcttctgacaaaactcacacatgcccaccctgcccagcacctgaagccgcagggggaccctcagtcttcctcttccccccaaaacccaaggacaccctcatgatctcccggacccctgaggtcacatgcgtggtggtgtcagtgagccacgaagaccctgaggtcaagttcaactggtacgtggacggcgtggaggtgcataatgccaagacaaagccccgggaggagcagtacaacagcacgtaccgggtggtcagcgtcctcaccgtcctgcaccaggactggctgaatggcaaggagtacaagtgcaaggtctccaacaaagccctcccagcccccatcgagaaaaccatctccaaagccaaaggccagccccgggaaccacaggtgtacgtgtaccccccatcccgggacgagctgaccaagaaccaggtcagcctgacctgcctggtcaaaggcttctatcccagcgacatcgccgtggagtgggagagcaatggccagcccgagaacaactacaagaccacccctcccgtgctggactccgacggctccttcgccctcgtgagcaagctcaccgtggacaagagcaggtggcagcagggcaacgtcttctcatgctccgtgatgcatgaggctctgcacaaccactacacccagaagagcctctccctgtctcccggc

SEQ ID NO: 117 - DNA, 2232 bp, Artificial
  Full-length nucleotide sequence of NYF-0011-HC2-k delete
atgaaacacctgtggttcttcctcctgctggtggcagctcccagatgggtgctgagcggagaggtgcagctggtggagtctgggggaggcgtggtccagcctgggaggtccctgacaccctcctgttcagcgtctggattctccatccgtagctatgatatacactgggtccgcctggctccaggcaaggggctagagtgggtggccactatatcatatgatggaagtcagaagtacttcgcagactccgtgaagggccgatttaccatcttcagagacgaatcggagaacatggtgtatctgcaaatgagcggcctgagagttgaggacacggctgtttatcactgtgcgagagggagtagtggtcattatgaggcttttgatatctggggccaagggacaatggtcaccgtctcttcaggtggaggcggttcaggcggaggtggcagcggcggtggcgggagtcagtctgtgttgacgcagccgccctcagtgtctgcggccccaggacagaaggtcaccatctcctgctctggaagcagctccaacattgggaattggtatgtatcctggtaccagcagctcccaggaacagcccccaaactcctcatttatgacaataataagcgaccctcagggattcctgaccgattctctggctccaagtctggcacgtcagccaccctgggcatcaccggactccagactggggacgaggccgattattactgcggaacatgggatagcagcctgagtgccccttgggtgttcggcggagggaccaaggtcaccgtcctagggggaggcggttcagaagtgcagctggtggaatccggggggggcctggtgcagcctggggggagcctgagactgagttgtgccgcctctggggtgacatttaactactatggcatgtcttggatccgccaggcacctggaaagggcctggagtgggtggccagcatcactaggtccggcgggcgaatctactatcccgacagcgtcaagggcaggttcacaatttcccgcgagaacacacagaaaactctgtacctgcagatgaatagcctgagagccgaagatacagctgtgtactattgcactctggacggcagggatgggtgggtcgcctattgggggcagggaaccctggtgacagtcagctccggaggaggaggatctggcggaggaggcagtgggggaggcgggtcaaactttatgctcactcagccgtcctctgtttctggcgtacctggccaacgggtgaccattagctgtacgggtaataccgggaatatcgggtctaactacgtgaactggtatcagcagcttccagggacagctcccaagttgctgatctatcgcgacgacaaaagaccctcaggggtccctgaccgatttagtggcagcaaaagcggtacttccgcttccctggcgataaccggctttcaggccgaagatgaggcagactactattgccagtcatattccagcggcttcatcttcggaggcggaactaagctgacagtgttggcagccgagcccaaatcttctgacaaaactcacacatgcccaccctgcccagcacctgaagccgcagggggaccctcagtcttcctcttccccccaaaacccaaggacaccctcatgatctcccggacccctgaggtcacatgcgtggtggtgtcagtgagccacgaagaccctgaggtcaagttcaactggtacgtggacggcgtggaggtgcataatgccaagacaaagccccgggaggagcagtacaacagcacgtaccgggtggtcagcgtcctcaccgtcctgcaccaggactggctgaatggcaaggagtacaagtgcaaggtctccaacaaagccctcccagcccccatcgagaaaaccatctccaaagccaaaggccagccccgggaaccacaggtgtacgtgtaccccccatcccgggacgagctgaccaagaaccaggtcagcctgacctgcctggtcaaaggcttctatcccagcgacatcgccgtggagtgggagagcaatggccagcccgagaacaactacaagaccacccctcccgtgctggactccgacggctccttcgccctcgtgagcaagctcaccgtggacaagagcaggtggcagcagggcaacgtcttctcatgctccgtgatgcatgaggctctgcacaaccactacacccagaagagcctctccctgtctcccggc

SEQ ID NO: 118 - protein, 744 aa, Artificial
  Full-length amino acid sequence of NYF-0010-HC2-k delete
MKHLWFFLLLVAAPRWVLSGEVQLVESGGGVVQPGRSLTPSCSASGFSIRSYDMHWVRQAPGKGLEWVATISYDGSQKYFADSVKGRFTIFRDESENMVYLQMSGLRVEDTAVYHCARGSSNHYEAFDIWGQGTMVTVSSGGGGSGGGGSGGGGSQSVLTQPPSVSAAPGQKVTISCSGSSSNIGNNYVSWYQRLPGTAPKLLIYDNNKRPSGIPDRFSGSKSGTSATLGITGLQTGDEADYYCGAWDSSLSAPWVFGGGTKVTVLGGGGSEVQLVESGGGLVQPGGSLRLSCAASGVTFNYYGMSWIRQAPGKGLEWVASITRSGGRIYYPDSVKGRFTISRENTQKTLYLQMNSLRAEDTAVYYCTLDGRDGWVAYWGQGTLVTVSSGGGGSGGGGSGGGGSNFMLTQPSSVSGVPGQRVTISCTGNTGNIGSNYVNWYQQLPGTAPKLLIYRDDKRPSGVPDRFSGSKSGTSASLAITGFQAEDEADYYCQSYSSGFIFGGGTKLTVLAAEPKSSDKTHTCPPCPAPEAAGGPSVFLFPPKPKDTLMISRTPEVTCVVVSVSHEDPEVKFNWYVDGVEVHNAKTKPREEQYNSTYRVVSVLTVLHQDWLNGKEYKCKVSNKALPAPIEKTISKAKGQPREPQVYVYPPSRDELTKNQVSLTCLVKGFYPSDIAVEWESNGQPENNYKTTPPVLDSDGSFALVSKLTVDKSRWQQGNVFSCSVMHEALHNHYTQKSLSLSPG

SEQ ID NO: 119 - protein, 744 aa, Artificial
  Full-length amino acid sequence of NYF-0004-HC2-k delete
MKHLWFFLLLVAAPRWVLSGEVQLVESGGGLVQPGGSLRLSCAASGVTFNYYGMSWIRQAPGKGLEWVASITRSGGRIYYPDSVKGRFTISRENTQKTLYLQMNSLRAEDTAVYYCTLDGRDGWVAYWGQGTLVTVSSGGGGSGGGGSGGGGSNFMLTQPSSVSGVPGQRVTISCTGNTGNIGSNYVNWYQQLPGTAPKLLIYRDDKRPSGVPDRFSGSKSGTSASLAITGFQAEDEADYYCQSYSSGFIFGGGTKLTVLGGGGSEVQLVESGGGVVQPGRSLTPSCSASGFSIRSYDMHWVRQAPGKGLEWVATISYDGSQKYFADSVKGRFTIFRDESENMVYLQMSGLRVEDTAVYHCARGSSNHYEAFDIWGQGTMVTVSSGGGGSGGGGSGGGGSQSVLTQPPSVSAAPGQKVTISCSGSSSNIGNNYVSWYQRLPGTAPKLLIYDNNKRPSGIPDRFSGSKSGTSATLGITGLQTGDEADYYCGAWDSSLSAPWVFGGGTKVTVLAAEPKSSDKTHTCPPCPAPEAAGGPSVFLFPPKPKDTLMISRTPEVTCVVVSVSHEDPEVKFNWYVDGVEVHNAKTKPREEQYNSTYRVVSVLTVLHQDWLNGKEYKCKVSNKALPAPIEKTISKAKGQPREPQVYVYPPSRDELTKNQVSLTCLVKGFYPSDIAVEWESNGQPENNYKTTPPVLDSDGSFALVSKLTVDKSRWQQGNVFSCSVMHEALHNHYTQKSLSLSPG

SEQ ID NO: 120 - protein, 744 aa, Artificial
  Full-length amino acid sequence of NYF-0011-HC2-k delete
MKHLWFFLLLVAAPRWVLSGEVQLVESGGGVVQPGRSLTPSCSASGFSIRSYDIHWVRLAPGKGLEWVATISYDGSQKYFADSVKGRFTIFRDESENMVYLQMSGLRVEDTAVYHCARGSSGHYEAFDIWGQGTMVTVSSGGGGSGGGGSGGGGSQSVLTQPPSVSAAPGQKVTISCSGSSSNIGNWYVSWYQQLPGTAPKLLIYDNNKRPSGIPDRFSGSKSGTSATLGITGLQTGDEADYYCGTWDSSLSAPWVFGGGTKVTVLGGGGSEVQLVESGGGLVQPGGSLRLSCAASGVTFNYYGMSWIRQAPGKGLEWVASITRSGGRIYYPDSVKGRFTISRENTQKTLYLQMNSLRAEDTAVYYCTLDGRDGWVAYWGQGTLVTVSSGGGGSGGGGSGGGGSNFMLTQPSSVSGVPGQRVTISCTGNTGNIGSNYVNWYQQLPGTAPKLLIYRDDKRPSGVPDRFSGSKSGTSASLAITGFQAEDEADYYCQSYSSGFIFGGGTKLTVLAAEPKSSDKTHTCPPCPAPEAAGGPSVFLFPPKPKDTLMISRTPEVTCVVVSVSHEDPEVKFNWYVDGVEVHNAKTKPREEQYNSTYRVVSVLTVLHQDWLNGKEYKCKVSNKALPAPIEKTISKAKGQPREPQVYVYPPSRDELTKNQVSLTCLVKGFYPSDIAVEWESNGQPENNYKTTPPVLDSDGSFALVSKLTVDKSRWQQGNVFSCSVMHEALHNHYTQKSLSLSPG

SEQ ID NO: 121 - protein, 9 aa, Artificial
  Amino acid sequence of point mutated NY-ESO peptide 1F
FLLMWITQC

SEQ ID NO: 122 - protein, 9 aa, Artificial
  Amino acid sequence of point mutated NY-ESO peptide 2M
SMLMWITQC

SEQ ID NO: 123 - protein, 9 aa, Artificial
  Amino acid sequence of point mutated NY-ESO peptide 3A
SLAMWITQC

SEQ ID NO: 124 - protein, 9 aa, Artificial
  Amino acid sequence of point mutated NY-ESO peptide 4A
SLLAWITQC

SEQ ID NO: 125 - protein, 9 aa, Artificial
  Amino acid sequence of point mutated NY-ESO peptide 5A
SLLMAITQC

SEQ ID NO: 126 - protein, 9 aa, Artificial
  Amino acid sequence of point mutated NY-ESO peptide 6L
SLLMWLTQC

SEQ ID NO: 127 - protein, 9 aa, Artificial
  Amino acid sequence of point mutated NY-ESO peptide 7F
SLLMWIFQC

SEQ ID NO: 128 - protein, 9 aa, Artificial
  Amino acid sequence of point mutated NY-ESO peptide 8A
SLLMWITAC

SEQ ID NO: 129 - protein, 9 aa, Artificial
  Amino acid sequence of point mutated NY-ESO peptide 9A
SLLMWITQA

SEQ ID NO: 130 - protein, 9 aa, Artificial
  Amino acid sequence of gp100 peptide
IMDQVPFSV

SEQ ID NO: 131 - protein, 9 aa, Artificial
  Amino acid sequence of homologous peptide DOLPP1
SQFMWFFSV

SEQ ID NO: 132 - protein, 9 aa, Artificial
  Amino acid sequence of homologous peptide IL20RB
SLFMWFFYA

SEQ ID NO: 133 - protein, 9 aa, Artificial
  Amino acid sequence of homologous peptide PRKD2
SLDMWSVGV

SEQ ID NO: 134 - protein, 9 aa, Artificial
  Amino acid sequence of homologous peptide CD163
SIPMWVDNV

SEQ ID NO: 135 - protein, 9 aa, Artificial
  Amino acid sequence of homologous peptide P2RY8
SVAMWAVFL

SEQ ID NO: 136 - protein, 269 aa, Artificial
  Amino acid sequence of C3E-7034
GEVQLVESGGGLVQPGGSLRLSCAASGVTFNYYGMSWIRQAPGKGLEWVASITNSGGRIYYPDSVKGRFTISRENTQKTLYLQMNSLRAEDTAVYYCTLDGRDGWVAYWGQGTLVTVSSGGGGSGGGGSGGGGSNFMLTQPHSVSESPGKTVTISCKRNTGNIGSNYVNWYQQHEGSSPTTIIYRDDKRPDGVSDRFSGSIDRSSKSASLTISNLKTEDEADYFCQSYSSGFIFGGGTKLTVLGAAAGAGGDYKDDDDKGAAAHHHHHH

SEQ ID NO: 137 - protein, 267 aa, Artificial
  Amino acid sequence of C3E-7036
GEVQLVESGGGLVQPGGSLRLSCAASGVTFNYYGMSWIRQAPGKGLEWVASITNSGGRIYYPDSVKGRFTISRENTQKTLYLQMNSLRAEDTAVYYCTLDGRDGWVAYWGQGTLVTVSSGGGGSGGGGSGGGGSNFMLTQPSSVSGVPGQRVTISCTGNTGNIGSNYVNWYQQLPGTAPKLLIYRDDKRPSGVPDRFSGSKSGTSASLAITGFQAEDEADYYCQSYSSGFIFGGGTKLTVLGAAAGAGGDYKDDDDKGAAAHHHHHH

SEQ ID NO: 138 - protein, 267 aa, Artificial
  Amino acid sequence of C3E-7085
GEVQLVESGGGLVQPGGSLRLSCAASGVTFNYYGMSWIRQAPGKGLEWVASITRSGGRIYYPDSVKGRFTISRENTQKTLYLQMNSLRAEDTAVYYCTLDGRDGWVAYWGQGTLVTVSSGGGGSGGGGSGGGGSNFMLTQPSSVSGVPGQRVTISCTGNTGNIGSNYVNWYQQLPGTAPKLLIYRDDKRPSGVPDRFSGSKSGTSASLAITGFQAEDEADYYCQSYSSGFIFGGGTKLTVLGAAAGAGGDYKDDDDKGAAAHHHHHH

SEQ ID NO: 139 - protein, 269 aa, Artificial
  Amino acid sequence of C3E-7088
GEVQLVESGGGLVQPGGSLRLSCAASGVTFNYYGMSWIRQAPGKGLEWVASITRSGGRIYYPDSVKGRFTISRENTQKTLYLQMNSLRAEDTAVYYCTLDGRDGWVAYWGQGTLVTVSSGGGGSGGGGSGGGGSNFMLTQPHSVSESPGKTVTISCKRNTGNIGSNYVNWYQQHEGSSPTTIIYRNDKRPDGVSDRFSGSIDRSSKSASLTISNLKTEDEADYFCQSYSSGFIFGGGTKLTVLGAAAGAGGDYKDDDDKGAAAHHHHHH

SEQ ID NO: 140 - protein, 269 aa, Artificial
  Amino acid sequence of C3E-7093
GEVQLVESGGGLVQPGGSLRLSCAASGVTFNYYGMSWIRQAPGKGLEWVASITSSGGRIYYPDSVKGRFTISRENTQKTLYLQMNSLRAEDTAVYYCTLDGRDGWVAYWGQGTLVTVSSGGGGSGGGGSGGGGSNFMLTQPHSVSESPGKTVTISCKRNTGNIGSNYVNWYQQHEGSSPTTIIYRNDKRPDGVSDRFSGSIDRSSKSASLTISNLKTEDEADYFCQSYSSGFIFGGGTKLTVLGAAAGAGGDYKDDDDKGAAAHHHHHH

SEQ ID NO: 141 - protein, 8 aa, Artificial
  Amino acid sequence of heavy chain CDR1 of C3E-7085
GVTFNYYG

SEQ ID NO: 142 - protein, 8 aa, Artificial
  Amino acid sequence of heavy chain CDR2 of C3E-7085
ITRSGGRI

SEQ ID NO: 143 - protein, 11 aa, Artificial
  Amino acid sequence of heavy chain CDR3 of C3E-7085
TLDGRDGWVAY

SEQ ID NO: 144 - protein, 8 aa, Artificial
  Amino acid sequence of light chain CDR1 of C3E-7085
TGNIGSNY

SEQ ID NO: 145 - protein, 3 aa, Artificial
  Amino acid sequence of light chain CDR2 of C3E-7085
RDD

SEQ ID NO: 146 - protein, 8 aa, Artificial
  Amino acid sequence of light chain CDR3 of C3E-7085
QSYSSGFI

SEQ ID NO: 147 - protein, 269 aa, Artificial
  Amino acid sequence of C3E-7078
GEVQLVESGGGLVQPGGSLRLSCAASGVTFNYYGMSWIRQAPGKGLEWVASITRSGGRIYYPDSVKGRFTISRENTQKTLYLQMNSLRAEDTAVYYCTLDGRDGWVAYWGQGTLVTVSSGGGGSGGGGSGGGGSNFMLTQPHSVSESPGKTVTISCKRNTGNIGSNYVNWYQQHEGSSPTTIIYRDDKRPDGVSDRFSGSIDRSSKSASLTISNLKTEDEADYFCQSYSSGFIFGGGTKLTVLGAAAGAGGDYKDDDDKGAAAHHHHHH

SEQ ID NO: 148 - DNA, 2235 bp, Artificial
  Full-length nucleotide sequence of NYF-0014-HC2
atgaaacacctgtggttcttcctcctgctggtggcagctcccagatgggtgctgagcggagaggtgcagctggtggagtctgggggaggcgtggtccagcctgggaggtccctgacaccctcctgttcagcgtctggattctccatccgtagttatgatatacactgggtccgccaggctccaggcaaggggctagagtgggtggccactatatcatatgatggaagtcagaagtacttcgcagactccgtgaagggccgatttaccatcttcagagacgaatcggagaacatggtgtatctgcaaatgagcggcctgagagttgaggacacggctgtttatcactgtgcgagagggagtagtggtcattatgaggcttttgatatctggggccaagggacaatggtcaccgtctcttcaggtggaggcggttcaggcggaggtggcagcggcggtggcgggagtcagtctgtgttgacgcagccgccctcagtgtctgcggccccaggacagaaggtcaccatctcctgctctggaagcagctccaacattgggaataattatgtatcctggtaccagcagctcccaggaacagcccccaaactcctcatttatgacaataataagcgaccctcagggattcctgaccgattctctggctccaagtctggcacgtcagccaccctgggcatcaccggactccagactggggacgaggccgattattactgcggaacatgggatagcagcctgagtgccccttgggtgttcggcggagggaccaaggtcaccgtcctagggggaggcggttcagaagtgcagctggtggaatccggggggggcctggtgcagcctggggggagcctgagactgagttgtgccgcctctggggtgacatttaactactatggcatgtcttggatccgccaggcacctggaaagggcctggagtgggtggccagcatcactaggtccggcgggcgaatctactatcccgacagcgtcaagggcaggttcacaatttcccgcgagaacacacagaaaactctgtacctgcagatgaatagcctgagagccgaagatacagctgtgtactattgcactctggacggcagggatgggtgggtcgcctattgggggcagggaaccctggtgacagtcagctccggaggaggaggatctggcggaggaggcagtgggggaggcgggtcaaactttatgctcactcagccgtcctctgtttctggcgtacctggccaacgggtgaccattagctgtacgggtaataccgggaatatcgggtctaactacgtgaactggtatcagcagcttccagggacagctcccaagttgctgatctatcgcgacgacaaaagaccctcaggggtccctgaccgatttagtggcagcaaaagcggtacttccgcttccctggcgataaccggctttcaggccgaagatgaggcagactactattgccagtcatattccagcggcttcatcttcggaggcggaactaagctgacagtgttggcagccgagcccaaatcttctgacaaaactcacacatgcccaccctgcccagcacctgaagccgcagggggaccctcagtcttcctcttccccccaaaacccaaggacaccctcatgatctcccggacccctgaggtcacatgcgtggtggtgtcagtgagccacgaagaccctgaggtcaagttcaactggtacgtggacggcgtggaggtgcataatgccaagacaaagccccgggaggagcagtacaacagcacgtaccgggtggtcagcgtcctcaccgtcctgcaccaggactggctgaatggcaaggagtacaagtgcaaggtctccaacaaagccctcccagcccccatcgagaaaaccatctccaaagccaaaggccagccccgggaaccacaggtgtacgtgtaccccccatcccgggacgagctgaccaagaaccaggtcagcctgacctgcctggtcaaaggcttctatcccagcgacatcgccgtggagtgggagagcaatggccagcccgagaacaactacaagaccacccctcccgtgctggactccgacggctccttcgccctcgtgagcaagctcaccgtggacaagagcaggtggcagcagggcaacgtcttctcatgctccgtgatgcatgaggctctgcacaaccactacacccagaagagcctctccctgtctcccggcaag

SEQ ID NO: 149 - protein, 745 aa, Artificial
  Full-length amino acid sequence of NYF-0014-HC2
MKHLWFFLLLVAAPRWVLSGEVQLVESGGGVVQPGRSLTPSCSASGFSIRSYDIHWVRQAPGKGLEWVATISYDGSQKYFADSVKGRFTIFRDESENMVYLQMSGLRVEDTAVYHCARGSSGHYEAFDIWGQGTMVTVSSGGGGSGGGGSGGGGSQSVLTQPPSVSAAPGQKVTISCSGSSSNIGNNYVSWYQQLPGTAPKLLIYDNNKRPSGIPDRFSGSKSGTSATLGITGLQTGDEADYYCGTWDSSLSAPWVFGGGTKVTVLGGGGSEVQLVESGGGLVQPGGSLRLSCAASGVTFNYYGMSWIRQAPGKGLEWVASITRSGGRIYYPDSVKGRFTISRENTQKTLYLQMNSLRAEDTAVYYCTLDGRDGWVAYWGQGTLVTVSSGGGGSGGGGSGGGGSNFMLTQPSSVSGVPGQRVTISCTGNTGNIGSNYVNWYQQLPGTAPKLLIYRDDKRPSGVPDRFSGSKSGTSASLAITGFQAEDEADYYCQSYSSGFIFGGGTKLTVLAAEPKSSDKTHTCPPCPAPEAAGGPSVFLFPPKPKDTLMISRTPEVTCVVVSVSHEDPEVKFNWYVDGVEVHNAKTKPREEQYNSTYRVVSVLTVLHQDWLNGKEYKCKVSNKALPAPIEKTISKAKGQPREPQVYVYPPSRDELTKNQVSLTCLVKGFYPSDIAVEWESNGQPENNYKTTPPVLDSDGSFALVSKLTVDKSRWQQGNVFSCSVMHEALHNHYTQKSLSLSPGK

SEQ ID NO: 150 - protein, 745 aa, Artificial
  Full-length amino acid sequence of NYF-0082-HC2
MKHLWFFLLLVAAPRWVLSGEVQLVESGGGVVQPGRSLTPSCSASGFSIRSYDIHWVRQAPGKGLEWVATISYDGSQKYFADSVKGRFTIFRDESENMVYLQMSGLRVEDTAVYHCARGSSGHYEAFDIWGQGTMVTVSSGGGGSGGGGSGGGGSQSVLTQPPSVSAAPGQKVTISCSGSSSNIGNNYVSWYQRLPGTAPKLLIYDNNKRPSGIPDRFSGSKSGTSATLGITGLQTGDEADYYCGSWDSSLSAPWVFGGGTKVTVLGGGGSEVQLVESGGGLVQPGGSLRLSCAASGVTFNYYGMSWIRQAPGKGLEWVASITRSGGRIYYPDSVKGRFTISRENTQKTLYLQMNSLRAEDTAVYYCTLDGRDGWVAYWGQGTLVTVSSGGGGSGGGGSGGGGSNFMLTQPSSVSGVPGQRVTISCTGNTGNIGSNYVNWYQQLPGTAPKLLIYRDDKRPSGVPDRFSGSKSGTSASLAITGFQAEDEADYYCQSYSSGFIFGGGTKLTVLAAEPKSSDKTHTCPPCPAPEAAGGPSVFLFPPKPKDTLMISRTPEVTCVVVSVSHEDPEVKFNWYVDGVEVHNAKTKPREEQYNSTYRVVSVLTVLHQDWLNGKEYKCKVSNKALPAPIEKTISKAKGQPREPQVYVYPPSRDELTKNQVSLTCLVKGFYPSDIAVEWESNGQPENNYKTTPPVLDSDGSFALVSKLTVDKSRWQQGNVFSCSVMHEALHNHYTQKSLSLSPGK

SEQ ID NO: 151 - protein, 207 aa, Homo sapiens
MQSGTHWRVLGLCLLSVGVWGQDGNEEMGGITQTPYKVSISGTTVILTCPQYPGSEILWQHNDKNIGGDEDDKNIGSDEDHLSLKEFSELEQSGYYVCYPRGSKPEDANFYLYLRARVCENCMEMDVMSVATIVIVDICITGGLLLLVYYWSKNRKAKAKPVTRGAGAGGRQRGQNKERPPPVPNPDYEPIRKGQRDLYSGLNQRRI

SEQ ID NO: 152 - DNA, 2235 bp, Artificial
  Full-length nucleotide sequence of NYZ-0038-HC2
atgaaacacctgtggttcttcctcctgctggtggcagctcccagatgggtgctgagcggtgaggtacagctggtggaatccggtggaggccttgtgcaaccgggaggctccctgcgactctcttgcgccgcatctggcttttccatacgatcctacgatattcattgggtccgacaagcccctggcaaaggtcttgaatgggttgccactatctcctacgacgggtctcagaaatattatgcggattcagtgaaggggcggttcacaatttcacgagacgagtcaaagaatacactgtacctccaaatgaattcactgagagccgaggatactgcagtctatcattgtgcaagagggtcctcaggccactacgaggcctttgatatatggggccaaggcaccttggtaaccgttagtagcggaggtggaggaagcggaggcggcggttccggaggaggtggaagtcaatccgttctgactcagccaccctccgcctctggcaccccgggccaacgggtcacaatatcatgttctggctcttcaagcaacatcggaaactggtacgtgagctggtaccagcagctccccggcacggcgcccaagcttctgatatatgacaacaacaaacggcccagtggagttcctgacagattcagtgggtctaaaagtggtacaagcgctagcctggccataagtggtctgcagagtgaagatgaggcggactattattgcggaacctgggactccagcctgagcgctccctgggttttcggcggaggtactaagctgaccgtcttgggaggaggcggttcagaagtgcagctggtggaatccggggggggcctggtgcagcctggggggagcctgagactgagttgtgccgcctctggggtgacatttaactactatggcatgtcttggatccgccaggcacctggaaagggcctggagtgggtggccagcatcactaggtccggcgggcgaatctactatcccgacagcgtcaagggcaggttcacaatttcccgcgagaacacacagaaaactctgtacctgcagatgaatagcctgagagccgaagatacagctgtgtactattgcactctggacggcagggatgggtgggtcgcctattgggggtgtggaaccctggtgacagtcagctccggaggaggaggatctggcggaggaggcagtgggggaggcgggtcaaactttatgctcactcagccgtcctctgtttctggcgtacctggccaacgggtgaccattagctgtacgggtaataccgggaatatcgggtctaactacgtgaactggtatcagcagcttccagggacatgtcccaagttgctgatctatcgcgacgacaaaagaccctcaggggtccctgaccgatttagtggcagcaaaagcggtacttccgcttccctggcgataaccggctttcaggccgaagatgaggcagactactattgccagtcatattccagcggcttcatcttcggaggcggaactaagctgacagtgttggcagccgagcccaaatcttctgacaaaactcacacatgcccaccctgcccagcacctgaagccgcagggggaccctcagtcttcctcttccccccaaaacccaaggacaccctcatgatctcccggacccctgaggtcacatgcgtggtggtgtcagtgagccacgaagaccctgaggtcaagttcaactggtacgtggacggcgtggaggtgcataatgccaagacaaagccccgggaggagcagtacaacagcacgtaccgggtggtcagcgtcctcaccgtcctgcaccaggactggctgaatggcaaggagtacaagtgcaaggtctccaacaaagccctcccagcccccatcgagaaaaccatctccaaagccaaaggccagccccgggaaccacaggtgtacgtgtaccccccatcccgggacgagctgaccaagaaccaggtcagcctgacctgcctggtcaaaggcttctatcccagcgacatcgccgtggagtgggagagcaatggccagcccgagaacaactacaagaccacccctcccgtgctggactccgacggctccttcgccctcgtgagcaagctcaccgtggacaagagcaggtggcagcagggcaacgtcttctcatgctccgtgatgcatgaggctctgcacaaccactacacccagaagagcctctccctgtctcccggcaag

SEQ ID NO: 153 - DNA, 2250 bp, Artificial
  Full-length nucleotide sequence of NYZ-0082-HC2
atgaaacacctgtggttcttcctcctgctggtggcagctcccagatgggtgctgagcggtgaggtacagctggtggaatccggtggaggccttgtgcaaccgggaggctccctgcgactctcttgcgccgcatctggcttttccatacgatcctacgatattcattgggtccgacaagcccctggcaaaggtcttgaatgggttgccactatctcctacgacgggtctcagaaatattatgcggattcagtgaaggggcggttcacaatttcacgagacgagtcaaagaatacactgtacctccaaatgaattcactgagagccgaggatactgcagtctatcattgtgcaagagggtcctcaggccactacgaggcctttgatatatggggccaaggcaccttggtaaccgttagtagcggaggtggaggaagcggaggcggcggttccggaggaggtggaagtggaggaggtggatctcaatccgttctgactcagccaccctccgcctctggcaccccgggccaacgggtcacaatatcatgttctggctcttcaagcaacatcggaaactggtacgtgagctggtaccagcagctccccggcacggcgcccaagcttctgatatatgacaacaacaaacggcccagtggagttcctgacagattcagtgggtctaaaagtggtacaagcgctagcctggccataagtggtctgcagagtgaagatgaggcggactattattgcggaacctgggactccagcctgagcgctccctgggttttcggcggaggtactaagctgaccgtcttgggaggaggcggttcagaagtgcagctggtggaatccggggggggcctggtgcagcctggggggagcctgagactgagttgtgccgcctctggggtgacatttaactactatggcatgtcttggatccgccaggcacctggaaagggcctggagtgggtggccagcatcactaggtccggcgggcgaatctactatcccgacagcgtcaagggcaggttcacaatttcccgcgagaacacacagaaaactctgtacctgcagatgaatagcctgagagccgaagatacagctgtgtactattgcactctggacggcagggatgggtgggtcgcctattgggggtgtggaaccctggtgacagtcagctccggaggaggaggatctggcggaggaggcagtgggggaggcgggtcaaactttatgctcactcagccgtcctctgtttctggcgtacctggccaacgggtgaccattagctgtacgggtaataccgggaatatcgggtctaactacgtgaactggtatcagcagcttccagggacatgtcccaagttgctgatctatcgcgacgacaaaagaccctcaggggtccctgaccgatttagtggcagcaaaagcggtacttccgcttccctggcgataaccggctttcaggccgaagatgaggcagactactattgccagtcatattccagcggcttcatcttcggaggcggaactaagctgacagtgttggcagccgagcccaaatcttctgacaaaactcacacatgcccaccctgcccagcacctgaagccgcagggggaccctcagtcttcctcttccccccaaaacccaaggacaccctcatgatctcccggacccctgaggtcacatgcgtggtggtgtcagtgagccacgaagaccctgaggtcaagttcaactggtacgtggacggcgtggaggtgcataatgccaagacaaagccccgggaggagcagtacaacagcacgtaccgggtggtcagcgtcctcaccgtcctgcaccaggactggctgaatggcaaggagtacaagtgcaaggtctccaacaaagccctcccagcccccatcgagaaaaccatctccaaagccaaaggccagccccgggaaccacaggtgtacgtgtaccccccatcccgggacgagctgaccaagaaccaggtcagcctgacctgcctggtcaaaggcttctatcccagcgacatcgccgtggagtgggagagcaatggccagcccgagaacaactacaagaccacccctcccgtgctggactccgacggctccttcgccctcgtgagcaagctcaccgtggacaagagcaggtggcagcagggcaacgtcttctcatgctccgtgatgcatgaggctctgcacaaccactacacccagaagagcctctccctgtctcccggcaag

SEQ ID NO: 154 - DNA, 2250 bp, Artificial
  Full-length nucleotide sequence of NYZ-0083-HC2
atgaaacacctgtggttcttcctcctgctggtggcagctcccagatgggtgctgagcggtgaggtacagctggtggaatccggtggaggccttgtgcaaccgggaggctccctgcgactctcttgcgccgcatctggcttttccatacgatcctacgatattcattgggtccgacaagcccctggcaaaggtcttgaatgggttgccactatctcctacgacgggtctcagaaatattatgcggattcagtgaaggggcggttcacaatttcacgagacgagtcaaagaatacactgtacctccaaatgaattcactgagagccgaggatactgcagtctatcattgtgcaagagggtcctcaggccactacgaggcctttgatatatggggccaaggcaccttggtaaccgttagtagcggaggtggaggaagcggaggcggcggttccggaggaggtggaagtggaggaggtggatctcaatccgttctgactcagccaccctccgcctctggcaccccgggccaacgggtcacaatatcatgttctggctcttcaagcaacatcggaaactggtacgtgagctggtaccagcagctccccggcacggcgcccaagcttctgatatatgacaacaacaaacggcccagtggagttcctgacagattcagtgggtctaaaagtggtacaagcgctagcctggccataagtggtctgcagagtgaagatgaggcggactattattgcggaacctgggactccagcctgagcgctccctgggttttcggcggaggtactaagctgaccgtcttgggaggaggcggttcagaagtgcagctggtggaatccggggggggcctggtgcagcctggggggagcctgagactgagttgtgccgcctctggggtgacatttaactactatggcatgtcttggatccgccaggcacctggaaagtgtctggagtgggtggccagcatcactaggtccggcgggcgaatctactatcccgacagcgtcaagggcaggttcacaatttcccgcgagaacacacagaaaactctgtacctgcagatgaatagcctgagagccgaagatacagctgtgtactattgcactctggacggcagggatgggtgggtcgcctattgggggcagggaaccctggtgacagtcagctccggaggaggaggatctggcggaggaggcagtgggggaggcgggtcaaactttatgctcactcagccgtcctctgtttctggcgtacctggccaacgggtgaccattagctgtacgggtaataccgggaatatcgggtctaactacgtgaactggtatcagcagcttccagggacagctcccaagttgctgatctatcgcgacgacaaaagaccctcaggggtccctgaccgatttagtggcagcaaaagcggtacttccgcttccctggcgataaccggctttcaggccgaagatgaggcagactactattgccagtcatattccagcggcttcatcttcggatgtggaactaagctgacagtgttggcagccgagcccaaatcttctgacaaaactcacacatgcccaccctgcccagcacctgaagccgcagggggaccctcagtcttcctcttccccccaaaacccaaggacaccctcatgatctcccggacccctgaggtcacatgcgtggtggtgtcagtgagccacgaagaccctgaggtcaagttcaactggtacgtggacggcgtggaggtgcataatgccaagacaaagccccgggaggagcagtacaacagcacgtaccgggtggtcagcgtcctcaccgtcctgcaccaggactggctgaatggcaaggagtacaagtgcaaggtctccaacaaagccctcccagcccccatcgagaaaaccatctccaaagccaaaggccagccccgggaaccacaggtgtacgtgtaccccccatcccgggacgagctgaccaagaaccaggtcagcctgacctgcctggtcaaaggcttctatcccagcgacatcgccgtggagtgggagagcaatggccagcccgagaacaactacaagaccacccctcccgtgctggactccgacggctccttcgccctcgtgagcaagctcaccgtggacaagagcaggtggcagcagggcaacgtcttctcatgctccgtgatgcatgaggctctgcacaaccactacacccagaagagcctctccctgtctcccggcaag

SEQ ID NO: 155 - protein, 745 aa, Artificial
  Full-length amino acid sequence of NYZ-0038-HC2
MKHLWFFLLLVAAPRWVLSGEVQLVESGGGLVQPGGSLRLSCAASGFSIRSYDIHWVRQAPGKGLEWVATISYDGSQKYYADSVKGRFTISRDESKNTLYLQMNSLRAEDTAVYHCARGSSGHYEAFDIWGQGTLVTVSSGGGGSGGGGSGGGGSQSVLTQPPSASGTPGQRVTISCSGSSSNIGNWYVSWYQQLPGTAPKLLIYDNNKRPSGVPDRFSGSKSGTSASLAISGLQSEDEADYYCGTWDSSLSAPWVFGGGTKLTVLGGGGSEVQLVESGGGLVQPGGSLRLSCAASGVTFNYYGMSWIRQAPGKGLEWVASITRSGGRIYYPDSVKGRFTISRENTQKTLYLQMNSLRAEDTAVYYCTLDGRDGWVAYWGCGTLVTVSSGGGGSGGGGSGGGGSNFMLTQPSSVSGVPGQRVTISCTGNTGNIGSNYVNWYQQLPGTCPKLLIYRDDKRPSGVPDRFSGSKSGTSASLAITGFQAEDEADYYCQSYSSGFIFGGGTKLTVLAAEPKSSDKTHTCPPCPAPEAAGGPSVFLFPPKPKDTLMISRTPEVTCVVVSVSHEDPEVKFNWYVDGVEVHNAKTKPREEQYNSTYRVVSVLTVLHQDWLNGKEYKCKVSNKALPAPIEKTISKAKGQPREPQVYVYPPSRDELTKNQVSLTCLVKGFYPSDIAVEWESNGQPENNYKTTPPVLDSDGSFALVSKLTVDKSRWQQGNVFSCSVMHEALHNHYTQKSLSLSPGK

SEQ ID NO: 156 - protein, 750 aa, Artificial
  Full-length amino acid sequence of NYZ-0082-HC2
MKHLWFFLLLVAAPRWVLSGEVQLVESGGGLVQPGGSLRLSCAASGFSIRSYDIHWVRQAPGKGLEWVATISYDGSQKYYADSVKGRFTISRDESKNTLYLQMNSLRAEDTAVYHCARGSSGHYEAFDIWGQGTLVTVSSGGGGSGGGGSGGGGSGGGGSQSVLTQPPSASGTPGQRVTISCSGSSSNIGNWYVSWYQQLPGTAPKLLIYDNNKRPSGVPDRFSGSKSGTSASLAISGLQSEDEADYYCGTWDSSLSAPWVFGGGTKLTVLGGGGSEVQLVESGGGLVQPGGSLRLSCAASGVTFNYYGMSWIRQAPGKGLEWVASITRSGGRIYYPDSVKGRFTISRENTQKTLYLQMNSLRAEDTAVYYCTLDGRDGWVAYWGCGTLVTVSSGGGGSGGGGSGGGGSNFMLTQPSSVSGVPGQRVTISCTGNTGNIGSNYVNWYQQLPGTCPKLLIYRDDKRPSGVPDRFSGSKSGTSASLAITGFQAEDEADYYCQSYSSGFIFGGGTKLTVLAAEPKSSDKTHTCPPCPAPEAAGGPSVFLFPPKPKDTLMISRTPEVTCVVVSVSHEDPEVKFNWYVDGVEVHNAKTKPREEQYNSTYRVVSVLTVLHQDWLNGKEYKCKVSNKALPAPIEKTISKAKGQPREPQVYVYPPSRDELTKNQVSLTCLVKGFYPSDIAVEWESNGQPENNYKTTPPVLDSDGSFALVSKLTVDKSRWQQGNVFSCSVMHEALHNHYTQKSLSLSPGK

SEQ ID NO: 157 - protein, 750 aa, Artificial
  Full-length amino acid sequence of NYZ-0083-HC2
MKHLWFFLLLVAAPRWVLSGEVQLVESGGGLVQPGGSLRLSCAASGFSIRSYDIHWVRQAPGKGLEWVATISYDGSQKYYADSVKGRFTISRDESKNTLYLQMNSLRAEDTAVYHCARGSSGHYEAFDIWGQGTLVTVSSGGGGSGGGGSGGGGSGGGGSQSVLTQPPSASGTPGQRVTISCSGSSSNIGNWYVSWYQQLPGTAPKLLIYDNNKRPSGVPDRFSGSKSGTSASLAISGLQSEDEADYYCGTWDSSLSAPWVFGGGTKLTVLGGGGSEVQLVESGGGLVQPGGSLRLSCAASGVTFNYYGMSWIRQAPGKCLEWVASITRSGGRIYYPDSVKGRFTISRENTQKTLYLQMNSLRAEDTAVYYCTLDGRDGWVAYWGQGTLVTVSSGGGGSGGGGSGGGGSNFMLTQPSSVSGVPGQRVTISCTGNTGNIGSNYVNWYQQLPGTAPKLLIYRDDKRPSGVPDRFSGSKSGTSASLAITGFQAEDEADYYCQSYSSGFIFGCGTKLTVLAAEPKSSDKTHTCPPCPAPEAAGGPSVFLFPPKPKDTLMISRTPEVTCVVVSVSHEDPEVKFNWYVDGVEVHNAKTKPREEQYNSTYRVVSVLTVLHQDWLNGKEYKCKVSNKALPAPIEKTISKAKGQPREPQVYVYPPSRDELTKNQVSLTCLVKGFYPSDIAVEWESNGQPENNYKTTPPVLDSDGSFALVSKLTVDKSRWQQGNVFSCSVMHEALHNHYTQKSLSLSPGK

SEQ ID NO: 158 - DNA, 2172 bp, Artificial
  Full-length nucleotide sequence of NYZ-1010-HC2
atgaaacacctgtggttcttcctcctgctggtggcagctcccagatgggtgctgagcggtgaggtacagctggtggaatccggtggaggccttgtgcaaccgggaggctccctgcgactctcttgcgccgcatctggcttttccatacgatcctacgatattcattgggtccgacaagcccctggcaaaggtcttgaatgggttgccactatctcctacgacgggtctcagaaatattatgcggattcagtgaaggggcggttcacaatttcacgagacgagtcaaagaatacactgtacctccaaatgaattcactgagagccgaggatactgcagtctatcattgtgcaagagggtcctcaggccactacgaggcctttgatatatggggccaaggcaccttggtaaccgttagtagcggaggtggaggaagcggaggcggcggttccggaggaggtggaagtggaggaggtggatctcaatccgttctgactcagccaccctccgcctctggcaccccgggccaacgggtcacaatatcatgttctggctcttcaagcaacatcggaaactggtacgtgagctggtaccagcagctccccggcacggcgcccaagcttctgatatatgacaacaacaaacggcccagtggagttcctgacagattcagtgggtctaaaagtggtacaagcgctagcctggccataagtggtctgcagagtgaagatgaggcggactattattgcggaacctgggactccagcctgagcgctccctgggttttcggcggaggtactaagctgaccgtcttgggaggaggcggttcagaagtgcagctggtggaatccggggggggcctggtgcagcctggggggagcctgagactgagttgtgccgcctctggggtgacatttaactactatggcatgtcttggatccgccaggcacctggaaagggcctggagtgggtggccagcatcactaggtccggcgggcgaatctactatcccgacagcgtcaagggcaggttcacaatttcccgcgagaacacacagaaaactctgtacctgcagatgaatagcctgagagccgaagatacagctgtgtactattgcactctggacggcagggatgggtgggtcgcctattggggtcagggaaccctggtgacagtcagctccgcctccaccaagggcccaagcgtcttccccctggcaccctcctccaagagcacctctggcggcacagccgccctgggctgcctggtcaaggactacttccccgaacccgtgaccgtgagctggaactcaggcgccctgaccagcggcgtgcacaccttccccgctgtcctgcagtcctcaggactctactccctcagcagcgtggtgaccgtgccctccagcagcttgggcacccagacctacatctgcaacgtgaatcacaagcccagcaacaccaaggtggacaagagagttgagcccaagtcttgcgacaaaactcacacatgcccaccctgcccagcacctgaagccgcagggggaccctcagtcttcctcttccccccaaaacccaaggacaccctcatgatctcccggacccctgaggtcacatgcgtggtggtgtcagtgagccacgaagaccctgaggtcaagttcaactggtacgtggacggcgtggaggtgcataatgccaagacaaagccccgggaggagcagtacaacagcacgtaccgggtggtcagcgtcctcactgtcctgcaccaggactggctgaatggcaaggagtacaagtgcaaggtctccaacaaagccctcccagcccccatcgagaaaaccatctccaaagccaaaggccagccccgggaaccacaggtgtacgtgtaccccccatcccgggacgagctgaccaagaaccaggtcagcctgacctgcctggtcaaaggcttctatcccagcgacatcgccgtggagtgggagagcaatggccagcccgagaacaactacaagaccacccctcccgtgctggactccgacggctccttcgccctcgtgagcaagctcaccgtggacaagagcaggtggcagcagggcaacgtcttctcatgctccgtgatgcatgaggctctgcacaaccactacacccagaagagcctctccctgtctcccggcaag

SEQ ID NO: 159 - DNA, 699 bp, Artificial
  Full-length nucleotide sequence of C3E-7085-LC
atggtgctgcagacccaggtgttcatctccctgctgctgtggatctccggcgcgtacggcaactttatgctcactcagccgtcctctgtttctggcgtacctggccaacgggtgaccattagctgtacgggtaataccgggaatatcgggtctaactacgtgaactggtatcagcagcttccagggacagctcccaagttgctgatctatcgcgacgacaaaagaccctcaggggtccctgaccgatttagtggcagcaaaagcggtacttccgcttccctggcgataaccggctttcaggccgaagatgaggcagactactattgccagtcatattccagcggcttcatcttcggaggcggaactaagctgacagtgctgggccagcctaaggctgcccctagcgtgaccctgttccctccttccagcgaggagcttcaagctaacaaggccaccctggtgtgtcttatctctgacttctaccctggcgctgtgaccgtggcctggaaggctgacagctcccctgtgaaggccggagtggagaccaccacacctagcaagcagtctaacaacaagtacgctgccagctcctacctgagccttacccctgagcagtggaagtctcacagaagctactcctgtcaagtgacccacgagggcagcaccgtggagaagaccgtggctcctaccgagtgttcc

SEQ ID NO: 160 - protein, 724 aa, Artificial
  Full-length amino acid sequence of NYZ-1010-HC2
MKHLWFFLLLVAAPRWVLSGEVQLVESGGGLVQPGGSLRLSCAASGFSIRSYDIHWVRQAPGKGLEWVATISYDGSQKYYADSVKGRFTISRDESKNTLYLQMNSLRAEDTAVYHCARGSSGHYEAFDIWGQGTLVTVSSGGGGSGGGGSGGGGSGGGGSQSVLTQPPSASGTPGQRVTISCSGSSSNIGNWYVSWYQQLPGTAPKLLIYDNNKRPSGVPDRFSGSKSGTSASLAISGLQSEDEADYYCGTWDSSLSAPWVFGGGTKLTVLGGGGSEVQLVESGGGLVQPGGSLRLSCAASGVTFNYYGMSWIRQAPGKGLEWVASITRSGGRIYYPDSVKGRFTISRENTQKTLYLQMNSLRAEDTAVYYCTLDGRDGWVAYWGQGTLVTVSSASTKGPSVFPLAPSSKSTSGGTAALGCLVKDYFPEPVTVSWNSGALTSGVHTFPAVLQSSGLYSLSSVVTVPSSSLGTQTYICNVNHKPSNTKVDKRVEPKSCDKTHTCPPCPAPEAAGGPSVFLFPPKPKDTLMISRTPEVTCVVVSVSHEDPEVKFNWYVDGVEVHNAKTKPREEQYNSTYRVVSVLTVLHQDWLNGKEYKCKVSNKALPAPIEKTISKAKGQPREPQVYVYPPSRDELTKNQVSLTCLVKGFYPSDIAVEWESNGQPENNYKTTPPVLDSDGSFALVSKLTVDKSRWQQGNVFSCSVMHEALHNHYTQKSLSLSPGK

SEQ ID NO: 161 - protein, 233 aa, Artificial
  Full-length amino acid sequence of C3E-7085-LC
MVLQTQVFISLLLWISGAYGNFMLTQPSSVSGVPGQRVTISCTGNTGNIGSNYVNWYQQLPGTAPKLLIYRDDKRPSGVPDRFSGSKSGTSASLAITGFQAEDEADYYCQSYSSGFIFGGGTKLTVLGQPKAAPSVTLFPPSSEELQANKATLVCLISDFYPGAVTVAWKADSSPVKAGVETTTPSKQSNNKYAASSYLSLTPEQWKSHRSYSCQVTHEGSTVEKTVAPTECS

SEQ ID NO: 162 - protein, 5 aa, Artificial
  Peptide linker
GGGGS

SEQ ID NO: 163 - DNA, 891 bp, Artificial
  Full-length nucleotide sequence of NYA-3061
atgaaacacctgtggttcttcctcctgctggtggcagctcccagatgggtgctgagcggtgaggtacagctggtggaatccggtggaggccttgtgcaaccgggaggctccctgcgactctcttgcgccgcatctggcttttccatacgatcctacgatattcattgggtccgacaagcccctggcaaaggtcttgaatgggttgccactatctcctacgacgggtctcagaaatattatgcggattcagtgaaggggcggttcacaatttcacgagacgagtcaaagaatacactgtacctccaaatgaattcactgagagccgaggatactgcagtctatcattgtgcaagagggtcctcaggccactacgaggcctttgatatatggggccaaggcaccttggtaaccgttagtagcggaggtggaggaagcggaggcggcggttccggaggaggtggaagtggaggaggtggatctcaatccgttctgactcagccaccctccgcctctggcaccccgggccaacgggtcacaatatcatgttctggctcttcaagcaacatcggaaactggtacgtgagctggtaccagcagctccccggcacggcgcccaagcttctgatatatgacaacaacaaacggcccagtggagttcctgacagattcagtgggtctaaaagtggtacaagcgctagcctggccataagtggtctgcagagtgaagatgaggcggactattattgcggaacctgggactccagcctgagcgctccctgggttttcggcggaggtactaagctgaccgtcttgggcgcggccgcaggtgcaggtggtgattacaaagatgatgacgataaaggtgcagcggcgcatcaccatcatcaccac

SEQ ID NO: 164 - protein, 297 aa, Artificial
  Full-length amino acid sequence of NYA-3061
MKHLWFFLLLVAAPRWVLSGEVQLVESGGGLVQPGGSLRLSCAASGFSIRSYDIHWVRQAPGKGLEWVATISYDGSQKYYADSVKGRFTISRDESKNTLYLQMNSLRAEDTAVYHCARGSSGHYEAFDIWGQGTLVTVSSGGGGSGGGGSGGGGSGGGGSQSVLTQPPSASGTPGQRVTISCSGSSSNIGNWYVSWYQQLPGTAPKLLIYDNNKRPSGVPDRFSGSKSGTSASLAISGLQSEDEADYYCGTWDSSLSAPWVFGGGTKLTVLGAAAGAGGDYKDDDDKGAAAHHHHHH

SEQ ID NO: 165 - DNA, 903 bp, Artificial
  Full-length nucleotide sequence of NYC-0005
atgaagcacctgtggttctttctgctgctggtggccgctcctagatgggtgttgtctggcgaagtgcagctggtggaatctggtggcggagttgttcagcctggcggctctctgagactgagctgtgtggccagcggcttcaccttcgacgactacgccatgtactgggtccgacaggtgccaggcaaggacctggaatgggtgtccctgatttctggcgacggcgacatcacctactacgtggactctgtgaagggcagattcaccgtgtccagagacaacaacaagaacagcctgtacctgcagatgaagtccctgcgcgtggaagatacagccctgtactactgcgccaaggacatgatctactacgcctcttggagcggctacggcagcagcgattactactactatgtgatggacgtgtggggccagggcaccaccgttacagtttctagcggaggcggaggaagtggcggcggaggatctggcggtggtggttctgatatccagatgacacagagccccagcagcctgtctgcctctgtgggagacagagtgaccatcacctgtagagccagccagagcatcagcagctacctgaactggtatcagcagaagcccggcaaggcccctaaactgctgatctatgccgcctccagtctgcagagcggagtgcctagcagattttctggcagcggctccggcaccgatttcaccctgaccatatctagcctgcagcctgaggacttcgccacctactattgccagcagagctacagcacccctcctatcacctttggccagggaaccagactggaaatcaaaggcgctgctgcaggcgctggcggcgactacaaagacgatgatgataagggcgctgccgctcaccaccaccatcaccat

SEQ ID NO: 166 - protein, 301 aa, Artificial
  Full-length amino acid sequence of NYC-0005
MKHLWFFLLLVAAPRWVLSGEVQLVESGGGVVQPGGSLRLSCVASGFTFDDYAMYWVRQVPGKDLEWVSLISGDGDITYYVDSVKGRFTVSRDNNKNSLYLQMKSLRVEDTALYYCAKDMIYYASWSGYGSSDYYYYVMDVWGQGTTVTVSSGGGGSGGGGSGGGGSDIQMTQSPSSLSASVGDRVTITCRASQSISSYLNWYQQKPGKAPKLLIYAASSLQSGVPSRFSGSGSGTDFTLTISSLQPEDFATYYCQQSYSTPPITFGQGTRLEIKGAAAGAGGDYKDDDDKGAAAHHHHHH

SEQ ID NO: 167 - DNA, 903 bp, Artificial
  Full-length nucleotide sequence of NYC-0006
atgaagcacctgtggttctttctgctgctggtggccgctcctagatgggtgttgtctggcgaagtgcagctggtggaatctggtggcggagttgttcagcctggcggctctctgagactgtcttgtgccgccagcggcttcaccttcgacgactacgccatgtactgggtccgacaggcccctggcaaaggccttgaatgggtgtccctgatcagcggagatggcggcagcatgtactacgccgatagcgtgaagggcagattcaccatcagccgggacaacagcaagaacagcctgtacctgcagatgaactccctgcggaccgaggacacagccctgtactactgcgccaaggatatgatcttctacgccttttggagcggctacggcagcagcgattactactactacgtgatggacgtgtggggccagggcaccacagtgacagtttattctggcggcggaggatctggcggaggtggaagcggaggcggtggatctgatatccagatgacacagagccccagcagcctgtctgcctctgtgggagacagagtgaccatcacctgtcgggccagccagagaatcagcacctacctgaactggtatcagcagaagcccggcaaggcccctaagctgctgatctatgctgcctccagtctgcagagcggcgtgccaagcagattttctggcagcggctctggcaccgacttcaccctgaccatatctagcctgcagcctgaggacttcgccacctactactgccagcagagctacagcacccctcctatcacctttggccagggaaccagactggaaatcaaaggcgctgctgcaggcgcaggcggcgactacaaagacgatgatgataagggcgctgccgctcaccaccaccatcaccat

SEQ ID NO: 168 - protein, 301 aa, Artificial
  Full-length amino acid sequence of NYC-0006
MKHLWFFLLLVAAPRWVLSGEVQLVESGGGVVQPGGSLRLSCAASGFTFDDYAMYWVRQAPGKGLEWVSLISGDGGSMYYADSVKGRFTISRDNSKNSLYLQMNSLRTEDTALYYCAKDMIFYAFWSGYGSSDYYYYVMDVWGQGTTVTVYSGGGGSGGGGSGGGGSDIQMTQSPSSLSASVGDRVTITCRASQRISTYLNWYQQKPGKAPKLLIYAASSLQSGVPSRFSGSGSGTDFTLTISSLQPEDFATYYCQQSYSTPPITFGQGTRLEIKGAAAGAGGDYKDDDDKGAAAHHHHHH

SEQ ID NO: 169 - DNA, 888 bp, Artificial
  Full-length nucleotide sequence of NYC-0007
atgaagcacctgtggttctttctgctgctggtggccgctcctagatgggtgttgtctggcgaagtgcagctggtggaatctggtggcggagttgttcagcctggcggctctctgagactgtcttgtgccgccagcggcttcaccttcgacgattatgccatgcactgggtccgacaggcccctggcaaaggacttgaatgggtgtccctgatcagcggcgacggcgacaatacctactacgccgatagcgtgaagggcagattcaccatcagccgggacaacaacaagaacagcctgtacctgcagatgaactccctgcggaccgaggacaccgccttctactactgtgccaaagagctgatcttcggcaaggtgctgcacgacttttactactacgtgatggacgtgtggggccagggcaccacagtgacagtttctagcggaggcggaggaagtggcggcggaggatctggcggtggtggttctgatatccagatgacacagagccccagcagcctgtctgcctctgtgggagacagagtgaccatcacctgtagagccagccagagcatcagcagctacctgaactggtatcagcagaagcccggcaaggcccctaaactgctgatctatgccgcctccagtctgcagagcggagtgcctagcagattttctggcagcggctccggcaccgatttcaccctgaccatatctagcctgcagcctgaggacttcgccacctactactgccagcagagctacagcacccctcctatcacctttggccagggaaccagactggaaatcaaaggcgctgctgcaggcgcaggcggcgactacaaagacgatgatgataagggcgctgccgctcaccaccaccatcaccat

SEQ ID NO: 170 - protein, 296 aa, Artificial
  Full-length amino acid sequence of NYC-0007
MKHLWFFLLLVAAPRWVLSGEVQLVESGGGVVQPGGSLRLSCAASGFTFDDYAMHWVRQAPGKGLEWVSLISGDGDNTYYADSVKGRFTISRDNNKNSLYLQMNSLRTEDTAFYYCAKELIFGKVLHDFYYYVMDVWGQGTTVTVSSGGGGSGGGGSGGGGSDIQMTQSPSSLSASVGDRVTITCRASQSISSYLNWYQQKPGKAPKLLIYAASSLQSGVPSRFSGSGSGTDFTLTISSLQPEDFATYYCQQSYSTPPITFGQGTRLEIKGAAAGAGGDYKDDDDKGAAAHHHHHH

SEQ ID NO: 171 - DNA, 888 bp, Artificial
  Full-length nucleotide sequence of NYC-0008
atgaagcacctgtggttctttctgctgctggtggccgctcctagatgggtgttgtctggcgaagtgcagctggtggaatctggtggcggagttgttcagcctggcggctctctgagactgagctgtgaagcctccggcttcatcttcgacgactacgccatgcactgggtccgacaggcacctggcaaaggccttgaatgggtgtccctgatctctggcgacggcgacatcatctactacgccgactctgtgaagggcagattcaccatcagccgggacaacagcaagaacagcctgtacctgcagatgaactccctgatcatcgaggacacagccctgtactactgcgccaaggattgggtgttcggcgtcgtgatgacccactactggtacttcggcctggatgtgtggggccagggaaccacagtgacagtttctagcggaggcggaggaagtggcggcggaggatctggcggtggtggttctgatatccagatgacacagagccccagcagcctgtctgcctctgaaggcgacagagtgaccatcacctgtagagccagccagagcatcagcacctacctgaactggtatcagcagaagcccggcaaggcccctaagctgctgatctatggtgcctccagtctgcagagcggcgtgccaagcagattttctggcagcggctctggcaccgacttcaccctgaccatatctagcctgcagcctgaggacttcgccacctactactgccagcagtcctacagcacccctcctatcacatttggccagggcaccaaggtggaaatcaaaggcgctgctgcaggcgctggcggcgactacaaagacgatgatgataagggcgctgccgctcaccaccaccatcaccat

SEQ ID NO: 172 - protein, 296 aa, Artificial
  Full-length amino acid sequence of NYC-0008
MKHLWFFLLLVAAPRWVLSGEVQLVESGGGVVQPGGSLRLSCEASGFIFDDYAMHWVRQAPGKGLEWVSLISGDGDIIYYADSVKGRFTISRDNSKNSLYLQMNSLIIEDTALYYCAKDWVFGVVMTHYWYFGLDVWGQGTTVTVSSGGGGSGGGGSGGGGSDIQMTQSPSSLSASEGDRVTITCRASQSISTYLNWYQQKPGKAPKLLIYGASSLQSGVPSRFSGSGSGTDFTLTISSLQPEDFATYYCQQSYSTPPITFGQGTKVEIKGAAAGAGGDYKDDDDKGAAAHHHHHH

SEQ ID NO: 173 - DNA, 885 bp, Artificial
  Full-length nucleotide sequence of NYC-0009
atgaagcacctgtggttctttctgctgctggtggccgctcctagatgggtgttgtctggcgaagtgcagctggtggaatctggtggcggagttgttcagcctggcggctctctgagactgtcttgtgccgccagcggcttcaccttcgacgattatgccatgcactgggtccgacaggcccctggcaaaggacttgaatgggtgtccctgatctctggcggaggcggcggaacctactacagcgattctgtgaagggcagattcaccatcagccgggacaccagcaaggacagcctgtacctgcagatgaacagcctgcggaccgaggacacagccctgtactactgcgccaaggacatggtgttcggcgtggtcaccccttactactacttcgccctggatgtgtggggccagggcacaacagtgacagtctcttctggcggcggaggaagcggaggcggaggatccggtggtggtggatctgacatccagatgacacagagccccagcagcctgtctgcctctgtgggagacagagtgaccatcacctgtagagccagccagagcatcaacagctacctgaactggtatcagcagaagcccggcaaggcccctaagctgctgatctatgctgcctccagtctgcagagcggcgtgccaagcagattttctggcagcggctctggcaccgacttcaccctgaccatatctagcctgcagcctgaggacttcgccacctactactgccagcagagctacagcgcccctcctatcacatttggccagggaaccagactggaaatcaaaggcgctgctgcaggcgcaggcggcgactacaaagacgatgatgataagggcgctgccgctcaccaccatcaccatcat

SEQ ID NO: 174 - protein, 295 aa, Artificial
  Full-length amino acid sequence of NYC-0009
MKHLWFFLLLVAAPRWVLSGEVQLVESGGGVVQPGGSLRLSCAASGFTFDDYAMHWVRQAPGKGLEWVSLISGGGGGTYYSDSVKGRFTISRDTSKDSLYLQMNSLRTEDTALYYCAKDMVFGVVTPYYYFALDVWGQGTTVTVSSGGGGSGGGGSGGGGSDIQMTQSPSSLSASVGDRVTITCRASQSINSYLNWYQQKPGKAPKLLIYAASSLQSGVPSRFSGSGSGTDFTLTISSLQPEDFATYYCQQSYSAPPITFGQGTRLEIKGAAAGAGGDYKDDDDKGAAAHHHHHH

SEQ ID NO: 175 - DNA, 888 bp, Artificial
  Full-length nucleotide sequence of NYC-0010
atgaagcacctgtggttctttctgctgctggtggccgctcctagatgggtgttgtctggcgaagtgcagctggtggaatctggtggcggagttgttcagcctggcggctctctgagactgagctgtgctgtgtccggcttcaccttcgacgactacgccatgcactgggtccgacaggcacctggcaaaggccttgaatgggtgtccctgatcagcggagatggcggcagcacacactacgccgattctgtgaagggcagattcaccatcagccgggacaacagcaagaacagcctgtacctgcagatgaactccctgcggacaggcgacacagccctgtactactgcgccaaggacatgatcttcgccgtggtcatcaccgactaccactactacggcatggacgtgtggggccagggaaccacagtgacagtttctagcggaggcggaggaagtggcggcggaggatctggcggtggtggttctgatatccagatgacacagagccccagcagcctgtctgcctctgtgggagacagagtgaccatcacctgtagagccagccagagcatcagcagctacctgaactggtatcagcagaagcccggcaaggcccctaaactgctgatctatgccgcctccagtctgcagagcggagtgcctagcagattttctggcagcggctccggcaccgatttcaccctgaccatatctagcctgcagcctgaggacttcgccacctactactgccagcagagctacagcacccctcctatcacctttggccagggcaccagactggaaatcaaaggcgctgctgcaggcgctggcggcgactacaaagacgatgatgataagggcgctgccgctcaccaccaccatcaccat

SEQ ID NO: 176 - protein, 296 aa, Artificial
  Full-length amino acid sequence of NYC-0010
MKHLWFFLLLVAAPRWVLSGEVQLVESGGGVVQPGGSLRLSCAVSGFTFDDYAMHWVRQAPGKGLEWVSLISGDGGSTHYADSVKGRFTISRDNSKNSLYLQMNSLRTGDTALYYCAKDMIFAVVITDYHYYGMDVWGQGTTVTVSSGGGGSGGGGSGGGGSDIQMTQSPSSLSASVGDRVTITCRASQSISSYLNWYQQKPGKAPKLLIYAASSLQSGVPSRFSGSGSGTDFTLTISSLQPEDFATYYCQQSYSTPPITFGQGTRLEIKGAAAGAGGDYKDDDDKGAAAHHHHHH

SEQ ID NO: 177 - DNA, 738 bp, Artificial
  Full-length nucleotide sequence of HC-h
atgaaacacctgtggttcttcctcctgctggtggcagctcccagatgggtgctgagcgacaaaactcacacatgcccaccctgcccagcacctgaagccgccggcggaccctcagtcttcctcttccccccaaaacccaaggacaccctcatgatctcccggacccctgaggtcacatgcgtggtggtggacgtgagccacgaagaccctgaggtcaagttcaactggtacgtggacggcgtggaggtgcataatgccaagaccaagcctagagaggaacagtacaacagcacctaccgggtggtgtccgtgctgacagtgctgcaccaggactggctgaacggcaaagagtacaagtgcaaggtgtccaacaaggccctgcctgcccccatcgagaaaaccatcagcaaggccaagggccagccccgcgaacctcaagtgtgcaccctgccaccctcccgggatgagctgaccaagaaccaggtgtccctgagctgtgccgtgaagggcttctacccctccgatatcgccgtggaatgggagagcaacggccagcccgagaacaactacaagaccaccccccctgtgctggacagcgacggctcattcttcctggtgtccaagctgaccgtggacaagtccagatggcagcagggcaacgtcttctcatgctccgtgatgcatgaggctctgcacaaccactacacccagaagagcctctccctgtctcccggcaaa

SEQ ID NO: 178 - protein, 246 aa, Artificial
  Full-length amino acid sequence of HC-h
MKHLWFFLLLVAAPRWVLSDKTHTCPPCPAPEAAGGPSVFLFPPKPKDTLMISRTPEVTCVVVDVSHEDPEVKFNWYVDGVEVHNAKTKPREEQYNSTYRVVSVLTVLHQDWLNGKEYKCKVSNKALPAPIEKTISKAKGQPREPQVCTLPPSRDELTKNQVSLSCAVKGFYPSDIAVEWESNGQPENNYKTTPPVLDSDGSFFLVSKLTVDKSRWQQGNVFSCSVMHEALHNHYTQKSLSLSPGK

SEQ ID NO: 179 - DNA, 1500 bp, Artificial
  Full-length nucleotide sequence of NYD-2047-HC-k
atgaagcacctgtggttctttctgctgctggtggccgctcctagatgggtgctgtctggtcaagtacagctggtggaatccggtggaggcgtggtccagccgggacgcagcttgagactgtcctgcgctgcatctggcttttccatacgatcctacgatatgcactgggttcgccaagcccctggcaaaggtcttgaatgggttgccactatctcctacgacgggtctcagaaatattacgcggattcagtgaaggggcggttcacaatttcacgggacaattcaaagaataccttgtatctccagatgtcttcactgagagccgaggatactgcagtctatcattgtgcaagagggtcctcaggccactacgaggcctttgatatatggggccaaggcaccttggtaaccgttagtagcggaggtggaggaagcggaggcggcggttccggaggaggtggaagtcaatccgttctgactcagccaccctccgtgagtgcagcgcctggacagaaggtcacaatatcatgttctggctcttcaagcaacatcggaaactggtacgtgagctggtaccagcagctccccggcacggcgcccaagcttctgatatatgacaacaacaaacggcccagtggaatccctgacagattcagtgggtctaaaagtggtacaagcgctaccctgggtatcaccggattgcagaccggagatgaggcggactattattgcggaacctgggactccagcctgagcgctccctgggttttcggcggaggtactaaggttaccgtcttgggcggagaacccaagagcgcagacaagacccacacctgtcctccatgtcctgctccagaagctgcaggcggcccttccgtgtttctgttccctccaaagcctaaggacaccctgatgatcagccggacacctgaagtgacctgcgtggtggtggatgtgtcccacgaggatcccgaagtgaagttcaattggtacgtggacggcgtggaagtgcacaacgccaagaccaagcctagagaggaacagtacaacagcacctacagagtggtgtctgtgctgacagtgctgcaccaggactggctgaacggcaaagagtacaagtgcaaggtgtccaacaaggccctgcctgctcctatcgagaaaaccatcagcaaggccaagggccagcctagggaaccccaggtttacaccctgcctccatgcagggatgagctgaccaagaaccaggtgtccctgtggtgcctggttaagggcttctacccctccgatatcgccgtggaatgggagagcaatggccagccagagaacaactacaagacaacccctcctgtgctggactccgacggctcattcttcctgtacagcaagctgaccgtggacaagagcagatggcagcagggcaacgtgttcagctgcagcgtgatgcacgaggccctgcacaaccactacacacagaagtccctgtctctgagccccggcaaa

SEQ ID NO: 180 - protein, 500 aa, Artificial
  Full-length amino acid sequence of NYD-2047-HC-k
MKHLWFFLLLVAAPRWVLSGQVQLVESGGGVVQPGRSLRLSCAASGFSIRSYDMHWVRQAPGKGLEWVATISYDGSQKYYADSVKGRFTISRDNSKNTLYLQMSSLRAEDTAVYHCARGSSGHYEAFDIWGQGTLVTVSSGGGGSGGGGSGGGGSQSVLTQPPSVSAAPGQKVTISCSGSSSNIGNWYVSWYQQLPGTAPKLLIYDNNKRPSGIPDRFSGSKSGTSATLGITGLQTGDEADYYCGTWDSSLSAPWVFGGGTKVTVLGGEPKSADKTHTCPPCPAPEAAGGPSVFLFPPKPKDTLMISRTPEVTCVVVDVSHEDPEVKFNWYVDGVEVHNAKTKPREEQYNSTYRVVSVLTVLHQDWLNGKEYKCKVSNKALPAPIEKTISKAKGQPREPQVYTLPPCRDELTKNQVSLWCLVKGFYPSDIAVEWESNGQPENNYKTTPPVLDSDGSFFLYSKLTVDKSRWQQGNVFSCSVMHEALHNHYTQKSLSLSPGK

SEQ ID NO: 181 - DNA, 1500 bp, Artificial
  Full-length nucleotide sequence of NYD-2061-HC-k
atgaagcacctgtggttctttctgctgctggtggccgctcctagatgggtgctgtctggtgaggtacagctggtggaatccggtggaggccttgtgcaaccgggaggctccctgcgactctcttgcgccgcatctggcttttccatacgatcctacgatattcattgggtccgacaagcccctggcaaaggtcttgaatgggttgccactatctcctacgacgggtctcagaaatattatgcggattcagtgaaggggcggttcacaatttcacgagacgagtcaaagaatacactgtacctccaaatgaattcactgagagccgaggatactgcagtctatcattgtgcaagagggtcctcaggccactacgaggcctttgatatatggggccaaggcaccttggtaaccgttagtagcggaggtggaggaagcggaggcggcggttccggaggaggtggaagtcaatccgttctgactcagccaccctccgcctctggcaccccgggccaacgggtcacaatatcatgttctggctcttcaagcaacatcggaaactggtacgtgagctggtaccagcagctccccggcacggcgcccaagcttctgatatatgacaacaacaaacggcccagtggagttcctgacagattcagtgggtctaaaagtggtacaagcgctagcctggccataagtggtctgcagagtgaagatgaggcggactattattgcggaacctgggactccagcctgagcgctccctgggttttcggcggaggtactaagctgaccgtcttgggcggagaacccaagagcgcagacaagacccacacctgtcctccatgtcctgctccagaagctgcaggcggcccttccgtgtttctgttccctccaaagcctaaggacaccctgatgatcagccggacacctgaagtgacctgcgtggtggtggatgtgtcccacgaggatcccgaagtgaagttcaattggtacgtggacggcgtggaagtgcacaacgccaagaccaagcctagagaggaacagtacaacagcacctacagagtggtgtctgtgctgacagtgctgcaccaggactggctgaacggcaaagagtacaagtgcaaggtgtccaacaaggccctgcctgctcctatcgagaaaaccatcagcaaggccaagggccagcctagggaaccccaggtttacaccctgcctccatgcagggatgagctgaccaagaaccaggtgtccctgtggtgcctggttaagggcttctacccctccgatatcgccgtggaatgggagagcaatggccagccagagaacaactacaagacaacccctcctgtgctggactccgacggctcattcttcctgtacagcaagctgaccgtggacaagagcagatggcagcagggcaacgtgttcagctgcagcgtgatgcacgaggccctgcacaaccactacacacagaagtccctgtctctgagccccggcaaa

SEQ ID NO: 182 - protein, 500 aa, Artificial
  Full-length amino acid sequence of NYD-2061-HC-k
MKHLWFFLLLVAAPRWVLSGEVQLVESGGGLVQPGGSLRLSCAASGFSIRSYDIHWVRQAPGKGLEWVATISYDGSQKYYADSVKGRFTISRDESKNTLYLQMNSLRAEDTAVYHCARGSSGHYEAFDIWGQGTLVTVSSGGGGSGGGGSGGGGSQSVLTQPPSASGTPGQRVTISCSGSSSNIGNWYVSWYQQLPGTAPKLLIYDNNKRPSGVPDRFSGSKSGTSASLAISGLQSEDEADYYCGTWDSSLSAPWVFGGGTKLTVLGGEPKSADKTHTCPPCPAPEAAGGPSVFLFPPKPKDTLMISRTPEVTCVVVDVSHEDPEVKFNWYVDGVEVHNAKTKPREEQYNSTYRVVSVLTVLHQDWLNGKEYKCKVSNKALPAPIEKTISKAKGQPREPQVYTLPPCRDELTKNQVSLWCLVKGFYPSDIAVEWESNGQPENNYKTTPPVLDSDGSFFLYSKLTVDKSRWQQGNVFSCSVMHEALHNHYTQKSLSLSPGK

SEQ ID NO: 183 - DNA, 1515 bp, Artificial
  Full-length nucleotide sequence of NYD-3061-HC-k
atgaagcacctgtggttctttctgctgctggtggccgctcctagatgggtgctgtctggtgaggtacagctggtggaatccggtggaggccttgtgcaaccgggaggctccctgcgactctcttgcgccgcatctggcttttccatacgatcctacgatattcattgggtccgacaagcccctggcaaaggtcttgaatgggttgccactatctcctacgacgggtctcagaaatattatgcggattcagtgaaggggcggttcacaatttcacgagacgagtcaaagaatacactgtacctccaaatgaattcactgagagccgaggatactgcagtctatcattgtgcaagagggtcctcaggccactacgaggcctttgatatatggggccaaggcaccttggtaaccgttagtagcggaggtggaggaagcggaggcggcggttccggaggaggtggaagtggaggaggtggatctcaatccgttctgactcagccaccctccgcctctggcaccccgggccaacgggtcacaatatcatgttctggctcttcaagcaacatcggaaactggtacgtgagctggtaccagcagctccccggcacggcgcccaagcttctgatatatgacaacaacaaacggcccagtggagttcctgacagattcagtgggtctaaaagtggtacaagcgctagcctggccataagtggtctgcagagtgaagatgaggcggactattattgcggaacctgggactccagcctgagcgctccctgggttttcggcggaggtactaagctgaccgtcttgggcggagaacccaagagcgcagacaagacccacacctgtcctccatgtcctgctccagaagctgcaggcggcccttccgtgtttctgttccctccaaagcctaaggacaccctgatgatcagccggacacctgaagtgacctgcgtggtggtggatgtgtcccacgaggatcccgaagtgaagttcaattggtacgtggacggcgtggaagtgcacaacgccaagaccaagcctagagaggaacagtacaacagcacctacagagtggtgtctgtgctgacagtgctgcaccaggactggctgaacggcaaagagtacaagtgcaaggtgtccaacaaggccctgcctgctcctatcgagaaaaccatcagcaaggccaagggccagcctagggaaccccaggtttacaccctgcctccatgcagggatgagctgaccaagaaccaggtgtccctgtggtgcctggttaagggcttctacccctccgatatcgccgtggaatgggagagcaatggccagccagagaacaactacaagacaacccctcctgtgctggactccgacggctcattcttcctgtacagcaagctgaccgtggacaagagcagatggcagcagggcaacgtgttcagctgcagcgtgatgcacgaggccctgcacaaccactacacacagaagtccctgtctctgagccccggcaaa

SEQ ID NO: 184 - protein, 505 aa, Artificial
  Full-length amino acid sequence of NYD-3061-HC-k
MKHLWFFLLLVAAPRWVLSGEVQLVESGGGLVQPGGSLRLSCAASGFSIRSYDIHWVRQAPGKGLEWVATISYDGSQKYYADSVKGRFTISRDESKNTLYLQMNSLRAEDTAVYHCARGSSGHYEAFDIWGQGTLVTVSSGGGGSGGGGSGGGGSGGGGSQSVLTQPPSASGTPGQRVTISCSGSSSNIGNWYVSWYQQLPGTAPKLLIYDNNKRPSGVPDRFSGSKSGTSASLAISGLQSEDEADYYCGTWDSSLSAPWVFGGGTKLTVLGGEPKSADKTHTCPPCPAPEAAGGPSVFLFPPKPKDTLMISRTPEVTCVVVDVSHEDPEVKFNWYVDGVEVHNAKTKPREEQYNSTYRVVSVLTVLHQDWLNGKEYKCKVSNKALPAPIEKTISKAKGQPREPQVYTLPPCRDELTKNQVSLWCLVKGFYPSDIAVEWESNGQPENNYKTTPPVLDSDGSFFLYSKLTVDKSRWQQGNVFSCSVMHEALHNHYTQKSLSLSPGK

SEQ ID NO: 185 - DNA, 1527 bp, Artificial
  Full-length nucleotide sequence of NYC-0011-HC-k
atgaagcacctgtggttctttctgctgctggtggccgctcctagatgggtgctgtctggcgaagtgcagctggtggaatctggtggcggagttgttcagcctggcggctctctgagactgagctgtgtggccagcggcttcaccttcgacgactacgccatgtactgggtccgacaggtgccaggcaaggacctggaatgggtgtccctgatttctggcgacggcgacatcacctactacgtggactctgtgaagggcagattcaccgtgtccagagacaacaacaagaacagcctgtacctgcagatgaagtccctgcgcgtggaagatacagccctgtactactgcgccaaggacatgatctactacgcctcttggagcggctacggcagcagcgattactactactatgtgatggacgtgtggggccagggcaccaccgttacagtttctagcggaggcggaggaagtggcggcggaggatctggcggtggtggttctgatatccagatgacacagagccccagcagcctgtctgcctctgtgggagacagagtgaccatcacctgtagagccagccagagcatcagcagctacctgaactggtatcagcagaagcccggcaaggcccctaaactgctgatctatgccgcctccagtctgcagagcggagtgcctagcagattttctggcagcggctccggcaccgatttcaccctgaccatatctagcctgcagcctgaggacttcgccacctactattgccagcagagctacagcacccctcctatcacctttggccagggaaccagactggaaatcaaaggcggagaacccaagagcgcagacaagacccacacctgtcctccatgtcctgctccagaagctgcaggcggcccttccgtgtttctgttccctccaaagcctaaggacaccctgatgatcagccggacacctgaagtgacctgcgtggtggtggatgtgtcccacgaggatcccgaagtgaagttcaattggtacgtggacggcgtggaagtgcacaacgccaagaccaagcctagagaggaacagtacaacagcacctacagagtggtgtctgtgctgacagtgctgcaccaggactggctgaacggcaaagagtacaagtgcaaggtgtccaacaaggccctgcctgctcctatcgagaaaaccatcagcaaggccaagggccagcctagggaaccccaggtttacaccctgcctccatgcagggatgagctgaccaagaaccaggtgtccctgtggtgcctggttaagggcttctacccctccgatatcgccgtggaatgggagagcaatggccagccagagaacaactacaagacaacccctcctgtgctggactccgacggctcattcttcctgtacagcaagctgaccgtggacaagagcagatggcagcagggcaacgtgttcagctgcagcgtgatgcacgaggccctgcacaaccactacacacagaagtccctgtctctgagccccggcaaa

SEQ ID NO: 186 - protein, 509 aa, Artificial
  Full-length amino acid sequence of NYC-0011-HC-k
MKHLWFFLLLVAAPRWVLSGEVQLVESGGGVVQPGGSLRLSCVASGFTFDDYAMYWVRQVPGKDLEWVSLISGDGDITYYVDSVKGRFTVSRDNNKNSLYLQMKSLRVEDTALYYCAKDMIYYASWSGYGSSDYYYYVMDVWGQGTTVTVSSGGGGSGGGGSGGGGSDIQMTQSPSSLSASVGDRVTITCRASQSISSYLNWYQQKPGKAPKLLIYAASSLQSGVPSRFSGSGSGTDFTLTISSLQPEDFATYYCQQSYSTPPITFGQGTRLEIKGGEPKSADKTHTCPPCPAPEAAGGPSVFLFPPKPKDTLMISRTPEVTCVVVDVSHEDPEVKFNWYVDGVEVHNAKTKPREEQYNSTYRVVSVLTVLHQDWLNGKEYKCKVSNKALPAPIEKTISKAKGQPREPQVYTLPPCRDELTKNQVSLWCLVKGFYPSDIAVEWESNGQPENNYKTTPPVLDSDGSFFLYSKLTVDKSRWQQGNVFSCSVMHEALHNHYTQKSLSLSPGK

SEQ ID NO: 187 - DNA, 1527 bp, Artificial
  Full-length nucleotide sequence of NYC-0012-HC-k
atgaagcacctgtggttctttctgctgctggtggccgctcctagatgggtgctgtctggcgaagtgcagctggtggaatctggtggcggagttgttcagcctggcggctctctgagactgtcttgtgccgccagcggcttcaccttcgacgactacgccatgtactgggtccgacaggcccctggcaaaggccttgaatgggtgtccctgatcagcggagatggcggcagcatgtactacgccgatagcgtgaagggcagattcaccatcagccgggacaacagcaagaacagcctgtacctgcagatgaactccctgcggaccgaggacacagccctgtactactgcgccaaggatatgatcttctacgccttttggagcggctacggcagcagcgattactactactacgtgatggacgtgtggggccagggcaccacagtgacagtttattctggcggcggaggatctggcggaggtggaagcggaggcggtggatctgatatccagatgacacagagccccagcagcctgtctgcctctgtgggagacagagtgaccatcacctgtcgggccagccagagaatcagcacctacctgaactggtatcagcagaagcccggcaaggcccctaagctgctgatctatgctgcctccagtctgcagagcggcgtgccaagcagattttctggcagcggctctggcaccgacttcaccctgaccatatctagcctgcagcctgaggacttcgccacctactactgccagcagagctacagcacccctcctatcacctttggccagggaaccagactggaaatcaaaggcggagaacccaagagcgcagacaagacccacacctgtcctccatgtcctgctccagaagctgcaggcggcccttccgtgtttctgttccctccaaagcctaaggacaccctgatgatcagccggacacctgaagtgacctgcgtggtggtggatgtgtcccacgaggatcccgaagtgaagttcaattggtacgtggacggcgtggaagtgcacaacgccaagaccaagcctagagaggaacagtacaacagcacctacagagtggtgtctgtgctgacagtgctgcaccaggactggctgaacggcaaagagtacaagtgcaaggtgtccaacaaggccctgcctgctcctatcgagaaaaccatcagcaaggccaagggccagcctagggaaccccaggtttacaccctgcctccatgcagggatgagctgaccaagaaccaggtgtccctgtggtgcctggttaagggcttctacccctccgatatcgccgtggaatgggagagcaatggccagccagagaacaactacaagacaacccctcctgtgctggactccgacggctcattcttcctgtacagcaagctgaccgtggacaagagcagatggcagcagggcaacgtgttcagctgcagcgtgatgcacgaggccctgcacaaccactacacacagaagtccctgtctctgagccccggcaaa

SEQ ID NO: 188 - protein, 509 aa, Artificial
  Full-length amino acid sequence of NYC-0012-HC-k
MKHLWFFLLLVAAPRWVLSGEVQLVESGGGVVQPGGSLRLSCAASGFTFDDYAMYWVRQAPGKGLEWVSLISGDGGSMYYADSVKGRFTISRDNSKNSLYLQMNSLRTEDTALYYCAKDMIFYAFWSGYGSSDYYYYVMDVWGQGTTVTVYSGGGGSGGGGSGGGGSDIQMTQSPSSLSASVGDRVTITCRASQRISTYLNWYQQKPGKAPKLLIYAASSLQSGVPSRFSGSGSGTDFTLTISSLQPEDFATYYCQQSYSTPPITFGQGTRLEIKGGEPKSADKTHTCPPCPAPEAAGGPSVFLFPPKPKDTLMISRTPEVTCVVVDVSHEDPEVKFNWYVDGVEVHNAKTKPREEQYNSTYRVVSVLTVLHQDWLNGKEYKCKVSNKALPAPIEKTISKAKGQPREPQVYTLPPCRDELTKNQVSLWCLVKGFYPSDIAVEWESNGQPENNYKTTPPVLDSDGSFFLYSKLTVDKSRWQQGNVFSCSVMHEALHNHYTQKSLSLSPGK

SEQ ID NO: 189 - DNA, 1512 bp, Artificial
  Full-length nucleotide sequence of NYC-0013-HC-k
atgaagcacctgtggttctttctgctgctggtggccgctcctagatgggtgctgtctggcgaagtgcagctggtggaatctggtggcggagttgttcagcctggcggctctctgagactgtcttgtgccgccagcggcttcaccttcgacgattatgccatgcactgggtccgacaggcccctggcaaaggacttgaatgggtgtccctgatcagcggcgacggcgacaatacctactacgccgatagcgtgaagggcagattcaccatcagccgggacaacaacaagaacagcctgtacctgcagatgaactccctgcggaccgaggacaccgccttctactactgtgccaaagagctgatcttcggcaaggtgctgcacgacttttactactacgtgatggacgtgtggggccagggcaccacagtgacagtttctagcggaggcggaggaagtggcggcggaggatctggcggtggtggttctgatatccagatgacacagagccccagcagcctgtctgcctctgtgggagacagagtgaccatcacctgtagagccagccagagcatcagcagctacctgaactggtatcagcagaagcccggcaaggcccctaaactgctgatctatgccgcctccagtctgcagagcggagtgcctagcagattttctggcagcggctccggcaccgatttcaccctgaccatatctagcctgcagcctgaggacttcgccacctactactgccagcagagctacagcacccctcctatcacctttggccagggaaccagactggaaatcaaaggcggagaacccaagagcgcagacaagacccacacctgtcctccatgtcctgctccagaagctgcaggcggcccttccgtgtttctgttccctccaaagcctaaggacaccctgatgatcagccggacacctgaagtgacctgcgtggtggtggatgtgtcccacgaggatcccgaagtgaagttcaattggtacgtggacggcgtggaagtgcacaacgccaagaccaagcctagagaggaacagtacaacagcacctacagagtggtgtctgtgctgacagtgctgcaccaggactggctgaacggcaaagagtacaagtgcaaggtgtccaacaaggccctgcctgctcctatcgagaaaaccatcagcaaggccaagggccagcctagggaaccccaggtttacaccctgcctccatgcagggatgagctgaccaagaaccaggtgtccctgtggtgcctggttaagggcttctacccctccgatatcgccgtggaatgggagagcaatggccagccagagaacaactacaagacaacccctcctgtgctggactccgacggctcattcttcctgtacagcaagctgaccgtggacaagagcagatggcagcagggcaacgtgttcagctgcagcgtgatgcacgaggccctgcacaaccactacacacagaagtccctgtctctgagccccggcaaa

SEQ ID NO: 190 - protein, 504 aa, Artificial
  Full-length amino acid sequence of NYC-0013-HC-k
MKHLWFFLLLVAAPRWVLSGEVQLVESGGGVVQPGGSLRLSCAASGFTFDDYAMHWVRQAPGKGLEWVSLISGDGDNTYYADSVKGRFTISRDNNKNSLYLQMNSLRTEDTAFYYCAKELIFGKVLHDFYYYVMDVWGQGTTVTVSSGGGGSGGGGSGGGGSDIQMTQSPSSLSASVGDRVTITCRASQSISSYLNWYQQKPGKAPKLLIYAASSLQSGVPSRFSGSGSGTDFTLTISSLQPEDFATYYCQQSYSTPPITFGQGTRLEIKGGEPKSADKTHTCPPCPAPEAAGGPSVFLFPPKPKDTLMISRTPEVTCVVVDVSHEDPEVKFNWYVDGVEVHNAKTKPREEQYNSTYRVVSVLTVLHQDWLNGKEYKCKVSNKALPAPIEKTISKAKGQPREPQVYTLPPCRDELTKNQVSLWCLVKGFYPSDIAVEWESNGQPENNYKTTPPVLDSDGSFFLYSKLTVDKSRWQQGNVFSCSVMHEALHNHYTQKSLSLSPGK

SEQ ID NO: 191 - DNA, 1512 bp, Artificial
  Full-length nucleotide sequence of NYC-0014-HC-k
atgaagcacctgtggttctttctgctgctggtggccgctcctagatgggtgctgtctggcgaagtgcagctggtggaatctggtggcggagttgttcagcctggcggctctctgagactgagctgtgaagcctccggcttcatcttcgacgactacgccatgcactgggtccgacaggcacctggcaaaggccttgaatgggtgtccctgatctctggcgacggcgacatcatctactacgccgactctgtgaagggcagattcaccatcagccgggacaacagcaagaacagcctgtacctgcagatgaactccctgatcatcgaggacacagccctgtactactgcgccaaggattgggtgttcggcgtcgtgatgacccactactggtacttcggcctggatgtgtggggccagggaaccacagtgacagtttctagcggaggcggaggaagtggcggcggaggatctggcggtggtggttctgatatccagatgacacagagccccagcagcctgtctgcctctgaaggcgacagagtgaccatcacctgtagagccagccagagcatcagcacctacctgaactggtatcagcagaagcccggcaaggcccctaagctgctgatctatggtgcctccagtctgcagagcggcgtgccaagcagattttctggcagcggctctggcaccgacttcaccctgaccatatctagcctgcagcctgaggacttcgccacctactactgccagcagtcctacagcacccctcctatcacatttggccagggcaccaaggtggaaatcaaaggcggagaacccaagagcgcagacaagacccacacctgtcctccatgtcctgctccagaagctgcaggcggcccttccgtgtttctgttccctccaaagcctaaggacaccctgatgatcagccggacacctgaagtgacctgcgtggtggtggatgtgtcccacgaggatcccgaagtgaagttcaattggtacgtggacggcgtggaagtgcacaacgccaagaccaagcctagagaggaacagtacaacagcacctacagagtggtgtctgtgctgacagtgctgcaccaggactggctgaacggcaaagagtacaagtgcaaggtgtccaacaaggccctgcctgctcctatcgagaaaaccatcagcaaggccaagggccagcctagggaaccccaggtttacaccctgcctccatgcagggatgagctgaccaagaaccaggtgtccctgtggtgcctggttaagggcttctacccctccgatatcgccgtggaatgggagagcaatggccagccagagaacaactacaagacaacccctcctgtgctggactccgacggctcattcttcctgtacagcaagctgaccgtggacaagagcagatggcagcagggcaacgtgttcagctgcagcgtgatgcacgaggccctgcacaaccactacacacagaagtccctgtctctgagccccggcaaa

SEQ ID NO: 192 - protein, 504 aa, Artificial
  Full-length amino acid sequence of NYC-0014-HC-k
MKHLWFFLLLVAAPRWVLSGEVQLVESGGGVVQPGGSLRLSCEASGFIFDDYAMHWVRQAPGKGLEWVSLISGDGDIIYYADSVKGRFTISRDNSKNSLYLQMNSLIIEDTALYYCAKDWVFGVVMTHYWYFGLDVWGQGTTVTVSSGGGGSGGGGSGGGGSDIQMTQSPSSLSASEGDRVTITCRASQSISTYLNWYQQKPGKAPKLLIYGASSLQSGVPSRFSGSGSGTDFTLTISSLQPEDFATYYCQQSYSTPPITFGQGTKVEIKGGEPKSADKTHTCPPCPAPEAAGGPSVFLFPPKPKDTLMISRTPEVTCVVVDVSHEDPEVKFNWYVDGVEVHNAKTKPREEQYNSTYRVVSVLTVLHQDWLNGKEYKCKVSNKALPAPIEKTISKAKGQPREPQVYTLPPCRDELTKNQVSLWCLVKGFYPSDIAVEWESNGQPENNYKTTPPVLDSDGSFFLYSKLTVDKSRWQQGNVFSCSVMHEALHNHYTQKSLSLSPGK

SEQ ID NO: 193 - DNA, 1509 bp, Artificial
  Full-length nucleotide sequence of NYC-0015-HC-k
atgaagcacctgtggttctttctgctgctggtggccgctcctagatgggtgctgtctggcgaagtgcagctggtggaatctggtggcggagttgttcagcctggcggctctctgagactgtcttgtgccgccagcggcttcaccttcgacgattatgccatgcactgggtccgacaggcccctggcaaaggacttgaatgggtgtccctgatctctggcggaggcggcggaacctactacagcgattctgtgaagggcagattcaccatcagccgggacaccagcaaggacagcctgtacctgcagatgaacagcctgcggaccgaggacacagccctgtactactgcgccaaggacatggtgttcggcgtggtcaccccttactactacttcgccctggatgtgtggggccagggcacaacagtgacagtctcttctggcggcggaggaagcggaggcggaggatccggtggtggtggatctgacatccagatgacacagagccccagcagcctgtctgcctctgtgggagacagagtgaccatcacctgtagagccagccagagcatcaacagctacctgaactggtatcagcagaagcccggcaaggcccctaagctgctgatctatgctgcctccagtctgcagagcggcgtgccaagcagattttctggcagcggctctggcaccgacttcaccctgaccatatctagcctgcagcctgaggacttcgccacctactactgccagcagagctacagcgcccctcctatcacatttggccagggaaccagactggaaatcaaaggcggagaacccaagagcgcagacaagacccacacctgtcctccatgtcctgctccagaagctgcaggcggcccttccgtgtttctgttccctccaaagcctaaggacaccctgatgatcagccggacacctgaagtgacctgcgtggtggtggatgtgtcccacgaggatcccgaagtgaagttcaattggtacgtggacggcgtggaagtgcacaacgccaagaccaagcctagagaggaacagtacaacagcacctacagagtggtgtctgtgctgacagtgctgcaccaggactggctgaacggcaaagagtacaagtgcaaggtgtccaacaaggccctgcctgctcctatcgagaaaaccatcagcaaggccaagggccagcctagggaaccccaggtttacaccctgcctccatgcagggatgagctgaccaagaaccaggtgtccctgtggtgcctggttaagggcttctacccctccgatatcgccgtggaatgggagagcaatggccagccagagaacaactacaagacaacccctcctgtgctggactccgacggctcattcttcctgtacagcaagctgaccgtggacaagagcagatggcagcagggcaacgtgttcagctgcagcgtgatgcacgaggccctgcacaaccactacacacagaagtccctgtctctgagccccggcaaa

SEQ ID NO: 194 - protein, 503 aa, Artificial
  Full-length amino acid sequence of NYC-0015-HC-k
MKHLWFFLLLVAAPRWVLSGEVQLVESGGGVVQPGGSLRLSCAASGFTFDDYAMHWVRQAPGKGLEWVSLISGGGGGTYYSDSVKGRFTISRDTSKDSLYLQMNSLRTEDTALYYCAKDMVFGVVTPYYYFALDVWGQGTTVTVSSGGGGSGGGGSGGGGSDIQMTQSPSSLSASVGDRVTITCRASQSINSYLNWYQQKPGKAPKLLIYAASSLQSGVPSRFSGSGSGTDFTLTISSLQPEDFATYYCQQSYSAPPITFGQGTRLEIKGGEPKSADKTHTCPPCPAPEAAGGPSVFLFPPKPKDTLMISRTPEVTCVVVDVSHEDPEVKFNWYVDGVEVHNAKTKPREEQYNSTYRVVSVLTVLHQDWLNGKEYKCKVSNKALPAPIEKTISKAKGQPREPQVYTLPPCRDELTKNQVSLWCLVKGFYPSDIAVEWESNGQPENNYKTTPPVLDSDGSFFLYSKLTVDKSRWQQGNVFSCSVMHEALHNHYTQKSLSLSPGK

SEQ ID NO: 195 - DNA, 1512 bp, Artificial
  Full-length nucleotide sequence of NYC-0016-HC-k
atgaagcacctgtggttctttctgctgctggtggccgctcctagatgggtgctgtctggcgaagtgcagctggtggaatctggtggcggagttgttcagcctggcggctctctgagactgagctgtgctgtgtccggcttcaccttcgacgactacgccatgcactgggtccgacaggcacctggcaaaggccttgaatgggtgtccctgatcagcggagatggcggcagcacacactacgccgattctgtgaagggcagattcaccatcagccgggacaacagcaagaacagcctgtacctgcagatgaactccctgcggacaggcgacacagccctgtactactgcgccaaggacatgatcttcgccgtggtcatcaccgactaccactactacggcatggacgtgtggggccagggaaccacagtgacagtttctagcggaggcggaggaagtggcggcggaggatctggcggtggtggttctgatatccagatgacacagagccccagcagcctgtctgcctctgtgggagacagagtgaccatcacctgtagagccagccagagcatcagcagctacctgaactggtatcagcagaagcccggcaaggcccctaaactgctgatctatgccgcctccagtctgcagagcggagtgcctagcagattttctggcagcggctccggcaccgatttcaccctgaccatatctagcctgcagcctgaggacttcgccacctactactgccagcagagctacagcacccctcctatcacctttggccagggcaccagactggaaatcaaaggcggagaacccaagagcgcagacaagacccacacctgtcctccatgtcctgctccagaagctgcaggcggcccttccgtgtttctgttccctccaaagcctaaggacaccctgatgatcagccggacacctgaagtgacctgcgtggtggtggatgtgtcccacgaggatcccgaagtgaagttcaattggtacgtggacggcgtggaagtgcacaacgccaagaccaagcctagagaggaacagtacaacagcacctacagagtggtgtctgtgctgacagtgctgcaccaggactggctgaacggcaaagagtacaagtgcaaggtgtccaacaaggccctgcctgctcctatcgagaaaaccatcagcaaggccaagggccagcctagggaaccccaggtttacaccctgcctccatgcagggatgagctgaccaagaaccaggtgtccctgtggtgcctggttaagggcttctacccctccgatatcgccgtggaatgggagagcaatggccagccagagaacaactacaagacaacccctcctgtgctggactccgacggctcattcttcctgtacagcaagctgaccgtggacaagagcagatggcagcagggcaacgtgttcagctgcagcgtgatgcacgaggccctgcacaaccactacacacagaagtccctgtctctgagccccggcaaa

SEQ ID NO: 196 - protein, 504 aa, Artificial
  Full-length amino acid sequence of NYC-0016-HC-k
MKHLWFFLLLVAAPRWVLSGEVQLVESGGGVVQPGGSLRLSCAVSGFTFDDYAMHWVRQAPGKGLEWVSLISGDGGSTHYADSVKGRFTISRDNSKNSLYLQMNSLRTGDTALYYCAKDMIFAVVITDYHYYGMDVWGQGTTVTVSSGGGGSGGGGSGGGGSDIQMTQSPSSLSASVGDRVTITCRASQSISSYLNWYQQKPGKAPKLLIYAASSLQSGVPSRFSGSGSGTDFTLTISSLQPEDFATYYCQQSYSTPPITFGQGTRLEIKGGEPKSADKTHTCPPCPAPEAAGGPSVFLFPPKPKDTLMISRTPEVTCVVVDVSHEDPEVKFNWYVDGVEVHNAKTKPREEQYNSTYRVVSVLTVLHQDWLNGKEYKCKVSNKALPAPIEKTISKAKGQPREPQVYTLPPCRDELTKNQVSLWCLVKGFYPSDIAVEWESNGQPENNYKTTPPVLDSDGSFFLYSKLTVDKSRWQQGNVFSCSVMHEALHNHYTQKSLSLSPGK

SEQ ID NO: 197 - protein, 719 aa, Artificial
  Full-length amino acid sequence of NYZ-1007-HC2
MKHLWFFLLLVAAPRWVLSGEVQLVESGGGLVQPGGSLRLSCAASGFSIRSYDIHWVRQAPGKGLEWVATISYDGSQKYYADSVKGRFTISRDESKNTLYLQMNSLRAEDTAVYHCARGSSGHYEAFDIWGQGTLVTVSSGGGGSGGGGSGGGGSQSVLTQPPSASGTPGQRVTISCSGSSSNIGNWYVSWYQQLPGTAPKLLIYDNNKRPSGVPDRFSGSKSGTSASLAISGLQSEDEADYYCGTWDSSLSAPWVFGGGTKLTVLGGGGSEVQLVESGGGLVQPGGSLRLSCAASGVTFNYYGMSWIRQAPGKGLEWVASITRSGGRIYYPDSVKGRFTISRENTQKTLYLQMNSLRAEDTAVYYCTLDGRDGWVAYWGQGTLVTVSSASTKGPSVFPLAPSSKSTSGGTAALGCLVKDYFPEPVTVSWNSGALTSGVHTFPAVLQSSGLYSLSSVVTVPSSSLGTQTYICNVNHKPSNTKVDKRVEPKSCDKTHTCPPCPAPEAAGGPSVFLFPPKPKDTLMISRTPEVTCVVVSVSHEDPEVKFNWYVDGVEVHNAKTKPREEQYNSTYRVVSVLTVLHQDWLNGKEYKCKVSNKALPAPIEKTISKAKGQPREPQVYVYPPSRDELTKNQVSLTCLVKGFYPSDIAVEWESNGQPENNYKTTPPVLDSDGSFALVSKLTVDKSRWQQGNVFSCSVMHEALHNHYTQKSLSLSPGK

SEQ ID NO: 198 - protein, 719 aa, Artificial
  Full-length amino acid sequence of NYZ-1017-HC2
MKHLWFFLLLVAAPRWVLSGQVQLVESGGGVVQPGRSLRLSCAASGFSIRSYDMHWVRQAPGKGLEWVATISYDGSQKYYADSVKGRFTISRDNSKNTLYLQMSSLRAEDTAVYHCARGSSGHYEAFDIWGQGTLVTVSSGGGGSGGGGSGGGGSQSVLTQPPSVSAAPGQKVTISCSGSSSNIGNWYVSWYQQLPGTAPKLLIYDNNKRPSGIPDRFSGSKSGTSATLGITGLQTGDEADYYCGTWDSSLSAPWVFGGGTKVTVLGGGGSEVQLVESGGGLVQPGGSLRLSCAASGVTFNYYGMSWIRQAPGKGLEWVASITRSGGRIYYPDSVKGRFTISRENTQKTLYLQMNSLRAEDTAVYYCTLDGRDGWVAYWGQGTLVTVSSASTKGPSVFPLAPSSKSTSGGTAALGCLVKDYFPEPVTVSWNSGALTSGVHTFPAVLQSSGLYSLSSVVTVPSSSLGTQTYICNVNHKPSNTKVDKRVEPKSCDKTHTCPPCPAPEAAGGPSVFLFPPKPKDTLMISRTPEVTCVVVSVSHEDPEVKFNWYVDGVEVHNAKTKPREEQYNSTYRVVSVLTVLHQDWLNGKEYKCKVSNKALPAPIEKTISKAKGQPREPQVYVYPPSRDELTKNQVSLTCLVKGFYPSDIAVEWESNGQPENNYKTTPPVLDSDGSFALVSKLTVDKSRWQQGNVFSCSVMHEALHNHYTQKSLSLSPGK